European Patent Specification EP 3 615 552 B1, published June 17, 2026. Title: METHODS AND COMPOSITIONS OF ANTI-CRISPR PROTEINS FOR USE IN PLANTS. Applicant: DuPont Nutrition Biosciences APS Universite Laval Fremaux, Christophe Horvath, Philippe Hynes, Alexander Lemay, Marie-Laurence Moineau, Sylvain Romero, Dennis  A Rousseau, Genevieve Young, Joshua. The sequence listing filed with the application follows.

SEQUENCE LISTING (650 sequences)

SEQ ID NO: 1 - DNA, 327 bp, Bacteriophage O1205
atggcatacggaaaaagcagatacaactcatataggaaacgcagtttcaatagaagcgataagcaacgtagagaatacgcacaagaaatggatagattagaacaaacatttgaaaaacttgatggttggtatctatctagcatgaaagatagtgcgtataaagatttcggaaaatacgaaattcgcttatcaaatcattcagcagacaacaaatatcatgacctagaaaatggtcgtttaattgttaatgtcaaagcaagtaaattgaaattcgttgatatcaaatgttactataagggatttaagacaaagaaggatgtaatctaa

SEQ ID NO: 2 - protein, 108 aa, Bacteriophage O1205
MAYGKSRYNSYRKRSFNRSDKQRREYAQEMDRLEQTFEKLDGWYLSSMKDSAYKDFGKYEIRLSNHSADNKYHDLENGRLIVNVKASKLKFVDIKCYYKGFKTKKDVI

SEQ ID NO: 3 - DNA, 423 bp, Bacteriophage Sfi21
atggcatacggaaaaagtagatataactcatatagaaagcgcagttttaacagaagtaataagcaacgtagagaatacgcacaagaaatggatagattagagaaagctttcgaaaatcttgacggatggtatctatctagcatgaaagatagtgcgtacaaagatttcggaaaatacgaaattcgcttatcaaatcattcagcagacaacaaatatcatgacctagaaaatggtcgtttaattgttaatgtcaaagcaagtaaattgaacttcgttgatatcatcgagaacaaacttgataaaatcattgagaagattgatactcttgatttagataagtacagattcattaatgctactaaattggaacgtgatatcaaatgctactataaaggctataagacaaagaaggatgtaatctaa

SEQ ID NO: 4 - protein, 140 aa, Bacteriophage Sfi21
MAYGKSRYNSYRKRSFNRSNKQRREYAQEMDRLEKAFENLDGWYLSSMKDSAYKDFGKYEIRLSNHSADNKYHDLENGRLIVNVKASKLNFVDIIENKLDKIIEKIDTLDLDKYRFINATKLERDIKCYYKGYKTKKDVI

SEQ ID NO: 5 - DNA, 423 bp, Bacteriophage TP-778L
atggcatacggaaaaagcagatacaactcatatagaaaacgtagtttcaacataagtgacacaaagcgtagggaatatgcaaaagaaatggagaaattagaacaagcatttgaaaagctagatggttggtatctatctagcatgaaggatagtgcatacaaggattttggaaaatacgaaatccgcttatcaaatcattcagcagacaataaatatcatgacctagaaaatggtcgtttaattgttaatgttaaagcaagtaaattgaacttcgttgatatcatcgaaaacaaacttgataaaatcatcgagaagattgataagcttgatttagataagtacagatttattaacgctactagaatggagcatgacattaaatgctactataaaggatttaagacaaagaaagatgtaatctaa

SEQ ID NO: 6 - protein, 140 aa, Bacteriophage TP-778L
MAYGKSRYNSYRKRSFNISDTKRREYAKEMEKLEQAFEKLDGWYLSSMKDSAYKDFGKYEIRLSNHSADNKYHDLENGRLIVNVKASKLNFVDIIENKLDKIIEKIDKLDLDKYRFINATRMEHDIKCYYKGFKTKKDVI

SEQ ID NO: 7 - DNA, 423 bp, Streptococcus sp. HMSC072D07
atggcatttggcaagaacagatacaatccatacaggaaacgtagttttaatcgtagtgataaacaatgtcgagagtatgctcaggcaatggacgaactagaacaagcctttgaggaacttgatggatggcacttatctagtatgatggatagtgcttataagaattttgaaaagtaccaggttcgcctatcaaatcattcagcagacaaccaatatcatgacttagaaaatggttacttgattgtcaatgttaaagcaagtaaattgaactttgtcgatattatcgaaaataaattggataagattttagagaaagtagacaagcttgatcttgataagtataggtttatcaatgcgaccaatctggaacatgatattaaatgttatctcaaaggctataagacgaaaaaagacgtgatttaa

SEQ ID NO: 8 - protein, 140 aa, Streptococcus sp. HMSC072D07
MAFGKNRYNPYRKRSFNRSDKQCREYAQAMDELEQAFEELDGWHLSSMMDSAYKNFEKYQVRLSNHSADNQYHDLENGYLIVNVKASKLNFVDIIENKLDKILEKVDKLDLDKYRFINATNLEHDIKCYLKGYKTKKDVI

SEQ ID NO: 9 - DNA, 423 bp, Bacteriophage D4276
atggcatacggaaaaagtagatataactcatatagaaagcgcagttttaacagaagtaataagcaacgtagagaatacgcacaagaaatggatagattagagaaagctttcgaaaatcttgacggatggtatctatctagcatgaaagacagtgcttacaaggattttgggaaatacgaaattcgcttatcaaatcattcggcagacaacaaatatcacgacttagaaaacggtcgtttaattgttaatattaaagctagtaaattgaatttcgttgatatcatcgagaataagcttgataaaataatcgagaagattgataagcttgatttagataagtaccgattcatcaatgcgaccaacctagagcatgatatcaaatgctattacaaggggtttaaaacgaaaaaggaggtaatctaa

SEQ ID NO: 10 - protein, 140 aa, Bacteriophage D4276
MAYGKSRYNSYRKRSFNRSNKQRREYAQEMDRLEKAFENLDGWYLSSMKDSAYKDFGKYEIRLSNHSADNKYHDLENGRLIVNIKASKLNFVDIIENKLDKIIEKIDKLDLDKYRFINATNLEHDIKCYYKGFKTKKEVI

SEQ ID NO: 11 - DNA, 423 bp, Bacteriophage D1126
atggcatacggaaaaagcagatacaattcatataggaagcgaaacttctctataagcgacaatcagcgtagggaatatgctaaaaaaatgaaggagttagaacaagcgtttgaaaaccttgacggatggtatctatctagcatgaaagatagtgcgtacaaagatttcggaaaatacgaaattcgcttatcaaatcattcagcagacaatagatatcatgacctagaaaatggtcgcttaatcgttaatgttaaagctagtaaattgaacttcgttgatatcatcgagaataaacttggtaaaatcattgagaagattgatactcttgatttagataagtacagattcattaatgctactaaattggaacgtgatatcaaatgctactataaaggctataagacaaagaaggatgtaatctaa

SEQ ID NO: 12 - protein, 140 aa, Bacteriophage D1126
MAYGKSRYNSYRKRNFSISDNQRREYAKKMKELEQAFENLDGWYLSSMKDSAYKDFGKYEIRLSNHSADNRYHDLENGRLIVNVKASKLNFVDIIENKLGKIIEKIDTLDLDKYRFINATKLERDIKCYYKGYKTKKDVI

SEQ ID NO: 13 - DNA, 423 bp, Bacteriophage D4250
atggcatacggaaaaagtagatataactcatatagaaaacgcagtttcaacagaagcgataaacagcgtagagaatacgcacaagcaatggaagaattagagcaagcatttgaaaactttgatgattggtatctatcaagcatgaaagacagtgcttacaaggattttgggaaatacgaaattcgcttatcaaatcattcggcagacaacaaatatcacgacttagaaaacggtcgtttaattgttaatattaaagctagtaaattgaatttcgttgatatcatcgagaataagcttgataaaataatcgagaagattgataagcttgatttagataagtaccgattcatcaatgcgaccaacctagagcatgatatcaaatgctattacaaggggtttaaaacgaaaaaggaggtaatctaa

SEQ ID NO: 14 - protein, 140 aa, Bacteriophage D4250
MAYGKSRYNSYRKRSFNRSDKQRREYAQAMEELEQAFENFDDWYLSSMKDSAYKDFGKYEIRLSNHSADNKYHDLENGRLIVNIKASKLNFVDIIENKLDKIIEKIDKLDLDKYRFINATNLEHDIKCYYKGFKTKKEVI

SEQ ID NO: 15 - DNA, 423 bp, Bacteriophage D4252
atggcatacggaaaaagcagatacaactcatatagaaagcgcagttttaacagaagtgataagcaacgtagagaatacgctaaaaaaatgaaggagttagaacaagcgtttgaaaaccttgatggttggtatctatcgagcatgaatgacagtgcttataaaaattttggcaaatatgaagttcgattgtcaaatcattcggcagataataaatatcacgacatagaaaacggtcgtttaattgttaatgttaaagctagtaaattgaatttcgttgatatcatcgagaacaagcttgataaaataatcgagaagattgataagcttgatttagataagtaccgattcatcaacgctaccaatctagagcataatattaaatgctattacaagggatttaagacaaagaaggatgtaatataa

SEQ ID NO: 16 - protein, 140 aa, Bacteriophage D4252
MAYGKSRYNSYRKRSFNRSDKQRREYAKKMKELEQAFENLDGWYLSSMNDSAYKNFGKYEVRLSNHSADNKYHDIENGRLIVNVKASKLNFVDIIENKLDKIIEKIDKLDLDKYRFINATNLEHNIKCYYKGFKTKKDVI

SEQ ID NO: 17 - DNA, 423 bp, Bacteriophage D4598
atggcatacggaaaaagtagatataactcatatagaaaacgcagtttcaacagaagcgataaacagcgtggagaatacgcacaagcaatggaagaattagagcaagcatttgaaaactttgatgattggtatctatcaagcatgaaagacagtgcttacaaggattttgggaaatacgaaattcgcttatcaaatcattcggcagacaataaatatcatgacctagaaaatggtcgcttaatcgttaatgttaaagctagtaaattgaacttcgtcgatatcatcgagaataaaatcgataaaatcattgagaagattgataagcttgatttagataagtaccgattcatcaacgctaccaacctagagcatgatatcaaatgttattacaagggatttaagacaaaaaaggatgtaatctaa

SEQ ID NO: 18 - protein, 140 aa, Bacteriophage D4598
MAYGKSRYNSYRKRSFNRSDKQRGEYAQAMEELEQAFENFDDWYLSSMKDSAYKDFGKYEIRLSNHSADNKYHDLENGRLIVNVKASKLNFVDIIENKIDKIIEKIDKLDLDKYRFINATNLEHDIKCYYKGFKTKKDVI

SEQ ID NO: 19 - DNA, 423 bp, Streptococcus mutans
atggcatttggaaaaagaagatataactcgtatcgtaaacgcagttttaatagaagtgataagcaacgtcgagaatatgcacaagcaatggaagaacttgaacaaacatttgaaaatcttgaaggttggaatttatcaagcatgaaagatagtgcttataaagattatgataaatatgaagttcgactttcaaatcattcagctgataatcaatatcataacttacaagatggtaaattaatcatcaatatcaaagctagtaaaatgaattttgtttggattatagaaaataaacttgatgcaattcttgaaaaagtaaataagttagaccttagcaaatacagatttattaatgctacaagtttagatcatgatatcaaatgttattacaaaaattataaaacaaagaaagatgtaatttaa

SEQ ID NO: 20 - protein, 140 aa, Streptococcus mutans
MAFGKRRYNSYRKRSFNRSDKQRREYAQAMEELEQTFENLEGWNLSSMKDSAYKDYDKYEVRLSNHSADNQYHNLQDGKLIINIKASKMNFVWIIENKLDAILEKVNKLDLSKYRFINATSLDHDIKCYYKNYKTKKDVI

SEQ ID NO: 21 - DNA, 423 bp, Streptococcus mutans
atggcatttggaacaagaagatataattcatatcgtaaacgcagttttaatagaagtgataagcaacgtcgagaatatgcacaagcaatggaagaacttgaacaaacatttgaaaatcttgaagattggaatttgtcgagcatgaaagatagtgcttataaagattatgataaatatgaagttcgactttcaaatcattcagctgataatcaatatcataacttacaagatggtaaattaatcatcaatatcaaagctagtaaaatgaattttgtttggattatagaaaataaacttgatgcaattcttgaaaaagtaaataagttagaccttagcagatacagatttattaatgctacaaatttagaacatgatatcaaatgttattacaaaaattataaaacaaagaaagatgtaatttaa

SEQ ID NO: 22 - protein, 140 aa, Streptococcus mutans
MAFGTRRYNSYRKRSFNRSDKQRREYAQAMEELEQTFENLEDWNLSSMKDSAYKDYDKYEVRLSNHSADNQYHNLQDGKLIINIKASKMNFVWIIENKLDAILEKVNKLDLSRYRFINATNLEHDIKCYYKNYKTKKDVI

SEQ ID NO: 23 - DNA, 423 bp, Streptococcus mutans
atggcatttggaacaagaagatataattcatatcgtaaacgcagttttaatagaagtgataagcaacgtcgagaatatgcacaagcaatggaagaacttgaacaaacatttgaaaatcttgaagattggaatttgtcgagcatgaaagatagtgcttataaagattatgataaatatgaagttagactttcaaatcattcagctgataatcaatatcataacttacaagatggtaaattaatcatcaatatcaaagctagtaaaatgaattttgtttggattatagaaaataaacttgatgtaattcttgaaaaagtaaataagttagaccttagcaaatacagatttattaatgctacaagtttagatcatgatatcaaatgttattacaaaaattataaaacaaagaaagatgtaatctaa

SEQ ID NO: 24 - protein, 140 aa, Streptococcus mutans
MAFGTRRYNSYRKRSFNRSDKQRREYAQAMEELEQTFENLEDWNLSSMKDSAYKDYDKYEVRLSNHSADNQYHNLQDGKLIINIKASKMNFVWIIENKLDVILEKVNKLDLSKYRFINATSLDHDIKCYYKNYKTKKDVI

SEQ ID NO: 25 - DNA, 423 bp, Streptococcus mutans
atggcatttggaacaagaagatataattcatatcgtaaacgcaattttaatagaagtgataaacaacgtcgagaatatgcacaagcaatggaagaacttgaacaaacatttgaaaatcttgaagattggaatttgtcgagcatgaaagatagtgcttataaagattatgataaatttgaagttcgactttcaaatcattcagctgataatcaatatcataacttacaagatggtaaattaatcatcaatatcaaagctagtaaaatgaattttgtttggattatagaaaataaacttgatgcaattcttgaaaaggtaaataagttagaccttagcaaatacagatttattaatgctacaagtttagatcatgatatcaaatgttattacaaaaattataaaacaaaaaaagatgtaatttaa

SEQ ID NO: 26 - protein, 140 aa, Streptococcus mutans
MAFGTRRYNSYRKRNFNRSDKQRREYAQAMEELEQTFENLEDWNLSSMKDSAYKDYDKFEVRLSNHSADNQYHNLQDGKLIINIKASKMNFVWIIENKLDAILEKVNKLDLSKYRFINATSLDHDIKCYYKNYKTKKDVI

SEQ ID NO: 27 - DNA, 552 bp, Bacteriophage D1811
atgaaaataaatgacgacatcaaagagttaattttagaatatatgagccgttacttcaaattcgagaacgacttttataaactgccaggcatcaagttcactgatgcaaattggcagaagttcaaaaatggaggcactgacattgagaagatgggggcggcacgagtaaacgccatgctcgactgcctattcgacgatttcgagcttgctatgattggcaaggctcaaactaattattacaatgataattcactaaagatgaacatgccattttacacttactatgacatgttcaaaaagcagcaacttctaaaatggcttaaaaataaccgtgatgatgtcatcggcggaactggtaggatgtacacagcaagtggtaattacattgctaacgcttatttagaggtggcattagaatcgagctcgcttggtagtggctcttacatgcttcaaatgaggtttaaagactattcaaaaggtcaagaacctattccgtcaggtcgtcagaatcgacttgaatggattgaaaacaatctcgaaaacattcgataa

SEQ ID NO: 28 - protein, 183 aa, Bacteriophage D1811
MKINDDIKELILEYMSRYFKFENDFYKLPGIKFTDANWQKFKNGGTDIEKMGAARVNAMLDCLFDDFELAMIGKAQTNYYNDNSLKMNMPFYTYYDMFKKQQLLKWLKNNRDDVIGGTGRMYTASGNYIANAYLEVALESSSLGSGSYMLQMRFKDYSKGQEPIPSGRQNRLEWIENNLENIR

SEQ ID NO: 29 - DNA, 552 bp, Bacteriophage D1024
atgaaaataaatgacgacatcaaagagttaattttagaatatatgagccgttacttcaaattcgagaacgacttttataaactgccaggcatcaagttcactgatgcaaattggcagaagttcaaaaatggaggcactgacattgagaagatgggggcggcacgagtaaatgccatgctttcctgcctattcgaggattttgagcttgcaatgattggcaaggctcaaactaattattacattgataactcacttaaattgaacatgccattttacgcttactatgacatgttcaaaaagcaacttcttataaattggcttaaaaataaccgtgatgatgtcatctgcggaactggtaggatgtacacagcaagtggtaattacattgctaacgcttatttagaggtggcattagaatctagccgtctgggtggtggtgagtacatgttgcaaatgcgttttaaaaattattcaagaagtcaagaacctattccgtctggtcgtcagaatcgacttgaatggattgaaaacaatcttgaaaacattcgataa

SEQ ID NO: 30 - protein, 183 aa, Bacteriophage D1024
MKINDDIKELILEYMSRYFKFENDFYKLPGIKFTDANWQKFKNGGTDIEKMGAARVNAMLSCLFEDFELAMIGKAQTNYYIDNSLKLNMPFYAYYDMFKKQLLINWLKNNRDDVICGTGRMYTASGNYIANAYLEVALESSRLGGGEYMLQMRFKNYSRSQEPIPSGRQNRLEWIENNLENIR

SEQ ID NO: 31 - DNA, 552 bp, Bacteriophage D4530
atgaaaatcaataatgacatcaaagagctaattttggaatatgtaagtcgctattttaaatttgaaaacgacttctacaaattgccaggcatcaaattcactgatgcaaattggcaaaaattcaagaatggagatacttccatcgagaagatgggggcagcacgagtaaatgccatgcttgactgcctgttcgaagattttgagcttgcaatgattggcaaggctcaaactaattattacaatgataattcactaaagatgaacatgccattttacacttactatgacatgttcaaaaagcagcaacttctaaaatggcttaaaaataaccgtgatgatgtcatctgcggaactggtaggatgtacacagcaagtggtaattacattgctaacgcttatttagaaattgcgttagaatctagccgtctgggtagtggctcttacatgcttcaaatgagattcaaagactattcaagaagtcaagaacctattccgtctggtcgccaaaatagactagaatggattgagagcaacttggaaaacattcgataa

SEQ ID NO: 32 - protein, 183 aa, Bacteriophage D4530
MKINNDIKELILEYVSRYFKFENDFYKLPGIKFTDANWQKFKNGDTSIEKMGAARVNAMLDCLFEDFELAMIGKAQTNYYNDNSLKMNMPFYTYYDMFKKQQLLKWLKNNRDDVICGTGRMYTASGNYIANAYLEIALESSRLGSGSYMLQMRFKDYSRSQEPIPSGRQNRLEWIESNLENIR

SEQ ID NO: 33 - DNA, 552 bp, Bacteriophage D2759
atgaaaatcaataatgacatcaaagagctaattttggaatatgtaagtcgctattttaaatttgaaaacgacttctacaaattgccaggcatcaaattcactgatgcaaattggcaaaaattcaagaatggagatacttccatcgagaagatgggggcagcacgagtaaatgccatgcttgactgcctattcgacgattttgagcttgctttgattggcaaggctcaaactaattattacattgataactcacttaaattgaacatgccattttacgcttactatgacatgttcaaaaagcagcaacttctaaaatggcttaaaaataaccgtgatgatgtcatctgcggaactggtaggatgtacacagcaagtggtaattacattgctaactcttatttagaggtagcgttagaatctagccgtctgggtagtggctcttacatgcttcaaatgagattcaaagactattcaagaagtcaagaacctattccatctggtcgccaaaatagactagaatggattgagagcaacttggaaaacattcgataa

SEQ ID NO: 34 - protein, 183 aa, Bacteriophage D2759
MKINNDIKELILEYVSRYFKFENDFYKLPGIKFTDANWQKFKNGDTSIEKMGAARVNAMLDCLFDDFELALIGKAQTNYYIDNSLKLNMPFYAYYDMFKKQQLLKWLKNNRDDVICGTGRMYTASGNYIANSYLEVALESSRLGSGSYMLQMRFKDYSRSQEPIPSGRQNRLEWIESNLENIR

SEQ ID NO: 35 - DNA, 552 bp, Bacteriophage D1297
atgaaaatcaataatgacatcaaagagctaattttggaatatgtaagtcgctattttaaatttgaaaacgacttctacaaattgcaaggcatcaaattcactgatgcaaattggcaaaaattcaagaatggagatacttccatcgagaagatgggggcagcacgagtaaatgccatgcttgactgcctattcgacgattttgagcttgctttgattggcaaggctcaacaagaatactattcggataattccttgaaattgaacatgccattttacgcttactatgacatgttcaaaaagcagcaacttctaaaatggcttaaaaataaccgtgatgatgtcatctgcggaactggtaggatgtacacagcaagtggtaattacattgctaactcttatttagaggtagcgttagaatctagccgtctgggtagtggctcttacatgcttcaaatgagattcaaagactattcaagaagtcaagaacctattccgtcaggtcgcaaaaaccgacttgagtggattgaaaacaatctggaaaatattcgataa

SEQ ID NO: 36 - protein, 183 aa, Bacteriophage D1297
MKINNDIKELILEYVSRYFKFENDFYKLQGIKFTDANWQKFKNGDTSIEKMGAARVNAMLDCLFDDFELALIGKAQQEYYSDNSLKLNMPFYAYYDMFKKQQLLKWLKNNRDDVICGTGRMYTASGNYIANSYLEVALESSRLGSGSYMLQMRFKDYSRSQEPIPSGRKNRLEWIENNLENIR

SEQ ID NO: 37 - DNA, 552 bp, Bacteriophage M5728
atgaaaatcaataatgacatcaaagagctaattttggaatatgtaagtcgctattttaaatttgaaaacgacttctacaaattgccaggcatcaaattcactgatgcaaattggcaaaaattcaagaatggagatacttccatcgagaagatgggggcagcacgagtaaatgccatgcttgactgcctattcgacgattttgagcttgcttttattggcaaggctcaacaagaatactattcggataattccttgaaattgaacatgccattttacgcttactatgacatgttcaaaaagcagcaacttctaaaatggcttaaaaataaccgtgatgatgtcatctgcggaactggtaggatgtacacagcaagtggtaattacattgctaactcttatttagaggtagcgttagaatctagccgtctgggtagtggctcttacatgcttcaaatgagattcaaagactattcaagaagtcaagaacctattccatctggtcgccaaaatagactagaatggattgaaaacaatcttgagaatattcgataa

SEQ ID NO: 38 - protein, 183 aa, Bacteriophage M5728
MKINNDIKELILEYVSRYFKFENDFYKLPGIKFTDANWQKFKNGDTSIEKMGAARVNAMLDCLFDDFELAFIGKAQQEYYSDNSLKLNMPFYAYYDMFKKQQLLKWLKNNRDDVICGTGRMYTASGNYIANSYLEVALESSRLGSGSYMLQMRFKDYSRSQEPIPSGRQNRLEWIENNLENIR

SEQ ID NO: 39 - DNA, 552 bp, Bacteriophage D4419
atgaaaatcaataatgacatcaaagagctaattttggaatatgtaagtcgctattttaaatttgaaaacgacttctacaaattgccaggcatcaaattcactgatgcaaattggcaaaaattcaagaatggagatacttccatcgagaagatgggggcagcacgagtaaatgccatgcttgactgcctattcgacgattttgagcttgctttgattggcaaggctcaacaagaatactattcggataattccttgaaattgaacatgccattttacgcttactatgacatgttcaaaaagcagcaacttctaaaatggcttaaaaataaccgtgatgatgtcatctgcggaactggtaggatgtacacagcaagtggtaattacattgctaactcttatttagaggtagcgttagaatctagccgtctgggtagtggctcttacatgcttcaaatgagattcaaagactattcaagaagtcaagaacctattccatctggtcgccaaaatagactagaatggattgagagcaacttggaaaacattcgataa

SEQ ID NO: 40 - protein, 183 aa, Bacteriophage D4419
MKINNDIKELILEYVSRYFKFENDFYKLPGIKFTDANWQKFKNGDTSIEKMGAARVNAMLDCLFDDFELALIGKAQQEYYSDNSLKLNMPFYAYYDMFKKQQLLKWLKNNRDDVICGTGRMYTASGNYIANSYLEVALESSRLGSGSYMLQMRFKDYSRSQEPIPSGRQNRLEWIESNLENIR

SEQ ID NO: 41 - DNA, 552 bp, Bacteriophage D5891
atgaaaatcaataatgacatcaaagagctaattttggaatatgtaagtcgctattttaaatttgaaaacgacttctacaaattgccaggcatcaaattcactgatgcaaattggcaaaaattcaagaatggagatacttccatcgagaagatgggggcagcacgagtaaatgccatgcttgactgcctattcgacgattttgagcttgcttttattggcaaggctcaacaagaatactattcggataattccttgaaattgaacatgccattttacgcttactatgacatgttcaaaaagcagcaacttctaaaatggcttaaaaataaccgtgatgatgtcatctgcggaactggtaggatgtacacagcaagtggtaattacattgctaactcttatttagaggtagcgttagaatctagccgtctgggtagtggctcttacatgcttcaaatgagattcaaagactattcaagaagtcaagaacctattccatctggtcgccaaaatagactagaatggattgagagcaacttggaaaacattcgataa

SEQ ID NO: 42 - protein, 183 aa, Bacteriophage D5891
MKINNDIKELILEYVSRYFKFENDFYKLPGIKFTDANWQKFKNGDTSIEKMGAARVNAMLDCLFDDFELAFIGKAQQEYYSDNSLKLNMPFYAYYDMFKKQQLLKWLKNNRDDVICGTGRMYTASGNYIANSYLEVALESSRLGSGSYMLQMRFKDYSRSQEPIPSGRQNRLEWIESNLENIR

SEQ ID NO: 43 - DNA, 552 bp, Bacteriophage ALQ13.2
atgaaaatcaataatgacatcaaagagctaattttggaatatgtaagtcgctattttaaatttgaaaacgacttctacaaattgccaggcatcaaattcactgatgcaaattggcaaaaattcaagaacggagatacttccatcgagaagatgggggcagcacgagtaaatgccatgcttgactgcctattcgacgattttgagcttgctttgattggcaaggctcaacaagaatactattcggataattccttgaaattgaacatgccattttacgcttactatgacatgttaaaaaagcagcaacttctaaaatggcttaaaaataaccgtgatgatgtcatctgcggaactggtaggatgtacacagcaagtggtaattacattgctaactcttatttagaggtagcgttagaatctagccgtctgggtagtggctcttacatgcttcaaatgagattcaaagactattcaagaagtcaagaacctattccatctggtcgccaaaatagactagaatggattgagagcaacttggaaaacattcgatga

SEQ ID NO: 44 - protein, 183 aa, Bacteriophage ALQ13.2
MKINNDIKELILEYVSRYFKFENDFYKLPGIKFTDANWQKFKNGDTSIEKMGAARVNAMLDCLFDDFELALIGKAQQEYYSDNSLKLNMPFYAYYDMLKKQQLLKWLKNNRDDVICGTGRMYTASGNYIANSYLEVALESSRLGSGSYMLQMRFKDYSRSQEPIPSGRQNRLEWIESNLENIR

SEQ ID NO: 45 - DNA, 552 bp, Bacteriophage D802
atgaaaatcaataatgacatcaaagagctaattttggaatatgtaagtcgctattttaaattcgagaacgacttttacagattgcctggcatcaaattcactgatgccaactggcaaaaattcaagaatggaggcactgccattgagaagatgggagcagcacgagttaatgccatgctttcctgcctattcgaggattttgagcttgcaatgattggcaaggctcaatatgaatactattcggataattccttgaaattgaacatgccattttacgcttactatgacatgttcaaaaagcagcaacttctaaaatggcttaaaaataaccgtgatgatgtcatcggcggaactggtagaatgtacacgtcaagcggtagttacattgctaacgcttatttagaaattgcgttagaatctagccgtctgggtagtggctcttacatgcttcaaatgagattcaaagactattcaagaagtcaagaacctattccgtctggtcgccaaaatagacttgaatggattgagagcaacttggaaaacattcgataa

SEQ ID NO: 46 - protein, 183 aa, Bacteriophage D802
MKINNDIKELILEYVSRYFKFENDFYRLPGIKFTDANWQKFKNGGTAIEKMGAARVNAMLSCLFEDFELAMIGKAQYEYYSDNSLKLNMPFYAYYDMFKKQQLLKWLKNNRDDVIGGTGRMYTSSGSYIANAYLEIALESSRLGSGSYMLQMRFKDYSRSQEPIPSGRQNRLEWIESNLENIR

SEQ ID NO: 47 - DNA, 552 bp, Bacteriophage 73
atgaaaatcaataatgacatcaaagagctaattttggaatatgtaagtcgctattttaaatttgaaaacgacttctacaaattacctggcatcaaattcactgatgccaactggcaaaaattcaagaatggagatacttccatcgagaagatgggggcagcacgagtaaatgccatgcttgactgcctattcgaggattttgagcttgcaatgattggcaaggctcaaactaattattacattgataactcacttaaattgaacatgccattttacgcttactatgacatgttcaaaaagcagcaacttctaaaatggcttaaaaataaccgtgatgatgtcatcggcggaactggtaggatgtacacagcaagtggtaattacattgctaacgcttatttagaggtggcattagaatcgagctcgcttggtagtggctcttacatgcttcaaatgaggtttaaagactattcaaaaggtcaagaacctattccgtcaggtcgtcagaatcgacttgaatggattgaaaacaatctcgaaaacattcgataa

SEQ ID NO: 48 - protein, 183 aa, Bacteriophage 73
MKINNDIKELILEYVSRYFKFENDFYKLPGIKFTDANWQKFKNGDTSIEKMGAARVNAMLDCLFEDFELAMIGKAQTNYYIDNSLKLNMPFYAYYDMFKKQQLLKWLKNNRDDVIGGTGRMYTASGNYIANAYLEVALESSSLGSGSYMLQMRFKDYSKGQEPIPSGRQNRLEWIENNLENIR

SEQ ID NO: 49 - DNA, 552 bp, Bacteriophage DT1
atgaaaatcaataatgacatcaaagagctaattttggaatatgtaagtcgctattttaaatttgaaaacgacttctacaaattacctggcatcaaattcactgatgccaactggcaaaaattcaagaatggagaaacttcaatcgaaaaaatgggagcagcacgagttaatgccatgctttcatgcctattcgaggattttgagcttgcaatgattggcaaggctcaaactaattattacattgataactcacttaaattgaacatgccattttacgcttactatgacatgttcaaaaagcaacttcttataaattggcttaaaaataaccgtgatgatgtcatcggcggaactggtaggatgtacacagcaagtggtaattacattgctaacgcttatttagaggtggcattagaatcaagctcgcttggtagtggctcttacatgatccaaatgaggtttaaagactattcaaaaggtcaagaacctattccgtcaggtcgcaaaaaccgacttgagtggattgaaaacaatctggaaaatattcgataa

SEQ ID NO: 50 - protein, 183 aa, Bacteriophage DT1
MKINNDIKELILEYVSRYFKFENDFYKLPGIKFTDANWQKFKNGETSIEKMGAARVNAMLSCLFEDFELAMIGKAQTNYYIDNSLKLNMPFYAYYDMFKKQLLINWLKNNRDDVIGGTGRMYTASGNYIANAYLEVALESSSLGSGSYMIQMRFKDYSKGQEPIPSGRKNRLEWIENNLENIR

SEQ ID NO: 51 - DNA, 552 bp, Bacteriophage D1427
atgaaaatcaataatgacatcaaagagctaattttggaatatgtaagtcgctattttaaatttgaaaacgacttctacaaattacctggcatcaaattcactgatgccaactggcaaaaattcaagaatggagaaacttcaatcgaaaaaatgggagcagcacgagttaatgccatgctttcatgcctattcgaggattttgagcttgcaatgattggcaaggctcaaactaattattacattgataactcacttaaattgaacatgccattttacgcttactatgacatgttcaaaaagcaacttcttataaattggcttaaaaataaccgtgatgatgtcatcggcggaactggtaggatgtacacagcaagtggtaattacattgctaacgcttatttagaggtggcattagaatcaagctcgcttggtagtggctcttacatgatccaaatgaggtttaaagactattcaaaaggtcaagaacctattccgtcaggtcgccaaaatagactagaatggattgagagcaacttggaaaacattcgataa

SEQ ID NO: 52 - protein, 183 aa, Bacteriophage D1427
MKINNDIKELILEYVSRYFKFENDFYKLPGIKFTDANWQKFKNGETSIEKMGAARVNAMLSCLFEDFELAMIGKAQTNYYIDNSLKLNMPFYAYYDMFKKQLLINWLKNNRDDVIGGTGRMYTASGNYIANAYLEVALESSSLGSGSYMIQMRFKDYSKGQEPIPSGRQNRLEWIESNLENIR

SEQ ID NO: 53 - DNA, 552 bp, Bacteriophage N1162
atgaaaatcaataatgacatcaaagagctaattttggaatatgtaagtcgctattttaaatttgaaaacgacttctacaaattacctggcatcaaattcactgatgccaactggcaaaaattcaagaatggagatacttccatcgagaagatgggggcagcacgagtaaatgccatgcttgactgcctattcgaggattttgagcttgcaatgattggcaaggctcaaactaattattacattgataactcacttaaattgaacatgccattttacgcttactatgacatgttcaaaaagcagcaacttctaaaatggcttaaaaataaccgtgatgatgtcatcggcggaactggtaggatgtacacatcaaccggtaattacattgctaacgcttatttagaaattgcgttagaatctagccgtctgggtagtggctcttacatgatccaaatgaggtttaaagactattcaaaaggtcaagaacctattccgtctggtcgtcagaatcgacttgaatggattgaaaacaatctggaaaatattcgataa

SEQ ID NO: 54 - protein, 183 aa, Bacteriophage N1162
MKINNDIKELILEYVSRYFKFENDFYKLPGIKFTDANWQKFKNGDTSIEKMGAARVNAMLDCLFEDFELAMIGKAQTNYYIDNSLKLNMPFYAYYDMFKKQQLLKWLKNNRDDVIGGTGRMYTSTGNYIANAYLEIALESSRLGSGSYMIQMRFKDYSKGQEPIPSGRQNRLEWIENNLENIR

SEQ ID NO: 55 - DNA, 552 bp, Bacteriophage D1018
atgaaaatcaataatgatatcaaagagctaattttggaatatgtaagtcgctattttaaatttgaaaacgacttctacaaattgccagacatcaagttcacagatgctaattggcaaaaatttaagaatggagaaacttcaatcgaaaaaatgggagcagcacgagtaaatgccatgcttgactgcctattcgaggattttgagcttgcaatgattggcaaggctcaaactaattattacattgataactcacttaaattgaacatgccattttacgcttactatgacatgttcaaaaagcagcaacttctaaaatggcttaaaaataaccgtgatgatgtcatcggcggaactggtaggatgtacacatcaaccggtaattacattgctaacgcttatttagaaattgcgttagaatctagccgtctgggtagtggctcttacatgatccaaatgaggtttaaagactattcaaaaggtcaagaacctattccgtctggtcgtcagaatcgacttgaatggattgaaaacaatctggaaaatattcgataa

SEQ ID NO: 56 - protein, 183 aa, Bacteriophage D1018
MKINNDIKELILEYVSRYFKFENDFYKLPDIKFTDANWQKFKNGETSIEKMGAARVNAMLDCLFEDFELAMIGKAQTNYYIDNSLKLNMPFYAYYDMFKKQQLLKWLKNNRDDVIGGTGRMYTSTGNYIANAYLEIALESSRLGSGSYMIQMRFKDYSKGQEPIPSGRQNRLEWIENNLENIR

SEQ ID NO: 57 - DNA, 552 bp, Bacteriophage D3577
atgaaaataaacaacgatatcaaagagctaattttggaatacgctaaacgttatttcaagtttgaaaacgacttctacaaactgccagacatcaaattcactgatgccaactggcaaaaatttaagaatggagaaacttccatcgaaaaaatgggagcagcacgagttaatgccatgctttcctgcctgttcgacgattttgagcttgctatgattggcaaggctcaaactaattattacaatgataactcacttaaattgaacatgccattttacgcttactatgacatgttcaaaaagcagcaacttctaaaatggcttaaaaataaccgtgatgatatcatctgcggaactggtagaatgtacacttcaagaggtagttacattgctaacgcttatttagaggtagcgttagaatcaagcttgcttggtagtggctcttacatgcttcaaatgaggttcaaagactattcaaaaagtcaagaacctattccatctggtcgtcagaatcgacttgaatggattgagagcaacttggaaaatattcgataa

SEQ ID NO: 58 - protein, 183 aa, Bacteriophage D3577
MKINNDIKELILEYAKRYFKFENDFYKLPDIKFTDANWQKFKNGETSIEKMGAARVNAMLSCLFDDFELAMIGKAQTNYYNDNSLKLNMPFYAYYDMFKKQQLLKWLKNNRDDIICGTGRMYTSRGSYIANAYLEVALESSLLGSGSYMLQMRFKDYSKSQEPIPSGRQNRLEWIESNLENIR

SEQ ID NO: 59 - DNA, 552 bp, Bacteriophage CHPC577
atgaaaataaacaacgatatcaaagagctaattttggaatatggaagtcgctattttaaatttgaaaacgacttctacaaactgcctggcatcaagttcactgatgctaattggcaaaaattcaaaaatggtgatactttaatcgaaaaaatgggggcagcacgagtaaatgccatgcttgactgcctgttcgacgattttgagcttgctatgattggcaaggctcaaactaattattacaatgataattccttgaaattgaacatgccattttacgcttactatgacatgttcaaaaagcaacagcttatacattggctcaaaaacaaccgtgatgacatcgtaggcggaactggtagactgtacacttcaagcggtagttacattgctaacgcttatttagaaattgcattagaatcgagctcgcttggtagtggctcttacatgcttcaaatgagattcaaaaactattcaaaaagtcaagaacctattccatctggtcgccagaatcgacttgaatggattgaaaacaatcttgagaatattcgataa

SEQ ID NO: 60 - protein, 183 aa, Bacteriophage CHPC577
MKINNDIKELILEYGSRYFKFENDFYKLPGIKFTDANWQKFKNGDTLIEKMGAARVNAMLDCLFDDFELAMIGKAQTNYYNDNSLKLNMPFYAYYDMFKKQQLIHWLKNNRDDIVGGTGRLYTSSGSYIANAYLEIALESSSLGSGSYMLQMRFKNYSKSQEPIPSGRQNRLEWIENNLENIR

SEQ ID NO: 61 - DNA, 552 bp, Bacteriophage D4237
atgaaaataaataacgacatcaaagaattaattttagaatatatgagccgttacttcaaattcgaaaacgacttctacaaattgccagacatcaagttcacagatgctaattggcaaaaatttaagaatggagaaacttcaatcgaaaaaatgggagcagcacgagttaatgccatgctcaactgcctattcgaagattttgagcttgctatgattggcaaggctcaaattaattattacaatgataactcacttaaaatgaacatgccattttacgcttactatgatatgttcaaaaaacaacagcttctaaaatggcttaaagatcaccatgatgacatcatcggaggagctggcagaatgtacacatcaaccggtagttacattgctaatgcttatttagaggtagcgttagaatcaagctcgcttggtgatggtgagtacatgttgcaaatgcgttttaaaaattattcacgaagtcaagaacctattccgtcaggtcgcaaaaaccgacttgagtggattgaaaacaatctggaaaatattcgataa

SEQ ID NO: 62 - protein, 183 aa, Bacteriophage D4237
MKINNDIKELILEYMSRYFKFENDFYKLPDIKFTDANWQKFKNGETSIEKMGAARVNAMLNCLFEDFELAMIGKAQINYYNDNSLKMNMPFYAYYDMFKKQQLLKWLKDHHDDIIGGAGRMYTSTGSYIANAYLEVALESSSLGDGEYMLQMRFKNYSRSQEPIPSGRKNRLEWIENNLENIR

SEQ ID NO: 63 - DNA, 552 bp, Bacteriophage 9874
atgaaaataaatgacgacatcaaagaattaattttagaatatatgagccgttacttcaaattcgagaacgacttctacaaattgcctgacatcaaattcactgatgccaactggcaaaaattcaaaaatggagatacttccatcgagaagatgggggcagcacgagtaaatgccatgcttgactgcctattcgaagatttcgaacttgccatgattggcaaggctcaacaagaatactatttggataattcactaaagatgaacatgccattttacgcttattatgatatgttcaagaaaaaacagctcgtcaaatggcttaaagatcaccatgatgacatcctaggcggaactggtaggatgtacacttcagacggtagttacattgctaactcttatttagaggtagcgttagaatctagccgtctgggtagtggctcttacatgcttcaaatgagattcaaagactattcaagaagtcaagaacccattccgtcaggtcgcaaaaaccgacttgagtggattgaaaacaatctggaaaatattcgataa

SEQ ID NO: 64 - protein, 183 aa, Bacteriophage 9874
MKINDDIKELILEYMSRYFKFENDFYKLPDIKFTDANWQKFKNGDTSIEKMGAARVNAMLDCLFEDFELAMIGKAQQEYYLDNSLKMNMPFYAYYDMFKKKQLVKWLKDHHDDILGGTGRMYTSDGSYIANSYLEVALESSRLGSGSYMLQMRFKDYSRSQEPIPSGRKNRLEWIENNLENIR

SEQ ID NO: 65 - DNA, 552 bp, Bacteriophage 5093
atggaaatcaacaacgatatcaaagagttaattttggaatacgtgaaaagatacttcaagttcgagaacgacttctacaaattgcctgacatcaaattcactgatgccaactggcagaagttcaaaaatggcgaaacagccattgagaagatgggggcagcacgagtaaacgcaatgctcgactgcctattcgaagattttgagcttgccatgattggcaaggctcaaactaattattatattgataactcgcttaaattaaacatgccattttatgcttactatgatatgtttaagaaacaacagctcgtcaaatggcttgaaactagtcgtgaagacatcatcggaggggctggcagaatgtacacttcagacggtagttacattgctaacgcttatttagaagtagcgttagaatcaagctcgcttggtgatagtgaatacatgttgcaaatgcgttttaaaaattattcaaaaagtcaagaacctattccgtctggtcgtcaaaatagactggaatggattgaaaacaatcttaaaaacattcgataa

SEQ ID NO: 66 - protein, 183 aa, Bacteriophage 5093
MEINNDIKELILEYVKRYFKFENDFYKLPDIKFTDANWQKFKNGETAIEKMGAARVNAMLDCLFEDFELAMIGKAQTNYYIDNSLKLNMPFYAYYDMFKKQQLVKWLETSREDIIGGAGRMYTSDGSYIANAYLEVALESSSLGDSEYMLQMRFKNYSKSQEPIPSGRQNRLEWIENNLKNIR

SEQ ID NO: 67 - DNA, 552 bp, Bacteriophage D4154
atgctaataaataacgacatcaaagagttgattttggaatacgtcaaacgctattttaaatatgaaaatgacttctacagattgccgggcatcaagtttaccgatgcaaattggcagaagtttaaaaatggcgacacttccatcgagaagatgggggcagcacgagtaaacgccatgctcgactgcctattcgaagattttgagcttgccatgattggtaaggctcaaaccaattattatatcaataattcattgaaaatgaatatgccgttttacgcttactatgatatgttcaagaaggaacagcttatgaaatggcttgaaaccagccgtgaagacatcataggcggaactggcaggatgtacacttcagacggtagttacattgctaacgcttatttggaaattgcattagaatcgagctcgcttggtagtggctcttacatgcttcaaatgcgttttaaagattattcaaaaggtcaagagcctatcccgtctggtcgtcaaaaccgacttgagtggattgaaaacaatcttgaaaacattcgataa

SEQ ID NO: 68 - protein, 183 aa, Bacteriophage D4154
MLINNDIKELILEYVKRYFKYENDFYRLPGIKFTDANWQKFKNGDTSIEKMGAARVNAMLDCLFEDFELAMIGKAQTNYYINNSLKMNMPFYAYYDMFKKEQLMKWLETSREDIIGGTGRMYTSDGSYIANAYLEIALESSSLGSGSYMLQMRFKDYSKGQEPIPSGRQNRLEWIENNLENIR

SEQ ID NO: 69 - DNA, 552 bp, Streptococcus thermophilus DGCC11758
atgctaataaataacgacatcaaagagttgattttggaatacgtcaaacgctattttaaatttgaaaatgacttctacagattgccgggcatcaagtttaccgatgcaaattggcagaagtttaaaaatggcgacactgccattgagaagatgggggcatcacgagtaaactctatgcttgactgcctgttcgaagattttgagcttgctatgattggcaaggctcaagatgaatactatttggataattcactaaagatgaacatgccattttacgcttattatgatatgttcaagaaaaaacagctcgtcaaatggcttaaagatcaccatgatgacatcctaggcggaactggtaggatgtatacttcaagcggcaattacattgctaacgcttatttagaggtagcgttagaatcaagctcgcttggtagtggctcttacatgattcaaatgcgttttaaaaattattcaaaaggtcaagagcctatcccgtctggtcgtcaaaaccgacttgagtggattgaaaaaaacttggagaacattcgataa

SEQ ID NO: 70 - protein, 183 aa, Streptococcus thermophilus DGCC11758
MLINNDIKELILEYVKRYFKFENDFYRLPGIKFTDANWQKFKNGDTAIEKMGASRVNSMLDCLFEDFELAMIGKAQDEYYLDNSLKMNMPFYAYYDMFKKKQLVKWLKDHHDDILGGTGRMYTSSGNYIANAYLEVALESSSLGSGSYMIQMRFKNYSKGQEPIPSGRQNRLEWIEKNLENIR

SEQ ID NO: 71 - DNA, 552 bp, Streptococcus thermophilus DSM 20617
atggaaatcaacaacgatattaaacaactgatcttggaatacgctaaacgttatttcaagtttgagaacgacttttataaactgccaggcatcaagttcactgatgcaaattggcagaagttcaaaaatggaggcactgccattgagaagatgggggcagcacgagtaaacgccatgctcgactgcctattcgaagatttcgagcttgcaatgattggcaaggctcaacaagaatactattcggataattccttgaaagtaaatatggcattctatgcttattacgatcaattcaaaaaacaacagcttatgaaatggcttaaagataatcacgatgacatcataggagggactggtagaatgtacacgtcaagcggtagttacattgctaacgcttatttagaaattgcgttagaatctagccgtctgggtggtggttcttacatgatccaaatgaggtttaaagactattcaaaaggtcaagaacctattccgtctggtcgtcagaatcgacttgaatggattgagagcaacttggaaaacattcgataa

SEQ ID NO: 72 - protein, 183 aa, Streptococcus thermophilus DSM 20617
MEINNDIKQLILEYAKRYFKFENDFYKLPGIKFTDANWQKFKNGGTAIEKMGAARVNAMLDCLFEDFELAMIGKAQQEYYSDNSLKVNMAFYAYYDQFKKQQLMKWLKDNHDDIIGGTGRMYTSSGSYIANAYLEIALESSRLGGGSYMIQMRFKDYSKGQEPIPSGRQNRLEWIESNLENIR

SEQ ID NO: 73 - DNA, 552 bp, Bacteriophage Sfi19
atggaaatcaacaacgacattaaacaactgatcttggaatacgtgggacgctattttaaatttgaaaatgacttctacaaattgcccggcatcaaattcactgatgccaattggcagaagttcaaaaatggcgatacttccatcgaaaagatgggagcagcacgagtaaacgcaatgcttgactgcctgttcgaagatttcgaacttgccatgattggcaaggctcaaactaattattatattgataattcccttaaattaaacatgccattttacgcttattatgatatgttcaagaaggaacagcttatgaaatggcttaaagatcaccatgatgacatcataggcggaactggtaggatgtacatttcaagcggtagctacattgctaacgcttatttggaaattgcactagaatcaagtacgcttggtggtggtgagtacatgttgcaaatgcgctttaaaaattattcacgaagccaagaacctattccatcaggtcgcaaaaatagacttgaatggattgaaaacaatcttgaaaacattcgataa

SEQ ID NO: 74 - protein, 183 aa, Bacteriophage Sfi19
MEINNDIKQLILEYVGRYFKFENDFYKLPGIKFTDANWQKFKNGDTSIEKMGAARVNAMLDCLFEDFELAMIGKAQTNYYIDNSLKLNMPFYAYYDMFKKEQLMKWLKDHHDDIIGGTGRMYISSGSYIANAYLEIALESSTLGGGEYMLQMRFKNYSRSQEPIPSGRKNRLEWIENNLENIR

SEQ ID NO: 75 - DNA, 552 bp, Bacteriophage Sfi11
atggaaatcaacaacgacattaaacaactgatcttggaatacgtgggacgctattttaaatttgaaaatgacttctacaaattgcccggcatcaaattcactgatgccaattggcagaagttcaaaaatggcgatacttccatcgaaaagatgggagcagcacgagtaaacgcaatgcttgactgcctgttcgaagatttcgaacttgccatgattggcaaggctcaaactaattattatattgataattcccttaaattaaacatgccattttacgcttattatgatatgttcaagaaggaacagcttatgaaatggcttaaagatcaccatgatgacatcataggcggaactggtaggatgtacacttcaagcggtagctacattgctaacgcttatttggaaattgcactagaatcaagtacgcttggtggtggtgagtacatgttgcaaatgcgctttaaaaattattcacgaagccaagaacctattccatcaggtcgcaaaaatagacttgaatggattgaaaacaatcttgaaaacattcgataa

SEQ ID NO: 76 - protein, 183 aa, Bacteriophage Sfi11
MEINNDIKQLILEYVGRYFKFENDFYKLPGIKFTDANWQKFKNGDTSIEKMGAARVNAMLDCLFEDFELAMIGKAQTNYYIDNSLKLNMPFYAYYDMFKKEQLMKWLKDHHDDIIGGTGRMYTSSGSYIANAYLEIALESSTLGGGEYMLQMRFKNYSRSQEPIPSGRKNRLEWIENNLENIR

SEQ ID NO: 77 - DNA, 552 bp, Streptococcus thermophilus M17PTZA496
atggaaatcaacaaagacatcaaagagttgattttggaatacgtcaaacgctattttaaatttgaaaatgatttctacagattgccgggcatcaagtttaccgatgccaactggcaaaaattcaagaatggagatacttccatcgagaagatgggggcagcacgagtaaacgccatgcttgactgcctgttcgaagatttcgaacttgctatgattggcaaggctcaagatgaatactatttggataattcacttaagtttaatatggcattccatacttattacgatcaatttaaaaaacaacagcttatgaaatggcttgaaactagcctcgaagacatcataggcggaactggtaggatgtacacttcaagcggtagttacattgctaacgcttatttggaaattgcactagaatcaagctcgcttggtggtggtgagtacatgttgcaaatgcgttttaaaaattattcacgaagccaagaacctattccgtcaggtcgcaaaaaccgacttgagtggattgaaaacaatctggaaaatatccgataa

SEQ ID NO: 78 - protein, 183 aa, Streptococcus thermophilus M17PTZA496
MEINKDIKELILEYVKRYFKFENDFYRLPGIKFTDANWQKFKNGDTSIEKMGAARVNAMLDCLFEDFELAMIGKAQDEYYLDNSLKFNMAFHTYYDQFKKQQLMKWLETSLEDIIGGTGRMYTSSGSYIANAYLEIALESSSLGGGEYMLQMRFKNYSRSQEPIPSGRKNRLEWIENNLENIR

SEQ ID NO: 79 - DNA, 552 bp, Bacteriophage D4769
atgaaaatcaataatgacatcaaagagctaattttggaatatgtaagtcgctattttaaatttgaaaacgacttctacaaattacctggcatcaaattcactgatgccaactggcaaaaattcaagaatggagatacttccatcgagaagatgggggcagcacgagtaaacgccatgcttgactgcctgttcgaagatttcgaacttgctatgattggcaaggctcaagatgaatactatttggataattcacttaagtttaatatggcattccatacttattacgatcaatttaaaaaacaacagcttatgaaatggcttgaaactagcctcgaagacatcataggcggaactggtaggatgtacacttcaagcggtagttacattgctaacgcttatttggaaattgcactagaatcaagctcgcttggtggtggtgagtacatgttgcaaatgcgttttaaaaattattcacgaagccaagaacctattccgtcaggtcgcaaaaaccgacttgagtggattgaaaacaatctggaaaatatccgataa

SEQ ID NO: 80 - protein, 183 aa, Bacteriophage D4769
MKINNDIKELILEYVSRYFKFENDFYKLPGIKFTDANWQKFKNGDTSIEKMGAARVNAMLDCLFEDFELAMIGKAQDEYYLDNSLKFNMAFHTYYDQFKKQQLMKWLETSLEDIIGGTGRMYTSSGSYIANAYLEIALESSSLGGGEYMLQMRFKNYSRSQEPIPSGRKNRLEWIENNLENIR

SEQ ID NO: 81 - DNA, 552 bp, Bacteriophage D5691
atgattataaatattgatatcaaggaattgattttagagtatatgagtagatacttcaaatttgaaaatgatttctacaaactccccggcatcaaattcactgatgccaattggcaaaaatttaagaatggtgacacttccatcgaaaagatgggagcggctcgagtaaatgccatgctcgactgtctattcgatgactttgaacttgctatgattggcaaggctcaaattaattattacatagacaattcccttaaattgaacatgccattctatgcttattatgacatgttcaaaaaacaacaactgatcaaatggattgaaaccagccgtgatgatgtcatcggaggaactggcaggatgtatacagcaagcggaagctacatagctaacgcttatctagaaatagcactagaatctagctctctgggtggtggctcttatatgcttcaaatgagattcaaaaactactcacgaagccaagagccaataccatctggtcggaaaaaccgacttgagtggattgagagcaacttggaaaacattagataa

SEQ ID NO: 82 - protein, 183 aa, Bacteriophage D5691
MIINIDIKELILEYMSRYFKFENDFYKLPGIKFTDANWQKFKNGDTSIEKMGAARVNAMLDCLFDDFELAMIGKAQINYYIDNSLKLNMPFYAYYDMFKKQQLIKWIETSRDDVIGGTGRMYTASGSYIANAYLEIALESSSLGGGSYMLQMRFKNYSRSQEPIPSGRKNRLEWIESNLENIR

SEQ ID NO: 83 - DNA, 552 bp, Streptococcus sp. HMSC10E12
atggaaatcaacaatgacatcaaagagttaatcttggaatacgtgggacgctatttcaagtttgaaaatgatttttacaaattgccgggcatcaaatttaccgatgcaaattggcaaaaattcaaaaacggtgatacatccatcgagaaaatgggggcggcacgagtaaacgcaatgctcgactgcctattcgatgatttcgagcttgctatgattggcaaggctcaaactgattattacattgataactcacttaaattgaacatgccattttatgcttattatgacatgttcaaaaaacaacagcttctaaaatggattgagaatagtcgtgaagacatcatcggaggggctggcagaatgtacacagcgggcggtaattggatttctagcgcttatttagagatcgcattagaatctagttccatcggtggcggtggctatatgcttcaaatgcggttcaaaaactactcaagagaccctagaccgattccagcaggccaccaaaatcgtctcgaatggattgaaaacaacttggagaatatccgataa

SEQ ID NO: 84 - protein, 183 aa, Streptococcus sp. HMSC10E12
MEINNDIKELILEYVGRYFKFENDFYKLPGIKFTDANWQKFKNGDTSIEKMGAARVNAMLDCLFDDFELAMIGKAQTDYYIDNSLKLNMPFYAYYDMFKKQQLLKWIENSREDIIGGAGRMYTAGGNWISSAYLEIALESSSIGGGGYMLQMRFKNYSRDPRPIPAGHQNRLEWIENNLENIR

SEQ ID NO: 85 - DNA, 552 bp, Streptococcus sp. HSISS2
atggaaatcaacaatgacatcaaggacctaattttagaatacgtaggacgatattttcgatttgaaaacgacttctacaaacttcccagaatcaagtttaccgattccaattggcaaaaattcaagaacggtgacacttccatcgaaaaaatgggagctggcagagtgaacgcaatgctcgattgtctatttgatgattttgagcttgctatgattggtaaggctcaaaccgattactacatggacaattctttaaagatgaatatgccattttatgcctattatgaccaatttaagaaacagcaactattgaaatggatcgagaatagtagagaggatatcataggcggtgctggcagaatgtacacagctagtgggaattggatttctagtgcctatttagaaattgcattggaatccagctcgttaggtggtggtgagtacatgttgcaaatgcgtttcaaagactactcacgaagccaagagccgataccagcaggccgccagaatcgacttgagtggattgagaataatttggagaatattcgataa

SEQ ID NO: 86 - protein, 183 aa, Streptococcus sp. HSISS2
MEINNDIKDLILEYVGRYFRFENDFYKLPRIKFTDSNWQKFKNGDTSIEKMGAGRVNAMLDCLFDDFELAMIGKAQTDYYMDNSLKMNMPFYAYYDQFKKQQLLKWIENSREDIIGGAGRMYTASGNWISSAYLEIALESSSLGGGEYMLQMRFKDYSRSQEPIPAGRQNRLEWIENNLENIR

SEQ ID NO: 87 - DNA, 51 bp, Artificial
  primer/oligo
attacagctccagatccagtactgaattctcgctgatggtgatagcattgg

SEQ ID NO: 88 - DNA, 50 bp, Artificial
  primer/oligo
gaaaatatgcactcgagaagcttgagctcttgctttcgcagtctcgaatt

SEQ ID NO: 89 - DNA, 20 bp, Artificial
  primer/oligo
aatgtcactaacctgccccg

SEQ ID NO: 90 - DNA, 20 bp, Artificial
  primer/oligo
cattgaacatgctgaagagc

SEQ ID NO: 91 - DNA, 35 bp, Artificial
  primer/oligo
aaactccgttacaattagaacaaaattcttgtttg

SEQ ID NO: 92 - DNA, 35 bp, Artificial
  primer/oligo
aaaacaaacaagaattttgttctaattgtaacgga

SEQ ID NO: 93 - DNA, 30 bp, Artificial
  primer/oligo
gttcttagtgcatataacaaacatagagac

SEQ ID NO: 94 - DNA, 18 bp, Artificial
  primer/oligo
ccaagtagcgaagcgagc

SEQ ID NO: 95 - DNA, 52 bp, Artificial
  primer/oligo
attacagctccagatccagtactgaattcttcgctgaaaaagtttgggaagt

SEQ ID NO: 96 - DNA, 54 bp, Artificial
  primer/oligo
gaaaatatgcactcgagaagcttgagctctcctctctcttatgatagtctgcca

SEQ ID NO: 97 - DNA, 20 bp, Artificial
  primer/oligo
aatgtcactaacctgccccg

SEQ ID NO: 98 - DNA, 20 bp, Artificial
  primer/oligo
cattgaacatgctgaagagc

SEQ ID NO: 99 - DNA, 327 bp, Bacteriophage O; identical to SEQ ID NO: 1

SEQ ID NO: 100 - DNA, 423 bp, Bacteriophage Sfi; identical to SEQ ID NO: 3

SEQ ID NO: 101 - DNA, 423 bp, Bacteriophage TPL; identical to SEQ ID NO: 5

SEQ ID NO: 102 - DNA, 423 bp, Streptococcus sp; identical to SEQ ID NO: 7

SEQ ID NO: 103 - DNA, 423 bp, Bacteriophage D; identical to SEQ ID NO: 9

SEQ ID NO: 104 - DNA, 423 bp, Bacteriophage D; identical to SEQ ID NO: 11

SEQ ID NO: 105 - DNA, 423 bp, Bacteriophage D; identical to SEQ ID NO: 13

SEQ ID NO: 106 - DNA, 423 bp, Bacteriophage D; identical to SEQ ID NO: 15

SEQ ID NO: 107 - DNA, 423 bp, Bacteriophage D; identical to SEQ ID NO: 17

SEQ ID NO: 108 - DNA, 423 bp, Streptococcus mutans; identical to SEQ ID NO: 19

SEQ ID NO: 109 - DNA, 423 bp, Streptococcus mutans; identical to SEQ ID NO: 21

SEQ ID NO: 110 - DNA, 423 bp, Streptococcus mutans; identical to SEQ ID NO: 23

SEQ ID NO: 111 - DNA, 423 bp, Streptococcus mutans; identical to SEQ ID NO: 25

SEQ ID NO: 112 - DNA, 552 bp, Bacteriophage D; identical to SEQ ID NO: 27

SEQ ID NO: 113 - DNA, 552 bp, Bacteriophage D; identical to SEQ ID NO: 29

SEQ ID NO: 114 - DNA, 552 bp, Bacteriophage D; identical to SEQ ID NO: 31

SEQ ID NO: 115 - DNA, 552 bp, Bacteriophage D; identical to SEQ ID NO: 33

SEQ ID NO: 116 - DNA, 552 bp, Bacteriophage D; identical to SEQ ID NO: 35

SEQ ID NO: 117 - DNA, 552 bp, Bacteriophage M; identical to SEQ ID NO: 37

SEQ ID NO: 118 - DNA, 552 bp, Bacteriophage D; identical to SEQ ID NO: 39

SEQ ID NO: 119 - DNA, 552 bp, Bacteriophage D; identical to SEQ ID NO: 41

SEQ ID NO: 120 - DNA, 552 bp, Bacteriophage ALQ; identical to SEQ ID NO: 43

SEQ ID NO: 121 - DNA, 552 bp, Bacteriophage D; identical to SEQ ID NO: 45

SEQ ID NO: 122 - DNA, 552 bp, Bacteriophage; identical to SEQ ID NO: 47

SEQ ID NO: 123 - DNA, 552 bp, Bacteriophage DT; identical to SEQ ID NO: 49

SEQ ID NO: 124 - DNA, 552 bp, Bacteriophage D; identical to SEQ ID NO: 51

SEQ ID NO: 125 - DNA, 552 bp, Bacteriophage N; identical to SEQ ID NO: 53

SEQ ID NO: 126 - DNA, 552 bp, Bacteriophage D; identical to SEQ ID NO: 55

SEQ ID NO: 127 - DNA, 552 bp, Bacteriophage D; identical to SEQ ID NO: 57

SEQ ID NO: 128 - DNA, 552 bp, Bacteriophage CHPC; identical to SEQ ID NO: 59

SEQ ID NO: 129 - DNA, 552 bp, Bacteriophage D; identical to SEQ ID NO: 61

SEQ ID NO: 130 - DNA, 552 bp, Bacteriophage; identical to SEQ ID NO: 63

SEQ ID NO: 131 - DNA, 552 bp, Bacteriophage; identical to SEQ ID NO: 65

SEQ ID NO: 132 - DNA, 552 bp, Bacteriophage D; identical to SEQ ID NO: 67

SEQ ID NO: 133 - DNA, 552 bp, Streptococcus thermophilus; identical to SEQ ID NO: 69

SEQ ID NO: 134 - DNA, 552 bp, Streptococcus thermophilus; identical to SEQ ID NO: 71

SEQ ID NO: 135 - DNA, 552 bp, Bacteriophage Sfi; identical to SEQ ID NO: 73

SEQ ID NO: 136 - DNA, 552 bp, Bacteriophage Sfi; identical to SEQ ID NO: 75

SEQ ID NO: 137 - DNA, 552 bp, Streptococcus thermophilus; identical to SEQ ID NO: 77

SEQ ID NO: 138 - DNA, 552 bp, Bacteriophage D; identical to SEQ ID NO: 79

SEQ ID NO: 139 - DNA, 552 bp, Bacteriophage D; identical to SEQ ID NO: 81

SEQ ID NO: 140 - DNA, 552 bp, Streptococcus sp; identical to SEQ ID NO: 83

SEQ ID NO: 141 - DNA, 552 bp, Streptococcus sp; identical to SEQ ID NO: 85

SEQ ID NO: 142 - DNA, 315 bp, Bacteriophage D
atgaaaaaagctaaacaactactcaaagaaattaaaaccaataatgtatcatacgcaattatggacgaggataatgaaatttattgcaacaaggaaactaacaacatcatggatatttatgaatatgataatgaaaatggccatttctatggtgtttatagtgacgttgttggtggtaaagttgatagtagatacttatctgacgaatatattttgaaagctatcgataaattgctaaatttaggcgatcccgtgaaacgcactgaactacctgcggacgctgatttcaaacgcacattcttttttgaagaataa

SEQ ID NO: 143 - DNA, 315 bp, Bacteriophage D
atgaaaaaagctcaacaactgctcaaagaaattaaaaacactaatgtatcatacgcaattatggacgaggataatgaaatttattgcaacaaggaaactaacaacatcatggatatttatggatatgataatgaaaatggccatttctatggtgtttatagtgacgttgttggtggtaaagttgatagtagatacttatctgacgaatatattttgaaagctatcgataaattgctattcctaggcgaccctataaaacgaacagatctaccttcggacgctgatttcaaacgcacattcttttttgaagaataa

SEQ ID NO: 144 - DNA, 291 bp, Bacteriophage P
atgaaaaacagacttttgggttctcgatatactgacgcgatcaaaaacgattgcggaacagccaataaaatgtcgaatatttacaataaattgaacaaagatagtttgcgagaaatccatagtgcactatatggcctattaacagctggatacgacattagtaacatgcgaaacatcgaagatttagaaaaatatgtgaatttaaaaaaatcacgtggccaactattaaatgtttcgagcgatgatattaagctataccataaattatttgtcatcagatttgaaaaatag

SEQ ID NO: 145 - DNA, 279 bp, Bacteriophage CHPC
atgaaaaacaaactttatactgacgcaatcaaaaacgattccagaacagccagtaaaatggcgaacatttacaataaattggaaagcgatactatgcgagaaatccatagtgcactatctggcctattaacggctggatacgacattagtaacatgcgaaacatcgaagagttagaaaaatatgtgactttaaaaaaatcacgtggccaactattaaatgtctctagcgaagacattaaattgtaccataaattatttgtcatcaggtttggcaaatag

SEQ ID NO: 146 - DNA, 297 bp, Bacteriophage D
atgaaaaacagacttttgggttctcgatatactgacgcgatcaaaaacgattgcggaacagccaataaaatgtcgaatatttacaataaattgaacaaagatagtttgcgagaaattcatagtgcactatatggcctattaacagctggttacgacattagtaacatgcgaaaaatagaagagttagaaaaatatgtgaatttaaaaaaatcacgtggccaactattaaatgtttctagcaacgatattaagctataccataaattatttgtcatcagatttggaaaagagaggtaa

SEQ ID NO: 147 - DNA, 285 bp, Bacteriophage D
atgaaaaacagactatatactgacgcgatcaaaaacgattgcggaacagccaataaaatgtcgaatatttacaataaattgaacaaagatagtttgcgagaaattcatagtgcactatatggcctattaacagctggttacgacattagtaacatgcgaaaaatagaagagttagaaaaatatgtgaatttaaaaaaatcacgtggccaactattaaatgtttctagcaacgatattaagctataccataaattatttgtcatcagatttggaaaagagaggtaa

SEQ ID NO: 148 - DNA, 279 bp, Bacteriophage D
atgaaaaacaaactttatactgacgcaatcaaaaacgattccgcaacagccaataaaatggcgaatatttatagcaagctaaacaaagatagtttgcgagaaatccatagtgcactatctggcctattaacggctggatacgacattagtaacatgcaaaacatcgcagagttacaaaaatatgtgattttaaaaaaatcacgggggcaactattaaatgtctctagcaaagacattgaactgtatcataaattatttgtcatcagatttggaaaataa

SEQ ID NO: 149 - DNA, 291 bp, Bacteriophage D
atgaaaaacagacttttgggttctcgatatactgacgcgatcaaaaacgattgcggaacagccaataaaatgtcgaatatttacaataaattgaacaaagatagtttgcgagaaattcatagtgcactatatggcctattaacagctggttacgacattagtaacatgcgaaaaatagaagagttagaaaaatatgtgaatttaaaaaaatcacgtggccaactattaaatgtttctagcaacgatattaagctataccataaattatttgtcatcagatttggaaaatag

SEQ ID NO: 150 - DNA, 285 bp, Bacteriophage D
atgaaaaacagacttttgggttctcgatatactgacgcgatcaaaaacgattgcggaacagccaataaaatgtcgaatatttacaataaattgaacaaagatagtttgcgagaaattcatagtgcactatatggcctattaacagctggttacgacattagtaacatgcgaaaaatagaagagttagaaaaatatgtgaatttatcacgtggccaactattaaatgtttctagcaacgatattaagctatatcataaattatttgtcatcagatttggaaaatag

SEQ ID NO: 151 - DNA, 303 bp, Bacteriophage D
atgaaaaacagacttttgggttctcgatatactgacgcaatcaaaaacgattccggaacagccaataaaatgtctaatatttacaattcagtcataaacaaggaggggttgcgaggaatccatagtgcactatatggcctattaacagctggatacgacattagtaacatgcgaaaaatagaagagttagaaaaatatgtgaatttaaaaaaatcacgtggccaactattaaatgtttctagcagcgatattaagctataccataaattatttgtcatcagatttggaaaaaagttaaaataa

SEQ ID NO: 152 - DNA, 297 bp, Bacteriophage D
atgaaaaatggtaacaaaattttaggttatcgatacactgatgagattaaaaacgattctgcaacagagaataaaatgtctaatctttataacaaattggacaaagatagtttacgagagatccatagtgcattatacggtctattaacagctggatatgatatcagcaacatgcgaaatgtcgaagaacttgaaaaatacgtgaacgttaaaaaatctcatggaaaattattagatgttactaatagtgacattcagttatatcataaattatttgttgttcgatttgggaagtag

SEQ ID NO: 153 - DNA, 291 bp, Bacteriophage D
atgaaaaacagacttttgggttctcgatatactgacgcgatcaaaaacgattgcggaacagccaataaaatgtcgaatatttacaataaattgaacaaagatagtttgcgagaaatccatagtgcactatatggcctattaacagctggatacgacattagtaacatgcgaaacatcgaagagttagaaaaatatgtgaatttaaaaaaatcacgtggccaactattaaatgtttctagcagcgatattaagctataccataaattatttgtcatcagatttggaaaatag

SEQ ID NO: 154 - DNA, 294 bp, Bacteriophage N
atgaaaaacagacttttgggttctcgatatactgacgcaatcaaaaacgattccggaacagccaataaaatgtctaatatttacaattcagtcataaacaaggaggggttgcgaggaatccatagtgcactatatggcctattaacagctggatacgacattagtaacatgcgaaaaatagaagagttagaaaaatatgtgaatttaaaaaaatcacgtggccaactattaaatgtttctagcagcgatattaagctataccataaattatttgtcatcagatttggaaaatag

SEQ ID NO: 155 - DNA, 294 bp, Bacteriophage N
atgaaaaacagacttttgggttctcgatatactgacgcaatcaaaaacgattccggaacagccaataaaatgtctaatatttacaattcagtcataaacaaggaggggttgcgagaaatccatagtgcactatatggcctattaacagctggttacgacattagtaacatgcgaaaaatagaagagttagaaaaatatgtgaatttaaaaaaatcacgtggccaactattaaatgtgtctagcaatgatattaagctataccataaattatttgtcaccagatttggaaaataa

SEQ ID NO: 156 - DNA, 291 bp, Bacteriophage P
atgaaaaacagacttttgggttctcgatatactgacgcaatcaaaaacgattccggaacagccaataaaatgtcgaatatttacaataaattgaacaaagatagtttgcgagaaattcatagtgcactatatggcctattaacagctggttacgacattagtaacatgcgaaacatcgaagagttagaaaaatatgtgaatttaaaaaaatcacgtggccaactattaaatgttactagcaatgatattaagctataccataaattatttgtcatcagatttggaaaatag

SEQ ID NO: 157 - DNA, 291 bp, Bacteriophage P
atgaaaaacagacttttgggttctcgatatactgacgcgatcaaaaacgattgcggaacagccaataaaatgtcgaatatttacaataaattgaacaaagatagtttgcgagagatccatagtgcactatatggcctattaacagctggatacgacattagtaacatgcgaaacatcgaagagttagaaaaatatgtgaatttaaaaaaatcacgtggccaactattaaatgtttcgagcgatgatattaagctataccataaattatttgtcatcagatttggaaaatag

SEQ ID NO: 158 - DNA, 297 bp, Bacteriophage V
atgaaaaatggtaacaaaattttaggttatcgatacactgatgagattaaaaacgattctgcaacagagaataaaatgtctaatctttataacaaattggacaaagatagtttacgagagatccatagtgcattatacggtctattaacagctggatatgatatcagcaacatgcgaaatgtcgaagaacttgaaaaatacgtgaacgttaaaaaatctcatggaaaattattagatgttactaatagtgacattcagttatatcataaattatttgttgttcgatttgggaggtaa

SEQ ID NO: 159 - DNA, 387 bp, Bacteriophage D
atgacagaatggaaaacaataaactttaatgcacaaaacattgaatacgaggcggcaaaagcaatcctcattaagatgccaaacaattctgaatggcacggttacactttctggcatccgtcaaaatgtgtgcgtacattaagcaagggtaatggttatttcaaaactttcagctatacagaaaattgggagtttaccattttcaaatcaaataaaaaaggggaaagaaccattgaacaagtacttacggcaagagatatggaaaaagcatttagtgtggtgaatgaacaaattgcaagtaatgcttcaacagaaagttaccttgaaattgaagaacctaaaaaggttgataaaacagttagtattaacaatgagttaaaacgttaa

SEQ ID NO: 160 - DNA, 387 bp, Bacteriophage D
atgacagaatggaaaacgattaattttaataaacaaaacattgaacatgaaacagcgaaagctgttctcattaagatgccaaataattctgaatggtacggctataaattctggcatccgtcaaaatgtgtgcgtacattaagcaagggcaatggttatttcaaaactttcagctatacagaaaattgggagtttaccattttcaaatcaaataaaaagggggaaagaaccgctgaacaaatacttacagcagaggatatggaaatagcttttgatgttgttaacgaacaaattagcgcgaacgcttcaacagaaagttatcttgaaattgaagaacctaaaaaggttgataaaacagttagtattaacaatgagttaaaacgttaa

SEQ ID NO: 161 - DNA, 387 bp, Bacteriophage D
atgacagaatggaaaacaataaactttaatgcacaaaacattgaatacgaggcggcaaaagcaatcctcattaagatgccaaacaattctgaatggcacggttacactttctggcatccgtcaaaatgtgtgcgtacattaagcaagggtaatggttatttcaaaactttcagctatacagaaaattgggagtttaccattttcaaatcaaataaaaagggggaaagaaccgctgaacaaatacttacagcagaggatatggaaatagcttttgatgttgttaacgaacaaatcagtgtagacgcttcgacagaaagttaccttgaaatcgaagagcctaaaaaggttgataaaacagttagtattaacaatgaattaaaacgttaa

SEQ ID NO: 162 - DNA, 381 bp, Bacteriophage D
atgtggaaatcaatcaattttaacgcacaaaacatcgaacacgagacagcgaaagctgttctcattaagatgccaaataattctgaatggagtggttataaattttggcacccatctaaatgcgtccgtactctaagcaagggcaaaggctatttcaaaattttcagctatacagaaaattgggagtttaccattttcaaatcaaataaaaagggggaaagaaccgctgaacaaatacttacagcagaggatatggaaatagcttttgatgttgttaacgaacaaattagcgcgaacgcttcaacagaaagttatcttgaaattgaagaacctaaaaaggttgataaaacagttagtattaacaatgagttaaaacgttaa

SEQ ID NO: 163 - DNA, 381 bp, Bacteriophage D
atgtggaaatcaatcaattttaacgcacaaaacatcgaacacgagacagcgaaagctgttctcattaagatgccaaataattctgaatggagtggttataaattttggcacccatctaaattcgtccgtactctaagcaagggcaaaggctatttcaaaattttcagctatacagaaaattgggagtttaccattttcaaatcaaataaaaagggggaaagaaccgctgaacaaatacttacagcagaggatatggaaatagcttttgatgttgttaacgaacaaattagcgcgaacgcttcaacagaaagttatcttgaaattgaagaacctaaaaaggttgataaaacagttagtattaacaatgagttaaaacgttaa

SEQ ID NO: 164 - DNA, 381 bp, Bacteriophage D
atgtggaaatcaatcaattttaacgcacaaaacatcgaacacgagacagcgaaagctgttctcattaagatgccaaataattctgaatggagtggttataaattttggcactcatctaaatgcgtccgtactctaagcaagggcaaaggctatttccaaagtttcagctatacagaaaattgggagtttaccattttcaaatcaaataaaaaaggggaaagaaccgctgaacaaatacttacagcagaggatatggaaatagcttttgatgttgttaacgaacaaattagcgcgaacgcttcaacagaaagttatcttgaaattgaagaacctaaaaaggttgataaaacagttagtattaacaatgagttaaaacgttaa

SEQ ID NO: 165 - DNA, 387 bp, Bacteriophage D
atgacagaatggaaaacgattaattttaataaacaaaacattgaacatgaaacagtgaaagctgttctcattaagatgccaaataattctgaatggtacggctataaattctggcatccgtcaaaatgtgtgcgtacattaagcaagggcaatggttatttcaaaactttcagctatacagaaaattgggagtttaccattttcaaatcaaataaaaagggggaaagaaccgctgaacaaatacttacagcagaggatatggaaatagcttttgatgttgttaacgaacaaattagcgcgaacgcttcaacagaaagttatcttgaaattgaagaacctaaaaaggttgataaaacagttagtattaacaatgagttaaaacgttaa

SEQ ID NO: 166 - DNA, 372 bp, Bacteriophage D
atgtggaaatcaatcaaatttaacgcacagaacataaaatttgagactgcgaaagcagtattgattaaaatgccgaataagtctaggtatgctggatatatgttctggcatcctttaaaacttgtccgtgttgaaggcggaaaaggctactttatgagttttagctatacagatgattttgagtttaaggtttttaaacaaggtaaaaatcgtcaaatcaccgctgaatcaatattatcacacgaagaaattgaggaagcttttgaaattgtgaatgaacaattatcttatatggatgaatgctatctagaggttacagaacctactaaaattgataaagaggtagaggtcaaagaagaattgagaaagtaa

SEQ ID NO: 167 - DNA, 372 bp, Bacteriophage D
atgtggaaatcaatcaaatttaatgcacaaaacatcaaattcgagacagcaaaagcagtcttgattaaaatgcccaataaatctaggtatgctgggtatatgttctggcatcctgcaaaactagtccgagtggtaggtggaaaaggttactttatgagttttagctatactgatgaatttgagtttaagatatttaaacaaggaaaaaatcgtcaaattactgttgaaaaaatcttatcacccgaagaaatagaagacgcttttgaagttgtgaacgaacaattatctgatatcgatgaatgctatttagaagtgacagaaccaactaaaattaatgataaggtagaaatcagagcagaattaagaaaataa

SEQ ID NO: 168 - DNA, 372 bp, Bacteriophage D
atgtggaaatcaatcaaatttaacgcacagaacataaaattcgagactgcgaaagcagtattaattaaaatgccaaataaatctaggtatgctggatatatgttctggcatccttcaaaacttgtccgtgttgaaggcggaaaaggctactttatgagttttagctatacagatgattttgagtttaaggtttttaaacaaggtaaaaatcgtcaaatcaccgctgaatcaatattatcacacgaagaaattgaggaagcttttgaaattgtgaatgaacaattatcttatatggatgaatgctatctagaggttacagaacctactaaaattgataaagaggtagaggtcaaagaagaattgagaaagtaa

SEQ ID NO: 169 - DNA, 372 bp, Bacteriophage D
atgtggaaatcaataaaatttaatgcacaaaacgtaaaattcgagactgcgaattcagttttgattaaaatgccgaataaatctagctatgctggatatatgttctggcaccctgcgaaactagttcgtgtgttaggtggcaaaggttactttttgagttttagctatacagatgaatttgagtttaaggtttttaagcaaggaaaaaatcgtcaaatcaccgctgaagcaatcttatcacacgaagaaatggaagacgcgtttgaaattgtgaatgagcatttgtcctatacagatgaatgctatctagaagttgcagaacctactaaaatcgataaagaggtagagatcagagaagaattgagaaagtaa

SEQ ID NO: 170 - DNA, 180 bp, Bacteriophage D
atgaaagtttattataatctagcagatagcggactcttcaaagaaatcaagaaacaactagctctggacgatgcggaaaacggcgatttaattcatacaacagaagacaacgaggcttcagatgggacaaaaatcgtcgcaatctggaacgcaaacagacaaaactattttataaagtaa

SEQ ID NO: 171 - DNA, 438 bp, Bacteriophage D
atgagaaacgattttattaataaagtttatgatgaattaaatcagattattaatcattgggctaaacaaaaatatttaagtgataagatttttgaatatactaatacttttagtattaagaaggtttatggactttattgggaagttaagattttatgtaagaatgattatcgaattttgttgagattttataaaaattatgagtggtataacgattctaatattttaaatgtatctgtattagcacctgcggtggaaagagttaaaaatgaagatggaagcgttgatgtttatccaagtaaaataattaaagataaaattgaatttattgaaggtgattttgatattgatggagatgattgggtagatgaagtgttggaatatataaataaatgggtaaataaagataaagctgatgtggaggtattagataaatga

SEQ ID NO: 172 - DNA, 438 bp, Bacteriophage D
atgagaaacgattttattaataaagtttatgatgaattaaatcagattattaatcattgggctaaacaaaaatatttaagtgataagatttttgaatatactaatacttttagtattaagaaggtttatggactttattgggaagttaagattttatgtaagaatgattatcgaattttgttgagattttataaaaattatgagtggtataacgattctaatattttaaatgtatctgtattagcacctgcggtggaaagagttaaaaatgaagatggaagcgttgatgtttatccaagtaaaaaaattaaagataaaattgaatttattgaaggtgattttgatattgatggagatgattgggtagatgaagtgttggaatatataaataaatgggtaaataaagataaagctgatgtggaggtattagataaatga

SEQ ID NO: 173 - DNA, 438 bp, Bacteriophage D
atgagaaacgattttattaataaagtttatgatgaattaaatcagattattaatcattgggctaaacaaaaatatttaagtgataagatttttgaatatactaatacttttagtattaagaaggtttatggactttattgggaagttaagattttatgtaagaatgattatcgaattttgttgagattttataaaaattatgagtggtataacgattctaatattttaaatgtatctgtattagcacctgcggtggaaagagttaaaaatgaagatggaagcgttgatgtttatccaagtaaaaaaattaaagataaaattgaatttattgaaggtaattttgatattgatggagatgattgggtagatgaagtgttggaatatataaataaatgggtaaataaagataaagctgatgtggaggtattagataaatga

SEQ ID NO: 174 - DNA, 366 bp, Bacteriophage D
atgagaaacgattttattaataaagtttatgatgaattaaatcagattattaatcattgggctaaacaaaaatatttaagtgataagatttttgaatatactaatacttttagtattaagaaggtttatggactttattgggaagttaagattttatgtaagaatgattatcgaattttgttgagattttataaaaattatgagtggtataacgattctaatattttaaatgtatctgtattagcacctgcggtggaaagagttaaaaatgaagatggaagcgttgatgtttatccaagtaaaaaattaaagataaaattgaatttattgaaggtgattttgatattgatggagatgattgggtag

SEQ ID NO: 175 - DNA, 438 bp, Bacteriophage D
atgagaaacgattttattaataaagtttatgatgaattaaatcagattattaatcattgggctaaacaaaaatatttaagtgataagatttttgaatatactaatacttttagtattaagaaggtttatggactttattgggaagttaagattttatgtaagaatgattatcgaattttgttgagattttataaaaattatgagtggtataacgattctaatattttaaatgtatctgtattagcacctgcggtggaaagagttgaaaatgaagatggaagcgttgatgtttatccaagtaaaataattaaagataaaattgaatttattgaaggtgattttgatatcgatggagatgattgggtagatgaagtgttggaatatataaataaatgggtaaataaagataaagctgatgtggaggtattagataaatga

SEQ ID NO: 176 - DNA, 438 bp, Bacteriophage D
atgagaaacgattttattaataaagtttatgatgaattaaatccgattattaatcattgggctaaacaaaaatatttaagtgataagatttttgaatatactaatacttttagtattaagaaggtttatggactttattgggaagttaagattttatgtaagaatgattatcgaattttgttgagattttataaaaatcatgagtggtataatgattctaatattttaaatgtatctgtattagcacctgcggtggaaagagttaaacatgaagatggaagcgttgatgtttatccaagtaaaataattaaagataaaattgaatttattgaaggtgattttgatattgatggatatgattgggtagatgaagtgttggaatatataaataaatgggtaaataaagataaagatgatgtggaggtattagataagtga

SEQ ID NO: 177 - DNA, 438 bp, Bacteriophage O
atgagaaacgattttattaataaagtctatgatgaattaaatcagattattaatcattgggctaaacaaaaatatttaagtgataagatttttgaatatactaatacttttagtattaagaaggtttatggactctattgggaagttaagattttatgtaagaatgattatcgaattttgttgagattttataaaaattatgagtggtataatgattctaatattttaaatgtatctgtattagcacctgcggtggaaagagttaaaaatgaagatggaagcgttgatgtttatccaagtaaaataattaaagataaaattgaatttattgaaggtaattttgatattgatggagatgattgggtagatgaagtgttggaatatataaataaatgggtaaataaagataaagctgatgtggaggtattagataaatga

SEQ ID NO: 178 - DNA, 318 bp, Bacteriophage D
atgaaaaatttcaaaataagctctacttatagagctgcacgaaaacagcagaaaactgctaatcgtaaatcgttttataacgatgagggctacatgatcagcccaagtgaatgggctgatggagtcattaaggggcttataaaccctaaaaactcttggtcaaatgaccatgtgaaagggtacctccctagagtttccccacgtagccattggacaaagaatggttatagggagtaccttggtattggtaaatcaagggatatccctgaaaaagagcctgaagttatcgagatgatggatctcgagttagttccttaa

SEQ ID NO: 179 - DNA, 318 bp, Bacteriophage P
atgaaaaatttcaaaataagctctacttatagagctgcacgaaaacagcagaaaactgctaatcgtaaatcgttttataacgatgagggctacatgatcagcccaagtgaatgggttgatggagtcattaaggggcttataaaccctaaaaactcttggtcaaatgaccatgtgaaagggtacctccctagagtttccccacgtagccattggacaaagaatggttatagggagtaccttggtattggtaaatcaagggatatccctgaaaaagagcctgaagttatcgagatgatggatctcgagttagttccttaa

SEQ ID NO: 180 - DNA, 318 bp, Bacteriophage Proph
atgaaaaatttcaaaataagctctacttatagagctgcacgaaaacagcagaaaactgctaatcgtaaatcgttttataacgatgagggctacatgatcagcccaagtgaatgggctgatggagtcattaaggggcttataaaccctaaaaactcttggtcaaatgaccatgtgaaagggtacctccctagagtttccccacgtagccattggacaaagaatggttatagggagtaccttggtattggtaaatcaagggatatccctaaaaaagagcctgaagttatcgagatgatggatctcgagttagttccttaa

SEQ ID NO: 181 - DNA, 387 bp, Bacteriophage D
atgaaatatgataagtcaggaatcatgaaagaagcttggaacttatttaataatgatgacatcacttttgcagactttgaatatctcactcgtgaagaacgccaaggtaaaaaaacatttactctttgcttgaaagaagcttgggcacacgaaaaagaaattgttgacagcatcaaaaaagaccacgctgatgctgaacattcagtggaagcaaaagcttgggattgggcttgtaaaaaattaggtgtctctattgaaatggatgcttacacaaaattcgttaacgttaacgatatgaaaaaagaagcatggcctggaacaagcgtttggtcattggctatgcgtgcggttaaactacatatcaaactttttggtcaagtagcttaa

SEQ ID NO: 182 - DNA, 522 bp, Bacteriophage D
ttgaatggattaaaaacaatcttgaaaacattcgataaaaacatatattttttaaccaaaagtgttgacatacgtcaacataggagatataatatatatgtaaagttaagagaggaagtaaatgacatgaaaaaatcaacatacgacaaatcaggaattatgaaagaagcttggaatttatttaataacgatgacatcactactgcagattttgaatatctcactcgtggagaattgcaagaaggaaaaacatttgctatttgcttaaaagaagcttgggctcacgaaaaagacattgttgaaagtttaaacgaagattatgaaaatgctgaacattcagtacaagctaaagcttgggactgggcttgtaaaaaattaggtgtctctattgaagtagatgcttacacaaaattggttaacgtcaacgacatgcaaaaagaatcatggcctggaacaagcgcatggtctttggctatgcgtgcagttaaactacatatcaaacttttcggtcaagcggcttaa

SEQ ID NO: 183 - DNA, 522 bp, Bacteriophage D
ttgaatggattaaaaacaatcttgaaaacattcgataaaaacatatattttttaaccaaaagtgttgacatacgtcaacacaggagatataatatatatgtaaagttaagagaggaagtaaatgacatgaaaaaatcaacatacgacaaatcaggaattatgaaagaagcttggaatttatttaataacgatgacatcactactgcagattttgaatatcttactcgtggagaattgcaagaaggaaaaacatttgctatttgcttaaaagaagcttgggctcacgaaaaagacattgttgaaagtttaaacgaagattatgaaaatgctgaacattcagtacaagctaaagcttgggactgggcttgtaaaaaattaggtgtctctattgaagtagatgcttacacaaaattggttaacgtcaacgacatgcaaaaagaatcatggcctggaacaagcgcatggtctttggctatgcgtgcagttaaactacatatcaaacttttcggtcaagcggcttaa

SEQ ID NO: 184 - DNA, 336 bp, Bacteriophage
atgaaaaaagaagttatgacaaacgcatggaaaatcgctaaagaagcagttaagaaattcggcggcaaagctatcgaatacatcgcagaagcattgaaaatggcttgggctgccgcaaaaggcggaaacgctagcctagctaaatttcaagcagtagaatctaaaatgcgtaaagctggtaaatactcaatgattcaagttttaaatttcgctaaggaagtgaaatttaacgaagttatgcacaaagttggtgcttactacggtatcgaagtagtagctgacggagacagcattggtacttactacatcgctgaaaaagtttgggatgcagcttaa

SEQ ID NO: 185 - DNA, 336 bp, Bacteriophage P
atgaaaaaagaaattatgacaaaagcatggaaaatcgctaaagaagcagttaaaacttttggtgggaaagctatcgaatacatcgctggggctatgaaaatggcttgggctgctatcaaagataacggaactagccttgctaaattccaagctgttgaagcaaaaatgcgtaaagctggtaaatactcaatgatccaagttcttgattttgctaaagaagtacgtttcaatgaagtaatgcacaaagttggcgcttattacggaatcgaagtaattgctgatggtgatagcattggtacttactacatcgctgagaatgtttggaacgcagcataa

SEQ ID NO: 186 - DNA, 336 bp, Bacteriophage CHPC
atgaaaaaagaaattatgacaaaagcatggaaaatcgctaaaaacgcaagtacaaaattcggtggcaaagctatcgaatacattgctggagctatgaaaatggcttgggctgctatcaaagaaaacggaactagccttgctaaattccaagcagttgaagctaaaatgcgcaaagctggcaaacactcaatggtccaagttttaaattttgctaaggaagtgaaatttaacgaagttatgcataaagttggtgcttactacggaattgaagtaattgctgatggtgatagcattggtacttactacatcgctgaaaaagtttggaacgcagcataa

SEQ ID NO: 187 - DNA, 336 bp, Bacteriophage D
atgaaaaaagaaattatgacaaaagcatggaaaatcgctaaagaagcagttgaaaaattcggtggcaaagctatcgaatacatcgctggagctatgaaaatggcttgggctgctgctaaagctggaaacactagcgtcgctaaatttcaagctgttgaagataaaatgcgcaaagctggtaaatactcaatgattcaagttttaaatttcgctaatgaagtgaaatttaacgaagttatgcacaaagctggtgcgtactacggcatcgaagtaattgctgatggtgatagcattggtacttactacatcgctgaaaaagtttgggaagtagcataa

SEQ ID NO: 188 - DNA, 327 bp, Bacteriophage D
atgaaaaaagaagttatgacaaacgcgtgggaaattgctaaaaacgcttctaaaaaattcggtggtaaagctatcgaatacatcgctggagctatgaaaatggcttgggctgctgcaaaaggcggcttagctaaattccaagcagtagaatctaaaatgcgtaaagctggaaaacattcaatggtgcaagtgttgaatttcgctaaggaagtgaaatttaacgaagttatgcacaaagctggtgcttactacggtatcgaagtaatcgctgatggtgatagcattggtacttactacatttctgaaaaagtttgggaagtagcttaa

SEQ ID NO: 189 - DNA, 336 bp, Bacteriophage D
atgaaaaaagaaattatgacaaaagcatggaaaatcgctaaagaagcagttaaaactttcggtggtaaagctatcgaatacattgctggagctatgaaaatggcttgggctgctgctaaagctggaaacactagcttagctaaattccaagcagtagaatctaaaatgcgtaaagctggtaaatactcaatgattcaagttttaaatttcgctaaggaagtgaaatttaacgaagttatgcacaaagttggcgcttattacggtatcgaagtaattgctgatggtgatagcattggtacttactacatcgctgaaagcgtttgggaagtagcataa

SEQ ID NO: 190 - DNA, 336 bp, Bacteriophage D
atgaaaaaagaaattatgacaaaagcatggaaaatcgctaaagaagcagttgaaaaattcggtggcaaagctatcgaatacatcgctggagctatgaaaatggcttgggctgctgctaaagctggaaacactagcgtcgctaaatttcaagctgttgaagataaaatgcgcaaagctggtaaatactcaatgattcaagttttaaatttcgctaatgaagtgaaatttaacgaagttatgcacaaagctggtgcgtactacggaatcgaagtaattgctgatggtgatagcattggtacttactacatcgctgaaaaagtttgggaagtagcataa

SEQ ID NO: 191 - DNA, 318 bp, Bacteriophage D
atgaaaaaagaaattatgacaaaagcatggaaaatcgctaaagaagcagttaaaactttcggtggaaaagctatcgaatacattgcggaagcaatgaaaatggcttgggctgctgctaaaggcggcttagctaaattccaagcagtagaatctaaaatgcgtaaagctggaatgattcaagttttaaatttcgctaaggaagtgaaatttaacgaagttatgcacaaagttggcgcttattacggtatcgaagtaattgctgatggtgatagcattggtacttactacatcgctgaaagcgtttgggaagtagcataa

SEQ ID NO: 192 - DNA, 336 bp, Bacteriophage D
atgaaatcacaagtaatgagcctagcatggaaaatcgctaaaaacgcaagtacaaaattcggtggcaaagctatcgaatacattgctagagctatgaaaatggcttggtctgctatcaaagaaaacggaactagccttgctaaatttcaagcaattgaagctaaaattcgcaaagctggaaaacactcaatggtccaagttttaaaattcgctaaggaagtgaaatttaacgaagttatgcataaagttggtgcttactacggaattgaagtaattgctgatggtgatagcattggtacttactacatcgctgaaaaagtttgggatgcagcgtaa

SEQ ID NO: 193 - DNA, 336 bp, Bacteriophage D
atgaaaaaagaaattatgaaaaaagcatggaaaatcgctaaagaagcagttaagaaattcggtggtaaagctatcgaatacatcgcagaagcattgaaaatggcttgggctgatgctaaaggtggtaacactagcttggctaaattccaagctgttgaggaaaagatgcgtaaagctggcaaatactcaatgattcaagtgctcaactttgctaaagaagtgaaattcaacgaagtaatgcataaagttggtgcttactacggaattgaagttattgctgacggagacaaaatcggtacttactttatcgctgaaaaagtttgggatgcagcttaa

SEQ ID NO: 194 - DNA, 336 bp, Bacteriophage D
atgaaaaaagaacttatgaaagacgcttgggaaattgctaaaaacgcttctaaaaaattcggtggtaaagctatcgaatacattgctggagctatgaaaatggcttgggctgctgctaaagctggaaacactagcgtcgctaaattccaagcggtagaagctaaaatgcgcaaagctggcaaacactcaatgattcaagttctcgatttcgctaaagaagttaagttcaacgaagtgatgcacaaagttggtgcgtactacggcatcgaagtagtcgctgacggcgatagcattggtacttactacatcgctgaaaaagtttgggatgtagcttaa

SEQ ID NO: 195 - DNA, 336 bp, Bacteriophage D
atgaaaaaagaagttatgacaaacgcatggaaaatcgctaaagaagcagttaagaaattcggtggtaaagctatcgaatacatctctgaagctatgaaaatggcttgggctgctgccaagggtgaaaacactagcttagctaaattccaagctgttgaggaaaagatgcgtaaagctggcaaatactcaatgattcaagttcttgactttgctaaagaagttaaattcaacgaagtaatgcataaagttggtgcttactacggaattgaagttattgctgacggagacaacattggtacttactacattgctgaaaaagtttgggaagtagcataa

SEQ ID NO: 196 - DNA, 321 bp, Bacteriophage D
atgacaaacgcatggaaaatcgctaaagaagcagttaagaaattcggtggtaaagctatcgaatacatctctgaagctatgaaaattgcttgggctgacgctaaagaaggaaacactagcgtagctaaattccaagctgtagaagctaaaatgcgtaaagctggaaaacattcaatggtgcaagtgttgaatttcgctaaagaagtgaaattcaacgaagtaatgcacaaagttggtgcttactacggtatcgaagtaatcgctgatggtgatagcattggtacttactacatttctgaaaaagtttgggaagtagcttaa

SEQ ID NO: 197 - DNA, 336 bp, Bacteriophage D
atgaaaaaagaaattatgacaaaagcatggaaaatcgctaaagaagcagttaaaactttcggtggaaaagctatcgaatacattgcggaagcaatgaaaatggcttgggctgctgctaaaggcggaaacgctagcttagctaaattccaagcagtagaatctaaaatgcgtaaagctggtaaatactcaatgattcaagttttaaatttcgctaaggaagtgaaatttaacgaagttatgcacaaagttggcgcttattacggtattgaagtaattgctgatggtgatagcattggtacttactacatcgctgaaagcgtttgggaagtagcataa

SEQ ID NO: 198 - DNA, 327 bp, Bacteriophage D
atgaaaaaagaaattatgacaaaagcatggaaaatcgctaaagaagcagttaaaactttcggtggaaaagctatcgaatacattgcggaagcaatgaaaatggcttgggctgctgctaaaggcggcttagctaaattccaagcagtagaatctaaaatgcgtaaagctggtaaatactcaatgattcaagttttaaatttcgctaaggaagtgaaatttaacgaagttatgcacaaagttggcgcttattacggtatcgaagtaattgctgatggtgatagcattggtacttactacatcgctgaaagcgtttgggaagtagcataa

SEQ ID NO: 199 - DNA, 336 bp, Bacteriophage D
atgaagaaagagattatgaaaaaagcgtgggaaatcgctaaagaagcagttaaaaaattcggtggcaaagctatcgaatacatcgcagaagcattgaaaatggcttggtctgatgcaaagggtagtaatactagcttagctaaattccaagctgttgaggaaaagatgcgtaaagctggcaaatactcaatgattcaagttcttgactttgctaaagaagttaaattcaatgaagtaatgcacaaagaaggtgcttactatggtatcgaagtggtagctgacggagacagcattggtacttattacattgctgaaaaagtttgggaagtagcataa

SEQ ID NO: 200 - DNA, 336 bp, Bacteriophage D
atgaaaaaagaaattatgacaaaagcatgggaaattgctaaaaacgcttctaaaaaattcggtggtaaagctatcgaatacatcgctggagctatgaaaatggcttgggctgctgctaaagctggaaacactagcgtcgctaaattccaagcggtagaagctaaaatgcgcaaagctggaaaacattcaatggtccaagttttgaattttgcaaaagaagttaagttcaacgaagtaatgcacaaagttggcacttattacggcatcgaagtagtagctgacggcgatagcattggtacttactacatcgctgaaaaagtttgggatgcagcataa

SEQ ID NO: 201 - DNA, 336 bp, Bacteriophage D
atgaaaaaagaaattatgacaaaagcttgggaaattgctaaaaacgcttctaaaaaattcggtggtaaagctatcgaatacatcgctggagctatgaaaatggcttgggctgctgctaaagctggaaaaactagcgtcgctaaattccaagcggtagaagctaaaatgcgcaaagctggaaaacattcaatggtccaagttttgaattttgctaaagaagtacgtttcaacgaagtaatgcacaaagctggcgcttattacggtatcgaagtaattgctgatggtgatagcattggtacttacttcattgctgagaatgtttggaacgcagcataa

SEQ ID NO: 202 - DNA, 336 bp, Bacteriophage D
atgaaaaaagaaattatgacaaaagcatggaaaatcgctaaagaagcagttaaaactttcggtggtaaagctatcgaatacatcgcagaagcattgaaaatggcttgggctgctgccaagggtgaaaacactagcttagctaaaattcaagctgttgaggaaaagatgcgtaaatctggtaaatactcaatgatccaagttcttgattttgctaaagaagtgaaatttaacgaagtaatgcacaaagctggtgcttactacggtatcgaagttattgctgatggcgatagcattggtacttattacattgctgaaaaagtttgggaagtagcttaa

SEQ ID NO: 203 - DNA, 336 bp, Bacteriophage D
atgaaaaaagaaattatgacaaaagcatggaaaatcgctaaagaagcagttaaaactttcggtggaaaagctatcgaatacattgcggaagcaatgaaaatggcttgggctgctgctaaaggcggaaacgctagcttagctaaattccaagcagtagaatctaaaatgcgtaaagctggtaaatactcaatgattcaagttttaaatttcgctaaggaagtgaaatttaacgaagttatgcacaaagttggcgcttattacggtatcgaagtaattgctgatggtgatagcattggtacttactacatcgctgaaaacgtttggaacgcagcataa

SEQ ID NO: 204 - DNA, 336 bp, Bacteriophage D
atgaaaaaagaaattatgacaaaagcatggaaaatcgctaaagaagcagttgagaagttcggtggtaaatctatcgaatacattgcggaagcaatgaaaatggcttgggctgctgcaaaaggcggaaacgctagcttagctaaatttcaagcggtagaagctaaaatgcgcaaagctggtaaatactcaatgattcaagttttaaatttcgctaaggaagtgaaatttaacgaagttatgcacaaagctggtgcttactatggaatcgaagtggtagctgacggagacagcattggtacttattacatcgctgaaaaagtttgggaagtagcataa

SEQ ID NO: 205 - DNA, 336 bp, Bacteriophage N
atgaaaaaagaaattatgacaaaagcttgggaaattgctaaaaacgcttctaaaaaattcggtggtaaagctatcgaatacatcgctggagctatgaaaatggcttgggctgctgctaaagctggaaacactagcgtcgctaaattccaagcggtagaagctaaaatgcgcaaagctggaaaacattcaatggtccaagttttgaattttgcaaaagaagttaagttcaacgaagtaatgcacaaagttggcacttattacggcatcgaagtagtagctgacggcgatagcattggtacttactacatcgctgaaaaagtttgggatgcagcataa

SEQ ID NO: 206 - DNA, 336 bp, Bacteriophage O
atgaaatcacaagtaatgagccaagcatggaaaatcgctaaagaagcagttaagaaattcggtggtaaagctatcgaatacatctctgaagctatgaaaatggcttgggctgctgccaagggtgaaaacactagcttaactaaatttcaagctgttgaggaaaagatgcgtaaagctggcaaatactcaatgattcaagttcttgactttgctaaagaagtgaaattcaacgaagtaatgcataaagttggtgcttactacggaattgaagttattgctgacggagacagcattggtacttactttatcgctgaaaaagtttgggatgtagcttaa

SEQ ID NO: 207 - DNA, 336 bp, Bacteriophage P
atgaaaaaagaaattatgaaaaaagcatggaaaatcgctaaagaagcagttaagaagttcggcggcaaagctatcgaatacatcgcagaagcattgaaaatggcttggtctgatgcaaagggtagtaatactagcttagctaaattccaagctgttgaggaaaagatgcgtaaagctggcaaatactcaatgatccaagttcttgattttgctaaagaagtgaaatttaacgaagtaatgcacaaagctggtgcttactacggtatcgaagttattgctgatggcgatagcattggtacttattacattgctgaaaaagtttgggaagtagcttaa

SEQ ID NO: 208 - DNA, 336 bp, Bacteriophage P
atgaaaaaagaaattatgacaaaagcttgggaaattgctaaaaacgcttctaaaaaattcggtggtaaagctatcgaatacatcgctggagctatgaaaatggcttgggctgctgctaaagctggaaacactagcgtcgctaaattccaagcggtagaagctaaaatgcgcaaagctggaaaacattcaatggtccaagttttgaattttgcaaaagaagttaagttcaacgaagtaatgcacaaagttggcgcttattacggcatcgaagtagtagctgacggcgatagcattggtacttattacattgctgaaaaagtttgggaagtagcataa

SEQ ID NO: 209 - DNA, 336 bp, Bacteriophage P
atgaaaaaagaaattatgacaaacgcgtgggaaattgctaaaaacgcttctaaaaaattcggtggtaaagctatcgaatacatcgcagaagcattgaaaatggcttggtctgatgcaaagggtagtaatactagcttagctaaattccaagctgttgaggaaaagatgcgtaaagctggcaaatactcaatgattcaagttttaaatttcgctaaagaagtgaaattcaatgaagtaatgcacaaagaaggtgcttactatggtatcgaagtagtagctgacggagacagcattggtacttattacattgctgaaaaagtttgggatgcagcgtaa

SEQ ID NO: 210 - DNA, 336 bp, Bacteriophage SFi
atgaaaaaagaagttatgacaaacgcatggaaaatcgctaaagaagcagttaagaaattcggtggtaaagctatcgaatacatctctgaagctatgaaaatggcttgggctgctgccaagggtgaaaacactagcttagctaaattccaagctgttgaggaaaagatgcgtaaagctggcaaatactcaatgattcaagttcttgactttgctaaagaagttaaaatcaacgaagtaatgcataaagttggtgcttactacggaattgaagttattgctgacggagacaacattggtacttactacattgctgaaaaagtttgggaagtagcataa

SEQ ID NO: 211 - DNA, 336 bp, Bacteriophage Sfi
atgaaaaaagaagttatgacaaacgcatggaaaatcgctaaagaagcagttaagaaattcggtggtaaagctatcgaatacatctctgaaggctatgaaatggcttgggctgctgccaagggtgaaaacactagcttagctaaattccaagctgttgaggaaaagatgcgtaaagctggcaaatactcaatgattcaagttcttgactttgctaaagaagttaaattcaacgaagtaatgcataaagttggtgcttactacggaattgaagttattgctgacggagacaacattggtacttactacattgctgaaaaagtttgggaagtagcataa

SEQ ID NO: 212 - DNA, 336 bp, Bacteriophage Sfi
atgaagaaagagattatgaaaaaagcgtgggaaatcgctaaagaagcagttaaaaaattcggtggcaaagctatcgaatacatcgcagaagcattgaaaatggcttggtctgatgcaaagggtagtaatactagcttagctaaattccaagctgttgaggaaaagatgcgtaaagctggcaaatactcaatgattcaagttcttgactttgctaaagaagttaaattcaatgaagtaatgcacaaagaaggtgcttactatggtatcgaagtggtagctgacggagacagcattggtacttactacattgctgaaaaagtttgggaagtagcataa

SEQ ID NO: 213 - DNA, 333 bp, Bacteriophage Sfi
atgaaaaaaattatgacaaacgcatggaaaatcgctaaagaagcagttaagaaattcggtggtaaagctatcgaatacatctctgaagctatgaaaattgcttgggctgatgctaaagaaggaaacactagcgtagctaaattccaagctgtagaagctaaaatgcgtaaagctggaaaacattcaatggtgcaagtgttgaatttcgctaaagaagtgaaattcaacgaagtaatgcacaaagttggtgcttactacggtatcgaagtaatcgctgatggtgatagcattggtacttactacatttctgaaaaagtttgggaagtagcttaa

SEQ ID NO: 214 - DNA, 336 bp, Bacteriophage Proph
atgaaaaaagaaattatgaaaaaagcatggaaaatcgctaaagaagcagttaagaagttcggcggcaaagctatcgaatacatcgcagaagcattgaaaatggcttggtctgatgcaaagggtagtaatactagcttagctaaattccaagctgtagaagataaaatgaacaaaaccggaaaacactcaatggtccaagtcttgaattttgctaaagaagtgaatttcaaagaagtaatgcataaagttggtgcttactacggtatcgaagtagtagctgacggagacagcattggtacttactacatcgctgaaaaggtttgggatgcagcttaa

SEQ ID NO: 215 - DNA, 111 bp, Bacteriophage D
atgaaaaaagaagttatgacaaacgcgtgggaaattgctaaaaacgcttctaaaaaattcggtggtaaagctatcgaatacatcgctgaaaacgtttggaacgcagcataa

SEQ ID NO: 216 - DNA, 345 bp, Bacteriophage D
atgaaatcacaagtaatgagcctagcatggaaaatcttcaaaaacgaaaaaaacgacgtaactttttctgaagcattgaagtttgcttggaaagccgttaaacgtcaaaatatggcagatgatttctacttcttccattcttcaaatgttaaatttcaaggtgttaagaaatggtttgctgaaaaagagttccgtggacgcaacaaaaaagacttggcgttcatgtcagtaagtgcaatcagtgttaaagggttggtcgaagaaactgataaagcagttaaacttgaaatcgtgacaccttatggggtttctgctaaatggtacccaaaaagtgtaattgcttaa

SEQ ID NO: 217 - DNA, 345 bp, Bacteriophage D
atgaaatcacaagtaatgagcctagcatggaaaatcttcaaaaacgaaaaaaacgatgtaactttttctgaagcgttgaaatttgcttggaaagccgttaaacgtcaaaacatggcggatgatttttacttcttccgttcttcaaatgttaaattccaaggtgttaagaaatggtttgctgaaaaagaatttcgtggacgcaacaagaaagacttggcgtttatgtcagtaactgcaatcagtgttaaagggttgattgaagaaactgataaagcggttaagcttgaaatcgtaacaccttatggagtttctactaaatggtatccaaagagtgtaattgcttaa

SEQ ID NO: 218 - DNA, 345 bp, Bacteriophage D
atgaaatcacaagtaatgagcctagcatggaaaattttcaaaaacgaaaaaaacgacgtaactttttctgaagcattgaagtttgcttggaaagccgttaaacgtcaaaacatggcggatgatttctacttcttccgttcttcaaacgttaaattccaaggtgttaagaaatggtttgctgaaaaagaatttcgtggacgcaacaagaaagacttggcgtttatgtcagtaactgcaatcagcattaaagggttggttgaagaaactgataaagcggttaagcttgaaatcgtgacaccttatggaatttctactaaatggtatccaaagagtgtaattgcttaa

SEQ ID NO: 219 - DNA, 345 bp, Bacteriophage Proph
atgaaatcacaagtaatgagcctagcatggaaaatcttcaaaaacgaaaaaaacgatgtaactttttctgaagcgttgaaatttgcttggaaagccgttaaacgtcaaaacatggcggatgatttctacttcttccgttcttcaaacgttaaattccaaggtgttaagaaatggtttgctgaaaaagaatttcgtggacgcaacaagaaagacttggcgtttatgtcagtaactgcaatcagcgttaaagggttgatcgaagaaactgataaagcggttaagcttgaaatcgtaacaccttatggagtttctactaaatggtatccaaagagtgtaattgcttaa

SEQ ID NO: 220 - DNA, 345 bp, Bacteriophage Proph
atgaaatcacaagtaatgagcctagcatggaaaatcttcaaaaacgaaaaaaacgatgtaactttttctgaagcgttgaaatttgcttggaaagccgttaaacgtcaaaacatggcggatgatttctacttcttccgttcttcaaacgttaaattccaaggtgttaagaaatggtttgctgaaaaagaatttcgtggacgcaacaagaaagacttggcgtttatgtcagtaactgcaatcagcattaaagggttggttgaagaaactgataaagcggttaagcttgaaatcgtgacaccttatggaatttctactaaatggtatccaaagagtgtaattgcttaa

SEQ ID NO: 221 - DNA, 261 bp, Bacteriophage
gtgaaaacaatggatgcatataaagaacaatttcaagaattacaagaatacgcttttaacgttttaagagaatatcctctagacaagacagcagttaatgtgctttctgcactcgttaactcaaaaaagaaagatcgcatcgagttttttaaactaaacaaaggcgaagatgccatgaaagtttattataatctagcagatagcggaacgattgaaaaatatttagaaacatctgcatttttagattacatcaatgaataa

SEQ ID NO: 222 - DNA, 252 bp, Bacteriophage D
atggatacatataaagaacaatttcaaaaattacaagaatacgcttttaacgttttaagagaataccctctagataagacagcagttaatgtactttctgcactcgttaactcaaaaaagaaagatcgcatcgagttttttaaactaaacaaaggcgaagatgccatgaaagtttattataatctagcagatagcggaacgattgaaaaatatttagaaacatctgcatttttagaatacataaatgaataa

SEQ ID NO: 223 - DNA, 252 bp, Bacteriophage D
atggatacatataaagaacaatttcaagaattacaagaatacgcttttaacgttttaagagaatatcctctagacaagacagcagttaatgtactttctgcactcgttaactcaaaaaagaaagatcgcatcgagttttttaaactaaacaaagacgaagatgccatgaaagtttattataatctagcagatagcggaacgattgaaaaatatttagaaacatctgcatttttagaatacatcaatgaataa

SEQ ID NO: 224 - DNA, 252 bp, Bacteriophage D
atggatacatataaagaacaatttcaagaattacaagaatacgcttttaacattttaagagaatatcctctagacaagacagcagttaatgtactttctgcactcgttaactcaaaaaagaaagatcgcatcgagttttttaaactaaacaaagacgaagatgccatgaaagtttattataatctagcagatagcggaacgattgaaaaatatttagaaacatctgcatttttagaatacatcaatgaataa

SEQ ID NO: 225 - DNA, 252 bp, Bacteriophage D
atggatacatacaaagaacaatttcaaaaattacaagaatacgcttttaacgttttaagagaataccctctagataagacagcagttaatgtactttctgcactcgttaactcaaaaaagaaagatcgcatcgagttttttaaactaaacaaaggcgaagatgccatgaaagtttattataatctagcagatagcggaacgattgaaaaatatttagaaacatctgcatttttagaatacacaaatgaataa

SEQ ID NO: 226 - DNA, 252 bp, Bacteriophage Sfi
atggatacatataaagaacaatttcaagaattacaagaatacgcttttaacattttaagagaatatcctctagacaagacagcagttaatgtactttctgcactcgttaactcaaaaaagaaagatcgcatcgagttttttaaacttaacaaagacgaagatgccatgaaagtttattataatctagcagatagcggaacgattgaaaaatatttagaaacatctgcatttttagaatacatcaatgaataa

SEQ ID NO: 227 - DNA, 252 bp, Bacteriophage Proph
atggatacatacaaagaacaatttcaagaattacaagaatacgcttttaacgttttaagagaataccctctagataagacagcagttaatgtactttctgcactcgttaactcaaaaaagaaagatcgcatcgagttttttaaactaaacaaaggcgaagacgccatgaaagtttattataatctagcagatagcggaacgattgaaaaatatttagaaacatctgcattcttagaatacatcaatgaataa

SEQ ID NO: 228 - DNA, 252 bp, Bacteriophage Proph
atggatacatataaagaacaatttcaagaattacaagaatacgcttttaacgttttaagagaatatcctctagacaagacagcagttaatgtactttctgcactcgttaactcaaaaaagaaagatcgcatcgagttttttaaactaaacaaaggcgaagatgccatgaaagtttattatagtctagcagatagcggaacgattgagagatacttggaagtctgtggatttttagagtacatcaacgaataa

SEQ ID NO: 229 - DNA, 282 bp, Bacteriophage D
atgataactaaagaacaattaaaagaatactacagcgaacacttggaagagctcgtcgaatgggcagacgatataaataaaatatgcctatttgcctacctagatgaagatgataacttgtattgtgggattaatcaactgtcctacacacaattcagagttccaattcaagctgaggtgacagtggatgatgattggaactacgatttcttcaaaaatccagctgcctatgatggatgggatgaaactttggaagaaatgttggaagaattaaatgattaa

SEQ ID NO: 230 - DNA, 282 bp, Bacteriophage D; identical to SEQ ID NO: 229

SEQ ID NO: 231 - DNA, 282 bp, Bacteriophage D
atgataactaaagaacaattaaaagaatactacagcgaacacttggaagagctcgtcgaatgggcagacgatataaataaaatatgcctatttgcctacctagatgaagatgataacttgtattgtgggataaatcaactgtcctacacacaattcagagttccaattcaagctgaggtgacagtggatgatgattggaactacgatttcttcaaaaatccagctgcctatgatggatgggatgaaactttggaagaaatgttggaagaattaaatgattaa

SEQ ID NO: 232 - DNA, 141 bp, Bacteriophage D
gtgaaaacaatggatacatataaagaacaattttattatttggatcctatttatattagtgtggatattaataggaggacttttattttaggaaaaagagggcaatcgctctcttttttttattgtaataaaacaatttaa

SEQ ID NO: 233 - DNA, 225 bp, Bacteriophage O
atgacacaaattaaagatggttggcacatggtttatgacgaaaaagtgtatgtagagagcgggaaagttgtccgtggaataactaaagacaataacaattctgaaatagcttgctacccttacgaatacaacaaagactatgattgctggattaacatttctgggaaagtaactctatcagcttatagatcaggtcgtaaaaaagggacaaaatgtatgaagtga

SEQ ID NO: 234 - DNA, 225 bp, Bacteriophage Sfi
atgacacaaattaaagatggttggcacatagtttatgacgaaaaagtgtacgtagagagcgggaaagttgtccgtggaataactaaagacaataacaattctgaaatagcttgctacccttacgaatacaacgaagactatgattgctggattaacatttctgggaaagtaactctatcagcttatagatcaggtcgtaaaaaagggacaaaatgtatgaagtga

SEQ ID NO: 235 - DNA, 153 bp, Bacteriophage D
ttgtttgaatgcttggcatcgtttcggttaaattctcgaactgtaacctcgactttttgtcggggttttctttttttacaaaaaaatctaaattcctttatcaaaagtgttgacaaactatcatatatgatatataatgtatacataagataa

SEQ ID NO: 236 - DNA, 192 bp, Bacteriophage D
atgaatgaaagtgaattgcttgagcagttctgcgtttctctttgtgaatttagctctagacagtggccacgagatgggtttttagaccctattaaccgtgtggtctacatcaatagggatttaccaaccgaaagacgtttaaaggtcctactgcacgaattagggcacttagaacacgaccctaaacactaa

SEQ ID NO: 237 - DNA, 150 bp, Bacteriophage D
ttgttgggggctaagaccaccctttttgatataatatacctatatcaatggcttcccacgcatacgcgcagatacgttctgagggaagttttttatttgctttgttttgatagaaatgctactatattaatggatacagttaaaagctga

SEQ ID NO: 238 - DNA, 150 bp, Bacteriophage D
ttgttgggggttaagaccaccctttttgatataatatacctatatcaatggcttcccacgcatacgcgcagatacgttctgagggaagttttttatttgctttgttttgatagaaatgctactatattaatggatacagttaaaagctga

SEQ ID NO: 239 - DNA, 138 bp, Bacteriophage
atgaggaggtgtcttttttttggtttgctcaaaaaacgcaacaatggtataataatttttgcaacgacaaaccccctgcaaccacatggacagatacgctctgacgcagggctttttttatttgctttatttttataa

SEQ ID NO: 240 - DNA, 423 bp, Bacteriophage
atgaaaatcaatacgacaagagttaaaatggtcttgaagaatgaggctatacctgctgattatttagagagcgagattggcattagtcgttccgttgttgaaaaagtgagagaagatgagagcgaatttaaaaatttaactcttgattttgttgcgaaaattcaaaagtggattgatgatggaaactacactttcagctatgattacagcgacttgatagaagagttggaagaagatattgcagaaggtctaacggatgagtatatctatgttgtcagaggacaatacaacgaaattttagagaaatgcccaataattgactactactacacttctgaagagattgaagaaggagatctcgcagagaagaccctaacagcttctgccttgtctgaaatgaaacaggacaacgaaatcttttaa

SEQ ID NO: 241 - DNA, 423 bp, Bacteriophage D
atgaaaatcaatacgacaagagttaaaatggtcttgaagaataaggttatacctgctatttatttagagaatgagcttggtatcagtcgttctgttattgaaaaagtgagagatggcgagcgaaaaatagagaatctaacgctcgaaacaattattaaagtccagaaatggatagattcgggcaaatataccttctcttatgattattccgacttgatagaagagttggaagaagatattgcagaaggcttggtagatgagtatatctacgtagtcagaggtccgtataatgaacttttagataaatgcccaataattgactactactacacttctgaagagattgaagaaggagatctcgcagagaagaccctaacagcttctgtcttggctgaaatgaaaaaggacaacgaaatcttttaa

SEQ ID NO: 242 - DNA, 423 bp, Bacteriophage D
atgaaaatcaatacgacaagaattaaaatggtcttgaagaatgaggctatacctgctatttatttagaaaatgagcttggtatcagtcgttctgttattgaaaaagtgagagaagacgagagcgaatttaaaaatctaactcttgatgttgttgcgaaaattcaaaagtggattgatgatggcaattacacgtttagttatgattacagtgaatttatcgaggaattagaagaagatctcgctgagggtttaatagatgattacctattcgttgttcgtggagattatgacgaagccttaggaaaatgtcccatcattgactattactacacttccgaagaaattgaagaaggagatctcgcagagaagaccctaacagcttctgtcttggctgaaatgaaaaaggacaacggaatcttttaa

SEQ ID NO: 243 - DNA, 423 bp, Bacteriophage D
atgaaaatcaatacaacaagagtcaacatggtcttgaagaacgaggctatacctgctgattatttagagaacgtgattggtatcagtcgttccgttattgaaagagtgagagaagatgagagcggatttaaaaatttaactcttgatgttattgcgaaaattcaaaagtggatagatgaaggaaactacacgtttagttatgattacagcgacttgatagaagagttggaagaagatattgcagaaggcttggtagatgagtatatctacgtagtcagaggtccttataatgagattttagagaaatgcccaatcattgactactactacacttctgaagaaattgaagaaggagatctcgcagagaagaccctgacagcctctgccttagctgaaatgaagttagacaacaaaatcttttaa

SEQ ID NO: 244 - DNA, 423 bp, Bacteriophage D
atgaaaatcaatacgacaagagttaacatggtcttgaagaacaaagctataccagctaattatttagaaaaggaactgggaataaaccgttcgacaattacaagagtgcggaacggtgagagaaagcttgagaatctaacgctcgaaacaatcataaaagtccagaaatggatagattcgggcaaatatacattctcttatgattattccgacttgatagaagagttggaagaagatattgaagaaggcctaacagatgagtatatctatgttgtcagaggtccgtataatgaacttttagagaaatgcccaataattgactactactacacttctgaagagattgaagaaggagatctcacagagaagaccctaacagcttctgccttggctgagatgaaacaggataacgaaatcttttaa

SEQ ID NO: 245 - DNA, 423 bp, Bacteriophage O
atgataataaacactgcacgagttgaattagttttaatgaacaaagctataccagcaaattatttagaaagcgaaataggtattagtcgttcagcaattactagggtaagaaatgatgagcgaaaaatagagaatctgaagctcgaaacaatcataaaagtccagaaatggatagattcgggcaaatacacattctcttatgattattccgacttgatagaagagttggaagaagatattgcaaaaggtctggcaggtaagtatatctacgttgtcagaggaccatacaacgagattttagagaaatgtccaatcattgactattactacacttccgaagagattgaagaaggagagctcgcagagaagaccttgacagcttctgtcttggctgaaatgaagtcagacaacgaaatcttttaa

SEQ ID NO: 246 - DNA, 396 bp, Bacteriophage Proph
atggtcttgaagaacgaggctatacctgctgattatttagagagcgagattggcattagtcgttccgttgttgaaaaagtgagagaagatgagagcgaatttaaaaatttaactcttgatgttgttgcgaaaattcaaaagtggattgatgatggaaactacactttcagctatgattacagcgacctaatcgaagaactggaggaagatattgcagaaggcttggtagatgagtatatctacgtagtcagaggtccgtataatgaacttttagagaaatgcccaatcattgactactactatacttctgaagaaattgaagaaggggatcttgcagagaagaccttgataacttctgtcttagctgaaatgaagtcagacaacaaaatcttttaa

SEQ ID NO: 247 - DNA, 423 bp, Bacteriophage Sfi
atgataataaatgttgcacgagttgaaacagttttaatgaacaatgctataccagctaattatttagaaagagaaataggaattagtcgttcagcaattactagggtaagaaacggtgagcgaaaaatagagaatctgaagctcgaaacaatcataaaagtccagaaatggatagattcgggcaaatatacattctcttatgattattccgacttgatagaagagttggaagaagatattgcagaaggactaacggatgagtatatctacgttgtcagaggagcatacaacgagattttagagaaatgcccaatcattgactattactacacttccgaagagattgaagaaggagatctcgcagagaagaccctaacagcttctgccttgtctgaaatgaaacaggacaacgaaatcttttaa

SEQ ID NO: 248 - DNA, 423 bp, Bacteriophage TPL
atgataataaacactgcacgagttgaattagttttaatgaacaaagctataccagcaaattatttagaaagagagataggaattagtcgttcagcaattacaagagttcggaacggtgagagaaagcttgagaacctaacccttgaaactattatgactattcaaaagtggatagatgaaggaaactatcgctttagttacgattatagtgagcttatcgaagaccttgaggaagatattgcagaaggcctaacagatgagtatatctatgttgtcagaggtccgtataatgaacttttagagaaatgtccaatcattgactattactacacttccgaagagattgaagaaggaaatctcgcagagaagaccttgacagcttctgtcttggctgaaatgaaacaggacaacgaaatattttaa

SEQ ID NO: 249 - DNA, 423 bp, Bacteriophage TPJ
atgaaaatcaatacgacaagaattaaaatggtcttgaagaatgaggctatacctgctatttatttagaaaatgagcttggtatcagtcgttctattattgaaaaagtgagagatgatgagagcgaatttaaaaatctaactcttgaaactattataaaaatacaaagtttgataaattcgggcaaatatacattctcttatgattattccgacttgatagaagagttggaagaagatattgcagaaggactaacggatgagtatatctacgttgtcagaggaccatacaacgagattttagagaaatgtccaatcattgactattactacacttccgaagagattgaagaaggaaatctcgcagagaagaccttgacagcttctgtcttggctgaaatgaaacaggacaacgaaatattttaa

SEQ ID NO: 250 - DNA, 423 bp, Bacteriophage Proph
atgaaaatcaatacgacaagagttaaaatggtcttgaagaatgaggttatacctgctatttatttagagaatgagcttggtatcagtcgttctgttattgaaaaagtgagagatggcgagcgaaaaatagagaatctaactcttgaaacgattataaaaattcaaaagtggatcgatgatggaaactacactttcagctacgactatagcgacctaatcgaagaactggaggaagatattgcagaaggcttggtagatgagtatatctacgtagtcagaggtccgtataatgaacttttagagaaatgcccaatcattgactactactatacttctgaagaaattgaagaaggggatcttgcagagaagaccttgataacttctgtcttagctgaaatgaagtcagacaacaaaatcttttaa

SEQ ID NO: 251 - DNA, 183 bp, Bacteriophage D
atggaccaagttaaattagttttaatgaacaaagctataccagctaattatttagaaagacaaactggtgttagtcgttcagcaattactagggttagaaatggcgagcgaaaaatagaaaatctaacacttgaaacaattattaaaattcaaagttggatagactctgagaatacgatatag

SEQ ID NO: 252 - DNA, 195 bp, Bacteriophage D
atgataattaatgtggaccgagttaaagcggttttaatggataaatctataccggcaaattatttagaaatgcaaactggcattagtcgttcggcaattaccagagtaaggaacggcgagcgaaagatagaaaatctaactatcggaacaattattaaaattcaaagttggttggatagaaggatgattagataa

SEQ ID NO: 253 - DNA, 183 bp, Bacteriophage D
atggaccgagttaaattagttttaatgaacaaagctataccagcaaattttttagaaagacaaactggagttagtcgttcagcaattactagggttagaaataacgagcgaaaaatagaaaatctaacacttgaaacaattattaaaattcaaagttggatagattctgacaatacgatatag

SEQ ID NO: 254 - DNA, 228 bp, Bacteriophage D
ttgggaagaaggataaggataaagataaagataatgataataaatatggaccaagttaaattagttttaatgaacaaagatataccagctaattttatagaaagacaaactggtgttagtcgttcagcaattactaaggttagaaatggtgagcgaaaaatagaaaatctaagacttgaaacaattattaaaattcaaagttggatagactctgggaatacgatatag

SEQ ID NO: 255 - DNA, 216 bp, Bacteriophage D
ttgggaagtaggataaggataatgataattaatgtggaccgagttaaagcggttttaatggataaatctataccggcaaattatttagaaatgcaaactggcattagtcgttcggcaattaccagagtaaggaacggcgagcgaaagatagaaaatctaactatcggaacaattattaaaattcaaagttggttggatagaaggatgattagataa

SEQ ID NO: 256 - DNA, 195 bp, Bacteriophage D
atgataataaatatggaccgagttaaattagttttaatgaacaaagatataccagctaattttttagaaagacaaactggtgttagtcgttcagcaattactaaggttagaaatggtgagcgaaaaatagaaaatctaacacttgaaacaattattaaaattcaaagttggttagactctgagaatacgatatag

SEQ ID NO: 257 - DNA, 195 bp, Bacteriophage D
atgataataaacactgcacgagttgaattagttttaatgaacaaagctataccagctaattttttagaaagacaaactggtgttagtcgttcagcaattactagggttagagatggtgagcgaaagatagaaaatctaacacttgaaacaattattaaaattcaaagttggatagactctgacaataagatatag

SEQ ID NO: 258 - DNA, 216 bp, Bacteriophage D
atgacaaaaaggataaagacaatgataataaatatggaccgagttaaattagttttaatgaaaaaagatataccagctaattttttagaaagacaaactggtgttagtcgttcagcaattactagggttagaaatggtgagcgaaaaatagaaaatctaacacttgaaacaattattaaaattcaaagttggatagactctgagaatacgatatag

SEQ ID NO: 259 - DNA, 195 bp, Bacteriophage D
atgataataaacactgcacgagttgaattagttttaatgaacaaagctataccagcaaattatttagaaagacaaactggtgttagtcgttcagcaattactagggtgaggaatggtgagcgaaagatagaaaatctaacacttgaaacaattattaaaattcaaagttggatagactctgacaataagatatag

SEQ ID NO: 260 - DNA, 195 bp, Bacteriophage P
atgataattaatgtggaccgagttaaagcggttttaatggataaatctatatcagcaaattatttagaaatagaaactggcattagtcgttcggcaattaccagagtaaggaacggcgagcgaaagatagaaaatctaactatcggaacaattattaaaattcaaagttggttggatagaaggatgattagataa

SEQ ID NO: 261 - DNA, 513 bp, Bacteriophage D
atggtagtaaaaattaaaagaattgtttgggttaaaaataatggttttgaaatcagagaacgtgagctagattgttactttaaaaatgatggaagttacaaaaagagttctggagattgggaaagtcgttgttatgaacaattcggagatgaatttcaactcattagagatagcaaagcattagaatcttatagtggtttgacaagagattatcaaaaagacttaaaaatcttgcgtaagtataaacatagagatatgactatttcagagtatgaagcaatgaaatatgtcgtggagaattggacaaaagaatggtctcagtcaccttacagttatagtttttatagttcaaaaaacattgactggggttacaaaccagaaggcagcttacgcatttctgaccattggaattttggcgaaaatggtgaacattgcccaacagctgaaccagttgatggctgggcagtatgtaagtttgaaaatggtaaatatcatttaattaaaaagttttaa

SEQ ID NO: 262 - DNA, 513 bp, Bacteriophage D
atggtagtaaaaattaaaagaattgtttgggttaaaaataatggttttgaaatcagagaacgtgagctagattgttactttaaaaatgatggaagttacaaaaaaagttctggagattgggaaagtcgttgttatgaacaattcggagatgaatttcaactcattagagatagcaaagcattagaatcttatagtggtttgacaagagattatcaaaaagacttaaaaatcttgcgtaagtataaacatagagatatgactatttcagagtatgaagcaatgaaatatgtcgtggagaattggacaaaagagtggtcacaatcaccatacagcaatagtttctatagctctaaagatattgattggggctacaaaccagaaggtagcttaagagtctcagaccattggaattttggcgaaaatggtgaacattgcccaacagctgaaccagttgatggctgggcagtatgtaagtttgaaaatggtaaatatcatttaattaaaaagttttaa

SEQ ID NO: 263 - DNA, 474 bp, Bacteriophage D
atggtagtaaaaattaaaagaattgtttgggttaaaaataatggttttgaaatcagagaacgtgagctagattgttactttaaaaatgatggaagttacaaaaagagttctggagattgggaaagtcgttgttatgaacaattcggtaataaacttcaacttattaaagacagtaaaaaattagaatcgtacaacggattaacaaaagattatcaaaaagatttaaaaatcttacgtaaatgtggacgttcggaaatgaatgcaacagagtacgaagcaatgaaatatgttgaagaaaactggacaaaagagtggtcacaatcaccatacagcaatagtttctatagctctaaagatattgattggggctacaaaccagaaggtagcttaagagtctcagaccattggaattttggcgaaaatggtgaacattgcccaacagctgaaccagttgatggctgggcagtattttga

SEQ ID NO: 264 - DNA, 513 bp, Bacteriophage D
atggtagtaaaaattaaaagaattgtttgggttaaaaataatggttttgaaatcagagaacgtgagctagattgttactttaaaaatgatggaagttacaaaaaaagttctggagattgggaaagtcgttgttatgaacaattcggagatgaatttcagctcattagagatagcaaagcattagaatcttatagtggtttgacaagagattatcaaaaagacttaaaaatcttgcgtaagtataaacatagagatatgactatttcagagtatgaagcaatgaaatatgtcgtggagaattggacaaaagagtggtcacaatcaccatacagcaatagtttctatagctctaaagatattgattggggctacaaaccagaaggtagcttaagagtctcagaccattggaattttggcgaaaatggtgaacattgcccaacagctgaaccagttgatggctgggcagtatgtaagtttgaaaatggtaaatatcatttaattaaaaagttttaa

SEQ ID NO: 265 - DNA, 513 bp, Bacteriophage D
atggtagtaaaaattaaaagaattgtttgggttaaaaataatggttttgaaatcagagaacgtgagctagattgttactttaaaaatgatggaagttacaaaaaaagttctggagattgggaaagtcgttgttatgaacaattcggagatgaatttcaactcattagagataacaaagcattagaatcttatagtggtttgacaagagattatcaaaaagacttaaaaatcttgcgtaagtataaacatagagatatgactatttcagagtatgaagcaatgaaatatgtcgtggagaattggacaaaagagtggtcacaatcaccatacagcaatagtttctatagctctaaagatattgattggggctacaaaccagaaggtagcttaagagtctcagaccattggaattttggcgaaaatggtgaacattgcccaacagctgaaccagttgatggctgggcagtatgtaagtttgaaaatggtaaatatcatttaattaaaaagttttaa

SEQ ID NO: 266 - DNA, 513 bp, Bacteriophage D
atggtagtaaaaattaaaagaattgtttgggttaaaaataatggttttgaaatcagagaacgtgagctagattgttactttaaaaatgatggaagttacaaaaaaagttctggagattgggaaagtcgttgttatgaacaattcggagatgaatttcaactcattagagataacaaagcattagaatcttatagtggtttgacaagagattatcaaaaagacttaaaaatcttgcgtaagtataaacatagagatatgactatttcagagtatgaagcaatgaaatatgtcgtggagaattggacaaaagagtggtcacaatcaccatacagcaatagtttttatagctctaaagatattgattggggctacaaaccagaaggtagcttaagagtctcagaccattggaattttggcgaaaatggtgaacattgcccaacagctgaaccagttgatggctgggcagtatgtaagtttgaaaatggtaaatatcatttaattaaaaagttttaa

SEQ ID NO: 267 - DNA, 225 bp, Bacteriophage D
atgattaaaacggaaatgattgacgatattctcactttgattgaagaaattgaagctgttagcgataagaataaagaaaagtttattgaaaaatttgacgagttagaaaccaatttacaagcattgaataaacaaaccactgatgatttggttgaaattttacaagaagattattctgataattgggtagcaaaagaggtgattgaacttgttactaacagctag

SEQ ID NO: 268 - DNA, 225 bp, Bacteriophage D
atgaataaaatagaaatgattgacgatattctcactttgattgaagagattgacgccattagtgataagagtaaagaaacgttttttgaaaaaattgatgagttggaaacaaatttacaagcattgaacagacaaatcactgatgaattggttgaaattttacaagaagattattctgataattgggtagcaaaagaggtgattgaacttgttactaacagctag

SEQ ID NO: 269 - DNA, 225 bp, Bacteriophage D
atgattaaaacggaaatgattgacgatattctcactttgattgaagaaattgaagctgttagcgataagaataaagaaaagtttattgaaaaatttgacgagttagaaaccaatttacaagcattgaataaacaaaccactgatgatttggttgaaattttacaagaagattattctgataattgggtagcaaaagaggtgattgaacttgtcgatgactactag

SEQ ID NO: 270 - DNA, 225 bp, Bacteriophage D
atgattaaaacggaaatgattgacgatattctcactttgattgaagaaattgaagctgttagcgataagaataaagaaaagtttattgaaaaatttgatgagttagaaaccaatttacaagcattgaataaacaaaccactgatgatttggttgaaattttacaagaagattattctgataattgggtagcaaaagaggtgattgaacttgtcgatgactactag

SEQ ID NO: 271 - DNA, 513 bp, Bacteriophage D
atgagttatacaagcccagtttataacattaaacgagtacccattgacaaaatccaagcaaacagttataatccaaatcatgtagcacctcccgaaatgaaattgctttataagtctattttagaggacggatacactatgccaatcgtttgttattatcttaaagacgaggataaatacgagattgtagacggttttcaccgttacagcactatgcttaaccacaaagatatttatgaacgtgagggtggttgtttgccagtatccgttattgataagccaattagcgaccgcatggcgtcaactatccgacacaatcgagcgagagggtcacatgatatcgacctaatgacaaacattgtcgctgaccttgtagacagtggtatgtctgacgcttggattttaaaaaatatcggaatggacgcagacgaattgttgcgtttgaaacaattaactggtttagcgagtttgtttgcagacaaagaattcagtaaatcatgggatgtagaataa

SEQ ID NO: 272 - DNA, 513 bp, Bacteriophage D
atgagttatacaagcccagtttataacattaaacgagtacccattgacaaaatccaagcaaacagttataatccaaatcatgtagcacctcccgaaatgaaattgctttataagtctattttagaggacggatacactatgccaatcgtttgttattatcttaaagacgaggataaatacgagattgtagacggttttcaccgttacagcactatgcttaaccacaaagatatttatgaacgtgagggtggttgtttgccagtatccgttattgataagccaattagcgaccgcatggcgtcaactatccgacacaatcgagcgagagggtcacatgatatcgacctaatgacaaacattgtcgctgaccttgtagacagtggtatgtctgacgcttggattttaaaaaatatcggaatggacgcagacgaattgttgcgtttgaaacaattaactggcttgtcgagtttgtttgcagacaaagaattcagtaaatcatgggatgtagaataa

SEQ ID NO: 273 - DNA, 513 bp, Bacteriophage D
atgagttacacaagtccagtttataacattaaacgagtacccattgacaaaattcaggcaaacagttataatccaaaccatgtagcacctcctgaaatgaaactactttacaagtctattttagaggatggatacacaatgccaatcgtttgttattatcttaaagatgaagataaatatgagattgtagatggctttcaccgttatagcactatgcttaaccacaaagatatttatgaccgtgagggcggttgtttgccagtatccgttattaataagccaatcagtgaccgtatggcatcaactatccgacataatcgagcgagagggtcacatgatattgacctaatgacaaacattgtcgctgaccttgtagacagtggtatgtctgacgcttggattttaaaaaatatcggaatggacgcagacgaattgttgcgtttgaaacaattaactggcttggcaagtttgtttgcagacaaagaattcagtaaatcatgggatgtagaataa

SEQ ID NO: 274 - DNA, 513 bp, Bacteriophage D
atgagttatacaagcccagtttataacattaaacgagtacccattgacaaaatccaagcaaatagttataatccaaatcatgtagcacctcccgaaatgaaattgctttataagtctattttagaggacggatacactatgccaatcgtttgttattatcttaaagacgaggataaatacgagattgtagacggttttcaccgttacagcactatgcttaaccacaaagatatttatgaacgtgagggtggttgtttgccagtatccgttattgataagccaattagcgaccgcatggcgtcaactatccgacacaatcgagcgagagggtcacatgatatcgacctaatgacaaacattgtcgctgaccttgtagacagtggtatgtctgacgcttggattttaaaaaatatcggaatggacgcagacgaattgttgcgtttgaaacaattaactggcttggcaagtttgtttgcagacaaagaattcagtaaatcatgggatgtagaataa

SEQ ID NO: 275 - DNA, 513 bp, Bacteriophage D
atgagttacacaagtccagtttataacattaaacgagtacctattgataaaattcaggcaaacagttataatccaaaccatgtagcacctcctgaaatgaaactactttacaagtctattttagaggatgggtacacaatgccaatcgtttgttattatcttaaagatgaagataaatatgagattgtagatggctttcatcgctatagcactatgcttaaccacaaagatatttatgaccgtgagggcggttgtttgccagtatccgttattaataaaccgattagtgaccgcatggcgtcaactatccgacacaaccgggcgagagggtcacatgatattgacctaatgacaaacattgttgctgaccttgtagatagtggcatgtctgacgcttggattttgaaaaatatcggaatggacgcagacgaattgttgcggttgaaacagttaactggtttagctagtctatttgcagacaaagaattcagtaaatcgtggatcgtagaataa

SEQ ID NO: 276 - DNA, 513 bp, Bacteriophage D
atgagttacacaagtccagtttataacattaaacgagtacccattgacaaaatccaagcaaacagttataatccaaatcatgtagcacctcccgaaatgaaattgctttataagtctattttagaggacggatacactatgccaatcgtttgttattatcttaaagacgaggataaatacgagattgtagacggttttcaccgttacagcactatgcttaaccacaaagatatttatgaacgtgagggtggttgtttgccagtatccgttattgataagccaattagcgaccgcatggcgtcaactatccgacacaatcgagcgagagggtcacatgatatcgacctaatgacaaacattgtcgccgaccttgtagacagtggtatgtctgacgcttggattttaaaaaatatcggaatggacgcagacgaattgttgcgtttgaaacaattaactggcttggcaagtttgtttgcagacaaagaattcagtaaatcatgggatgtagaataa

SEQ ID NO: 277 - DNA, 180 bp, Bacteriophage D
atgcctaaagtttccgagagcaaacggaaagcaaatgacaaatgggacaaaaagaacaaagaacgcaagcagtatatcaacagacgttctgtcgcaaggaactttattaagaatatggaaggcgaagatattccagaatttaaaaaactaatagaagaaagagcttccaaaatcaaataa

SEQ ID NO: 278 - DNA, 180 bp, Bacteriophage D
atgcctaaagtttccgagagcaaacggaaagcaaatgacaaatgggacaaaaagaacaaagaacgcaagcagtatattaacagacgttctgtcgcaaggaactttattaagaatatggaagacgaagatattccagaatttaaaaaactaatggaagaaagagcttccaaaatcaaataa

SEQ ID NO: 279 - DNA, 180 bp, Bacteriophage D
atgcctaaagtttccgagagcaaacggaaagcaaatgacaaatgggacaaaaagaacaaagaacgcaagcagtatattaacagacgttctgtcgcaaggaactttattaagaatatggaagacgaagatattccagaatttaaaaaactaatggaagaaagaacttccaaaatcaaataa

SEQ ID NO: 280 - DNA, 198 bp, Bacteriophage D
atgcctaaagtctcagaaagcaaacggagagcgaataataaatgggataaaaaaaataaagaacgtaaacaatatataaacaaacgttccgttgcaagaaactttattaagaacatggaagatgaagatgttccggaatttaaaaaactaatggaagaaagagcttccaaaacaaataaaacgtgttttagttcatga

SEQ ID NO: 281 - DNA, 180 bp, Bacteriophage D
atgcctaaagtttccgagagcaaacggaaagcaaacgacaaatgggataaaaataacaaagaacgcaagcagtatattaacagacgttctgtcgcaaggaactttattaagaatatggaagacgaagatattccagaatttaaaaaactaatggaagaaagaacttccaaaatcaaataa

SEQ ID NO: 282 - DNA, 246 bp, Bacteriophage D
atgaagttaactaatcaacagaatcaagcctttaagaaattcaaaaatttgagagttggagctctatttatggagcaaggaacaggtaagacaagagtagcactagagttaatcagaaaaacagatgctgatttagccttgttcttttgtccgttttcaaccaaaaacaatcttttatctgagattgaaaaatggggaattgatattgaatttatggtgtatggatatgaaacgatttcatcatag

SEQ ID NO: 283 - DNA, 177 bp, Bacteriophage D
gtggaaacagaaccaaattttcaaataatatgttataataaaagtacctcgtttgaggtatttttttatcttacaactgcacccgaattttttcaggtgtttttttttcgcccaaaaatcacccgaaaactttgggaaaagctagaaaaaataaaaataaacgaggtaaaaacatag

SEQ ID NO: 284 - DNA, 204 bp, Bacteriophage D
gtggaaacagaaccaaattttcaaataatatgttataataaaagtacctcgtttgaggtattttttatcttacaactgcacccgaattttttcaggtgttttttttgcccaaaaatcacccaaaaactttgggaaaagctagaaaaaataaaaaataaacgaggtaaaaacatagtatgttttactaattttcaagctgattaa

SEQ ID NO: 285 - DNA, 159 bp, Bacteriophage D
atgggttttacggttacatgttgcaataacctgcggtcactgagtaaccataaccactactgctgctttcttcgcctcgttttcgtcccaactaaaattgaaatcataccaataatctggtttatctttagggtgtctcacggatttcaaacggtgtga

SEQ ID NO: 286 - DNA, 453 bp, Bacteriophage D
ttggaatacttggcatcgtttcggttaaattctcgaactgtaacctcgacttttagtcgaggttttctttttttgcaaaaaaaactaaattccttaataaataaaaataaaaactataaaaacttagtacagcttcatttattctcaaattttatatattttcgttcaagaattgttctgttgttaaacctaaagcgcgagcgaaatcatcagctttattcagcgggaacacccgactacctgaaagatatcttgtttgaaatcccagctttatttgcattgacatggaactgttgtctaaatagctttttattatcgttgtttctcatatttaatagtataaacattatacaaaagttcccaaaaataaacaatatgttcccaaaaataaacttttttcatatttttttgattttagtgttgacaaatgggaacgtgttagatatactataa

SEQ ID NO: 287 - DNA, 282 bp, Bacteriophage D
atggaagttgaacaaagactagaacaactaagacaagattggttgaaacacccaaatttaacagatactttaaaagaatatctaaacgaatatttttacgatgattattcttattgtgagaaatgtgataggattgccagcgatagcgattggttttggtatgaaggcgaagactatacggattttttacacattgattgtaataaagaaaaattttacgaagcaacaaaaaaaacctctggaaggaggagaccagaggaaaacataaaaggagaaagttag

SEQ ID NO: 288 - DNA, 228 bp, Bacteriophage D
atgaaaactaagacacttgggcgccgtttaagacgtttaagaaaaatcaatggagaaacacaaaaggaatttgccgaaaattttggaagacattatagaaccgttcaaaattgggagctagattgttcaataccagacgttttcacagcaatggcattggcagaatattataacatggacgttgaagaattggtgaatggagaagatgactatgacaaagaattttga

SEQ ID NO: 289 - DNA, 378 bp, Bacteriophage D
atggagaagatgactatgacaaagaattttgaaaattttaaaaaaggctgggataatgttcaacaagtagtaaatgaatacagcaaaaaactcgttgaaaacagtcaagaaaatgtaaccaaccgagatagtgaagagtatcagcaaatcaaaggtaaagataacgtaattagtccaaaccactatgtaaccgataagggttttgaagtgtttgacgtgcaagaagcttttatccacgaattaaaaggaatggcagctagttactggtgcaatgttgtgaagtatattttgagatttcaaagaaagaatggagtggaagacttaaaaaaagctaagtactacttggaaaaattaattgaaaaagaggaaggtaaataa

SEQ ID NO: 290 - DNA, 546 bp, Bacteriophage D
atgaataaacaagaagcaattgaactagtaaaaaatacttcatacagtgtaccaattgatagcccagtgaaacatcttacagaagatacagttatcaatattatcaaacagcttgatgaaccagagaaagctacagtgccagattttgtagcaaaatacattgaagaaagcagagaatttgacagaaaattaaatgacgctttatcttactcaaacactaccgtcgcaatggacgactggtttgaagaaaacgaagtagacaacacggaaatatttgctaaggcatggcttcacggctatgaagtagaaaaagaaaaactttacacagttgaaattccagaccctaatgcaagtggttacggtaagacatttcttggcagagatgatgatggaaaagtagtgctatctacttggactggttttagttccattgaatttgctgatgattggaaacaatcagaacgtgcacagttgacagaagatgaaattaaaaaaggttttacttgggcttggaatgaagggtttgccgaagaggtgaaagaatga

SEQ ID NO: 291 - DNA, 162 bp, Bacteriophage D
atgaaacgctttgtagtaacaggttacaaagatggttggtttgtcttctcatttcctttaaacgccataaactcttattatgctatccaatatgcaagcgaagatgaattggtagaaggtatggagttcgataagctggttataaaagaggtgaaagaatga

SEQ ID NO: 292 - DNA, 147 bp, Bacteriophage D
atgaacataaaagaggtgttctgtattgattgctatgaatggaaaaagaaagaagacttaacagggagcaaattttccaatgatattttatattgcaaagaatgtggttacgccttagttcgtacgtgtgaccgtaataacaaatga

SEQ ID NO: 293 - DNA, 165 bp, Bacteriophage D
atgacaaacattgttgctgaccttgtagatagtggcatgtctgacgcttggattttgaaaaacattgggatggatgctgacgaattgctgcgactaaagcaacttagcggactggcttccttgttcaaagataaggaattcactacagcttgggaagtaggataa

SEQ ID NO: 294 - DNA, 273 bp, Bacteriophage D
atggaaacttataaagaatacaaacaacaacagaaagaagaacgtgaaagagtaagagcgcttcgtagtgaagtattttcaggcaacgctgaaaagcttgcgacagatattgtaaggatttcgagcggagatgtttataaaattatcccacgttttgggactagatatgaaaaaagtccaatcatcaaattagacccagaagaagtagaacgccacatcaaagaagctcgtgaagtcagagaacttgcgaaaattatggcaagcaaagaatag

SEQ ID NO: 295 - DNA, 243 bp, Bacteriophage D
atggcagtagtggtcgaagcctcagcattatgctggggctttttttgttataatatacctatatcaatggcctcccacgcatacgcgcagatacgttctgatgggaggttttttttgttgccgttaaaacggacaaaaaaatttaaaaagtttgattttattgttgataatacacgcataagcgtgtataatgtaattaaagataaggaaagcgaggaaaacaaaaatggtagtaaaaattaa

SEQ ID NO: 296 - DNA, 471 bp, Bacteriophage D
ttgctggggctttttttgtgttataatagaataaaaaaacaaatagatgaggtaagaaaaacggctattgacctgtatcgtgaactggatatccaatcgttggagcaaagattggaaaagaacgaagaaaacactcaacgcttcctccaacaaacagccaaaagcttaaaccaagacaagactgaactatctctccgaactgaccagttagggcgtagtgttgaaaagattgaaaacaaactagacgacatgtacgctaagaacgaactagacttgaaattccagatgatggatcaaaagattgacgctaaatttgatacctttggtcaacgcatggaaaacatgttcttagcacaaaccaataggcaacttgaggaacaagccaagaatagaaaagaattcacatattggtttatttgcattcttgtagctatcgctgttattgctattcctgtttggttcggcaaataa

SEQ ID NO: 297 - DNA, 204 bp, Bacteriophage D
atgtcattttttacgtcaacaaaaacggcaacgtcaacttttttcatagcaagtaatagaatacttgcatcatttcgattaaattctcgaactgtacacccgtcttttttaggtgggttttttgttttgcaaaaaaatctaaatttatttatcaaaagcattgacaaactatcatgtatgatatataatatacttataagataa

SEQ ID NO: 298 - DNA, 129 bp, Bacteriophage D
atgttactaatagtgacattcagttatatcataaattatttgttgttcgatttgggaagtagcttaattaaaaaaggagaaagaaaatgctactataaaggatttaagacaaagaaggatgtaatctaa

SEQ ID NO: 299 - DNA, 159 bp, Bacteriophage D
ttggagtgcttatattttaggaaaaaagagggcgcttgctctcttttttttatgtattcaataaaaagtatactttataaattttagagttattttgttaaaaactcaaaaaaacttgaaaaaaaatcaagaaaactgttgacattgaattttgtttaa

SEQ ID NO: 300 - DNA, 690 bp, Bacteriophage D
ttggatatttacgtttatactgatgaatcaggagtatttgataaagaacatgaaacaatatatgtttatggtggagtgatttttttaacttctgaggacaaagagaattcaggtagaagatatatatatgcggaaaaagcactaagaaaaagccatagtaattataggaaaggggaactgaaagcaagtaggcttaaaaatagacataaagccagtttgtttaggtcgcttaatagggaaataaaattttctatagtggtgagtattggcagggtgcatgataggattttttgtgagaaaaaaagtaagcagcgttacttagattatgtttacaaagttggtttgaaaaaggtgttacaacgtcttgtagcagattgtaaaatagagactaccgaagtagatacgatcagtatttttacagatgagcatagtactgcgactaatggaaaatatgagttaagagaggcgctgttaaacgagtttaaatatggcacgtttaacccagactggaatattttttatcctcccttattcgaaaaactatctagtttaactgttgaatactgtaattcagctaaaaagccacatatacgtatggcagatataatagcgaatagagcatattatcttgcaaagaatgatctttttggagagttgggagagaaaactatatcaatccacttcccttag

SEQ ID NO: 301 - DNA, 135 bp, Bacteriophage D
ttggagagttgggagagaaaactatatcaatccacttcccttagttttagaaagaggcgaggctgtaagcctctttttattataatggtcaagtatgtgggattttgcttaattctgttcatgacattagggtag

SEQ ID NO: 302 - DNA, 150 bp, Bacteriophage M
gtgcacaaaaagggaattcatataaaaaaagtcggctattttagtcgactcttttttttatgtcatgtaaacagcagtatagcgttttctattatgttatcgatgtcgtgtcgtttctctaactttttcaaatgttggaaacttttctga

SEQ ID NO: 303 - DNA, 141 bp, Bacteriophage M
ttgttgggggggctaagacgccccctttttgatatatcaacggcctcccacccgtcttttttaggtgggttttttgttttgcaaaaaatttttttatcaaaagtacggatacatacaaagaatacgcttttaacgttttaa

SEQ ID NO: 304 - DNA, 438 bp, Bacteriophage P
atgaacgaaatagcattatcggacaatcttgcacagattgaacttgaaatcaatcatcataagcagattgcaggtcagtctatttgggaaatcggcaggcgtttaaatcatgttaaagagcacgatttagcgcatgggcaatttatggaatgggttgaaaaacttggtataaatcaaccagaagccaatcgtatgatgagagttgctaaagaactaccaaattcttcaacgttgagtaatttaggaagcacggctctctacttaatcgccactcttccagatgatgaaaagcaagaacaaattgaaaagattgagcaaggtgaatcaccaacggtcagagaattgcaagagataaagcgtcgtctcaaactcaaagaccaagcactggaagcggtcaagggtgagttggaacgtgctatacttggtattaaagtttaa

SEQ ID NO: 305 - DNA, 438 bp, Bacteriophage P
atgaacgaaatagcattatcggacaatcttgcacagattgaacttgaaatcaatcatcataagcagattgcaggtcagtctatttgggaaatcggcaggcgtttaaatcatgttaaagagcacgatttagcgcatgggcaatttatggaatgggttgaaaaacttggtataaatcaaccagaagccaatcgtatgatgagagttgctaaagaactaccaaattcttcaacgttgagtaatttaggaagcacggctctctacttaatcgccactcttccagatgatgaaaagcaagaacaaattgaaaagattgagcaaggtgaatcaccaacggtcagagaattgcaagagataaagcgtcgtctcaaactcaaagaccaagaactggaagcggtcaagggtgagttggaacgtgctatacttggtattaaagtttaa

SEQ ID NO: 306 - DNA, 336 bp, Bacteriophage P
atggaagaattagaacaagcgtttgaaaatcttgatgattggtatctatcaagcatgaaagacagtgcttacaaggattttgggaaatacgaaattcgcttatcaaatcattcggcagacaataaatatcatgacctagaaaatggtcgcttaatcgttaatgttaaagctagtaaattgaacttcgttgatatcatcgagaataaaatctataaaatcattgagaaaattgaaactctcgatttagacaagtacagatttattaacgctactaaaatggaaaacgatatcaaatgttattacaagggatttaagacaaagaaggatgtgatctaa

SEQ ID NO: 307 - DNA, 177 bp, Bacteriophage P
atgacagatgcgcacaaaaaagctgttaagaagtggaataaaaacaacagagaacatagaaattatctaaacaagcgttcatcagctcgtggtttcatcagaaataatgcgactgctgaagatttgagagagctagaggagcttattgcagaaagaagaaaaaagaattttaggtaa

SEQ ID NO: 308 - DNA, 294 bp, Bacteriophage P
ttgttaaacctaaagcgcgagcgaaatcatcagctttattcagcgggaacacccgactacctgaaagatatcttgtttgaaatcccagctttatttgcattgacatggaactgttgtctaaatagctttttattatcgttgtttctcatatttaatagtataaacattatacaaaagttcccaaaaaataaacaatatgttcccaaaaataaacttttttcatatttttttgattttagtgttgacaaatgggaacgtgttagatatactataattgttctaaggaacaagtaa

SEQ ID NO: 309 - DNA, 105 bp, Bacteriophage P
ttgcaaaaaaaatatataattttttataaaaacagtttccgtctggtcgcaaaaatcgacttgaatggattgaaaacaatcttgaaaacattcgataaaaaataa

SEQ ID NO: 310 - DNA, 105 bp, Bacteriophage P
ttgcgcacacacaagcataagggaaaattttgttggggggggctaagacgccccctttttgatataatatacctatatcaacggcctcccacccgtcttttttag

SEQ ID NO: 311 - DNA, 132 bp, Bacteriophage P
atgctggggcttttttttaatataaatgctactatattaatggatacagttaaaagagaagcatccagatatgatggattttatggacctgatagattggtatttagaaaatcgcaaaccataagatattga

SEQ ID NO: 312 - DNA, 222 bp, Bacteriophage TPL
atgtacgctaagaacgaactagatttgaaattccagatgatggatcaaaagattgacgctaaatttgatacctttggtcaacgcatggaaaacatgttcttagcacaaaccaataggcaacttgaggaacaagccaagaatagaaaagaattcacatattggtttatttgcattcttgtagctatcgctgttattgctattcctgtttggttcggcaaataa

SEQ ID NO: 313 - DNA, 222 bp, Bacteriophage TPJ
atgtacgctaagaacgaactagacttgaaattccagatgatggatcaaaagattgacgctaaatttgatacctttggtcaacgcatggaaaacatgttcttagcacaaaccaataggcaacttgaggaacaagccaagaatagaaaagaattcacatattggtttatttgcattcttgtagctatcgctgttattgctattcctgtttggttcggcaaataa

SEQ ID NO: 314 - DNA, 183 bp, Bacteriophage D
atggatacatataaagaacaattttattatttggatcctatttatattagtgtggatattaataggaggacttttattttaggaaaaagagggcaatcgctctctttttttattgtaataaaacaatttaaaaatataactaaaaaaacttcaaaaaaatcgaaaaaaaatattgacaaataa

SEQ ID NO: 315 - DNA, 177 bp, Bacteriophage P
atgctggggctttttttgtgttataatatgaatgagatgtcaatccccccacatccttttatggacagatacgttctgagtgggggtttttttgttttgctattttttaacctaacagcccgtaattcccccacctctaaggtggcgggatgtaagggcttcggtctagtgcagtga

SEQ ID NO: 316 - DNA, 195 bp, Bacteriophage D
atgttcagcgaccttgtgcgttcgaaagtgtataagggaacattttgttgtgggctaagaccccctttttttgatataatatatctatatcaatgtcctcccacgcataagcgcagatacgttctgagggaggttttttatttgttttattttgataaaaatgctactatattaacggatacagttaaaagctga

SEQ ID NO: 317 - DNA, 195 bp, Bacteriophage D
atgttcagcgaccttgtgcgttcgcaagtgtataagggaacattttgttgtgggctaagaccccctttttttgatataatatatctatatcaatgtcctcccacgcataagcgcagatacgttctgagggaggttttttatttgttttattttgatataaatgctactataataatggatacagttaaaagctga

SEQ ID NO: 318 - DNA, 264 bp, Bacteriophage P
atgaatagcatgaaaaagccccacactgcggaaaacggcgatttaattcatacaacagaagacaacgaggcttcagatatatcaatcattacaatttcgtttgttcgcaaaacgaacaagcaaatattgaaaaattcgaaagtttgcctaaaacgttacaagctcaagtatctaaaccatctgccaatccagaggttaatcaagcagtattcgacggagatatcaaagcaaaaagaaattatagctcttgaaaaaaatgagtga

SEQ ID NO: 319 - DNA, 243 bp, Bacteriophage P
atgaatagcatgaaaaagccccacactgcggaaaacggcgatttaattcatacaacagaagacaacgaggcttcagatatatcaatcattacaatttcgtttgttcgcaaaacgaacaagcaaatattgaaaaattcgaaagtttgcctaaaacgttacaagctcaagtatctaaaccatctgccaatccagaggttaatcaagcagtattcgacggagatatcaaagcaaaaagaatattga

SEQ ID NO: 320 - DNA, 81 bp, Bacteriophage D
atgttcagcgaccttgtgcgttcgaaagtgtataagggaacattttgttgtgggctaagaccccccttttttttgatataa

SEQ ID NO: 321 - DNA, 153 bp, Bacteriophage D
atggcagtagtggtcgaagcctcagcatttttgctggggctttttttgtgttataatatgaaacatcattttatggacagatatttgctttgttttgataaaaatgctactatattaatggtcttcgataaactctctctcgccctgacttga

SEQ ID NO: 322 - DNA, 276 bp, Bacteriophage D
atgataactaaagaacaattaaaaggatactacagcgaacacttggaagagctcgtcgaatgggcagacgatataaataaaatcgcttatgagatagatgggaaaagtcatcaaactaagataggttgggtgaatgatagattaaaagaccattttatgaaagaaaaaggggttttagttattcattacaccaatgagcaagtcgaaacagcctacaatgagtgggtaaaaattacagaggaggcgtttaatggattctttaataacacaatctaa

SEQ ID NO: 323 - DNA, 138 bp, Bacteriophage P
atggcagcagtggtcgaagcctcagcatttttgctggggctttttttgtgttataatatgaatgagatgtcaatccccccacatccttttatggacagatacgttctgatgggaagttttttatttgctttgttttga

SEQ ID NO: 324 - DNA, 147 bp, Bacteriophage D
atggcagtagtggtcgaagcctcagcattatgctggggctttttttgtgttataatatacctatatcaatggcctcccacgcatacgcgcagatacgttctgatgggaggtttttttgttgccgttaaaacggacaaaaaaatttaa

SEQ ID NO: 325 - DNA, 120 bp, Bacteriophage D
gtggtcgaagcctcagcattatgctggggctttttttgtgttataatacatatatcaatggcttcccacgcatacgcgcagatacgttctgagggaagttttttatttgcttttttttga

SEQ ID NO: 326 - DNA, 126 bp, Bacteriophage D
atggcagtagtggtcgaagcctcagcattttgctggggctttttttgtgttataatatacatggaacgacaaaccccctgcatccacatggacagatacgctctgacgcagggcttttttatttga

SEQ ID NO: 327 - DNA, 132 bp, Bacteriophage P
atggcagcagtggtcgaagcctcagcatttttgctggggctttttttgtgttataatatacctatatcaatggcttcccacgcatacgcgcagatacgttctgagggaggttttttgtttgctttattttga

SEQ ID NO: 328 - DNA, 519 bp, Bacteriophage D
atggaaaattactctagtccagtgtataatattaaaaaaatcccgattgaaaaaattcaagcgaatagctataaccccaaccatgtagcgacaccagaaatgaagttgttatatgaatccatcaaagcagacggatacacaatgcctatcgtttgttattatcttaaagatgaagacaaatacgagattgtagatggctttcaccgttatacaactatgcttaatcataaagatatttacgaacgagagaatggctgtttacctgtatctgttattgataaaccattagaggagcgcatggcttctacagtacgacacaatcgagcaagaggtagtcatgatattggcttaatggctaatattgtaactgaattggttgatagcggaatgtctgatgccaaagttatgaaaagtcttggaatggacgcagacgagttattaagattaaaacaggttagcggtttagcaagtttgtttgcaaacaaggagttcagtaaatcgtgggatataaaaaaatag

SEQ ID NO: 329 - DNA, 516 bp, Bacteriophage D
atgcaaacatactctagccctgtatataatattaagcgcgtgcctattgagaaaattcaagcaaacagctacaatcctaaccatgtagcaagcccagaaatgaagttgctttaccaatccatcaaagaagatggttacacaatgccaatcgtatgttattaccttgaggatgaagataagtatgaaattgtggacggtttccatcggtatacaacgatgaaagaacacaaggatatctatgaaagagaggaggggtgtctaccagtttctgttatagataaaccaatcagtgaccgaatggcatcaactatcagacacaatagagcaagagggtcgcacgacatcggtctgatgactaatatcatttctgacctagttgattctgggatgtcagatgcgtggattatgaaaaatattggtatggatgctgatgaattactacgactaaaacaagttagcggactggcttccttgttcaaagataaggaattcacgacagcttgggaagaaggataa

SEQ ID NO: 330 - DNA, 516 bp, Bacteriophage D
atgcaaacatactctagccctgtatataatattaagcgcgtgcctattgataaaattcaagcaaacagctacaatcctaaccatgtagcaagcccagaaatgaagttgctttatcaatccatcaaagaagatggttacacaatgccaatcgtatgttattaccttgaggatgaagataagtatgaaattgtggacggttttcatcggtatacaacgatgaaagaacacaaggatatctatgaaagagaggaggggtgtctaccagtgtctgtcatagataaaccaatcagtgaccgaatggcatcaactatcagacacaatagagcaagaggttcgcacgacatcggtctgatgactaatatcatttctgacctagttgattctgggatgtcagatgcgtggattatgaaaaatattggtatggatgctgatgaattactacgactaaaacaagttagcggactggcttccttgttcaaagataaggaattcacgacagcttgggaagaaggataa

SEQ ID NO: 331 - DNA, 513 bp, Bacteriophage D
atgcaaacatactatagccctgtatataatattaagcgcgtgcctattgagaaaattcaagcaaacagctacaatcctaaccatgtagcaagcccagaaatgaagttgctttatcaatccatcaaagaagatggttacacaatgccaatcgtatgttattaccttgaggatgaagataagtatgaaattgtggacggtttccatcggtatacaacgatgaaagaacacaaggatatctatgaaagagaggaggggtgtctaccagtttctgtcatagataaaccaatcagtgaccgaatggcatcgactatcagacacaatagagcaagagggtcgcacgacatcggtctgatgactaatatcatttctgacctagttgattctgggatgtcagatgcgtggattatgaaaaatattggtatggatgctgatgaattactacgactaaaacaagttagcggactggcttccttgttcaaagataaggaattcacgacagcttgggaagaatga

SEQ ID NO: 332 - DNA, 225 bp, Bacteriophage D
atggcacaaattaaagatggttggcataaagtttataacgaaaatgtttatgttgaaaacgaaaaagtagtacgaggaacaaaaaaagattataacggttctgaggtcacttgttatccttacgaatacgataaaaaccaagattgttggattaatatttctgggaaagcaactctttcttcttatagagcaggactcaaaaaaggcactaagtgtatgaagtaa

SEQ ID NO: 333 - DNA, 138 bp, Bacteriophage D
atgttcagcgaccttgtgcgttcgaaagtgtataagggaacattttgttgtgggctaagaccccctttttttgatataatatatctatatcaatgtcctcccacgcataagcgcagatacgtgctgagtcttcgataa

SEQ ID NO: 334 - DNA, 123 bp, Bacteriophage D
atgctggggctttttttgtgttataatatgaatgagatgtcaatccccccacatccttttatggacagatacgttctgagtgggggtttttttgttttgctattttttaaaaatgtggtataa

SEQ ID NO: 335 - DNA, 141 bp, Bacteriophage D
atgctggggctttttttgtgttataatatgaatgagatgtcaatccccccacatccttttatggacagatacgttctgagtgggggttttttgttttgctattttttaaaaatgtggtataatataaatatccattcataa

SEQ ID NO: 336 - DNA, 258 bp, Bacteriophage D
atgaagaaattttggcatagcggtatgattgacaagaaggttattgaaaaacgtaaacaagatgattatatgaataaattacacaggactattcttgagttgagtataaaaccacctgaacccgaaccttggtacagacatccagaaatgagagcattgttggataggattgattctatggacatgatagattggtattcaaaatatctaaaacatcgcaaaccatacgataattatagtggagaattagagaaatga

SEQ ID NO: 337 - DNA, 180 bp, Bacteriophage
atgaagaaattttggcgtagtggaatgattgacaagaaggttatcgaaaaacgacaacaagaagagtatattaataagttacataggactattcttgagttgagtataaaaccacctgaaccagaaccttggtacagacatccagaaatgagagcattgttggatagaattgatgattag

SEQ ID NO: 338 - DNA, 198 bp, Bacteriophage D
atgaagaagttttggcgtagtggaatgattgacaagaaagttattgaaaaacgacaacaagatgattatatgaataagttacataggactattcttgagttgagtataaaaccacctgaacccgaaccttggtacagacatccagaaatgagagcatttttggataggatttatgattcgagaagcaatttaaagtaa

SEQ ID NO: 339 - DNA, 180 bp, Bacteriophage D
atgaagaaattttggcgtagtggaatgattgacaagaaaattattgcgaaacgtgaacaggatgagtatttgaataaattacacaggactattcttgagttgagtagaaaaccacctgaacaagaaccttggtacagacatccagaaatgagagcattgttggatagaattgatgattag

SEQ ID NO: 340 - DNA, 180 bp, Bacteriophage D
atgaaaaaattttggcatagcggtatgattgacaagaaagttattgaaaaacgtaaacaagatgattatatgaataagttacataggactattcttgagttgagtataaaaccacctgaaccagaaccttggtacagacatccagaaatgagagcattgttggataggattgatgattag

SEQ ID NO: 341 - DNA, 198 bp, Bacteriophage D
atgaagaagttttggcgtagtggaatgattgacaagaaagttattgaaaaacgacaacaagatgattatatgaataagttacataggactattcttgagttgagtataaaaccacctgaacccgaaccttggtacagacatccagaaatgagagcattgttggataggatttatgattcgagaagcaatttaaagtaa

SEQ ID NO: 342 - DNA, 180 bp, Bacteriophage TPJ
atgaagaaattttggcgtagtggaatgattgacaagaaggttattgaaaaacgtaaacaagatgattatatgaataaattacacaggactattcttgagttgagtataaaaccacctgaaccagaaccttggtacagacatccagaaatgagagcattgttggatagaattgatgattag

SEQ ID NO: 343 - DNA, 180 bp, Bacteriophage Proph
atgaagaaattttggcgtagtggcatgattgacaagaaggttattgaaaaacgtaaacaagatgattatatgaataaattacacaggactattcttgagttgagtataaaaccacctgaacccgaaccttggtacagacatccagaaatgagagcattgttggataggattgatgattag

SEQ ID NO: 344 - DNA, 177 bp, Bacteriophage D
atgaagaaattttggcgtagtggcatgattgacaagaaggttattaaaaaacgtaaacaggaagagtatatgaataagatgcataggactattcttgaattaaaaaatgagaagcatccagatatgatggattttatggacctgatagattggtatttagaaaatcgcaaaccataa

SEQ ID NO: 345 - DNA, 189 bp, Bacteriophage D
atgaagaaattttggcatagcggtatgatcgacaagaaagttattgaaaaacgtaaacaggatgagtatttgaataaattacacaggactattcttgagttaaaaaatgagaagcatccagatatgatggattttatggacctgatagattggtatttagagaatcgcaaaccacgagatattgattag

SEQ ID NO: 346 - DNA, 189 bp, Bacteriophage D
atgaagaaattttggcatagcggtatgattgacaagaaggttattgaaaaacgtaaacaggaagaatgtattaatgaactgcataggactattcttgagttgaaaaatgagaagcatccagatatgatggattttatggacctgatagattggtatttagaaaatcgcaaaccacgagatatttattag

SEQ ID NO: 347 - DNA, 183 bp, Bacteriophage D
atgatcgacaagaaagttattgaaaaacgtaaacaggatgagtatttgaataaattacacaggactattcttgagttaaaaaatgagaagcatccagatatgatagattttatggacctgatagattttatggacctgatagattggtatttagagaatcgcaaaccacgagatattgattag

SEQ ID NO: 348 - DNA, 189 bp, Bacteriophage D
atgaataaattttggcatagcggtatgatcgacaagaaagttattgaaaaccgtaaacaggaagaatatattaataaactgcatagcactattcttgaattgaaaaatgagaagcatccagatatgatggattttatggacctgatagattggtatttagaaaatcgcaaaccacaagatattgattag

SEQ ID NO: 349 - DNA, 189 bp, Bacteriophage P
atgaagaaattttggcgtagtggcatgattgacaataaggttattgaaaaacgtaaacaagatgattatatgaataaattacacaggactattcttgagttgacccgtgaaattgaattgagacgtggcccagatatgatggatttcatggatctgatagattggtatttaaacagccgcaaaccgtag

SEQ ID NO: 350 - DNA, 216 bp, Bacteriophage D
atgaagaagttttggcatagcggtatgattgacaagaaagttattgaaaaacgccaacatgatgagtatataaataaaatacataagactattattgagttgaggaaagaaccacctgaacctaaaccttgctcttgtcacaaagatatagatattaatgctttgattaatgatattgagtgggatgattattatacatggtttaaagataaataa

SEQ ID NO: 351 - DNA, 216 bp, Bacteriophage D
atgaagaaattttggcgtagtggaatgattgacaagaaggttattgaaaaacgtaaacaagatgattatatgaataaattacacaggactattcttgagttgagtataaaaccacctgaacctaaaccttgctcttgtcacaaagatatagatattaatgctttgattaatgatattgagtgggatgattattatacatggtttaaagataaataa

SEQ ID NO: 352 - DNA, 216 bp, Bacteriophage D
atgaagaaattttggcgtagtggcatgattgacaagaaggttattgaaaaacgtaaacaggaagagtatatgaataagatgcataggactattcttgagttgagtataaaaccacctgaacctaaaccttgctcttgtcacaaagatatagatattaatgctttgattaatgatattgagtgggatgattattatacatggtttaaagataaataa

SEQ ID NO: 353 - DNA, 192 bp, Bacteriophage D
atgattgacaagaaggttattgaaaaacgtaaacaagatgattatatgaataaattacacaggactattcttgagttgagtataaaaccacctgaacctaaaccttgctcttgtcacaaagatatagatattaatgctttgattaatgatattgagtgggatgattattatacatggtttaaagataaataa

SEQ ID NO: 354 - DNA, 216 bp, Bacteriophage D
atgaagaaattttggcatagcggtatgattgacaagaaagttattaaaaaacgtaaacaggaagaatatatgaataaacttcaaagaattatccttgagttgagtataaaaccacctgaacctaaaccttgctcttgtcacaaagatatagatattaatgctttgattaatgatattgagtgggatgattattatacatggtttaaagataaataa

SEQ ID NO: 355 - DNA, 213 bp, Bacteriophage O
atgaagaagttttggcatagcggtatgattgacaagaaaattattgaaaaacgtgaacatgatgagtatttgaataaattacatatgactattattgagttgagaaaagaaccacctgaaactaaaccttgctcttgtcacaaaaatgtagatattaatgaattaattaactatattgagtggaatgattattatacatggtttaaagattaa

SEQ ID NO: 356 - DNA, 183 bp, Bacteriophage D
atgaagaaattttggcatagcggtatgatcgacaagaaagttattgaaaaacgtaaacaggatgagtatttgaataaattacacaggactattcttgagatagactttccaattcaacgtgtttgtcaccggtcactatcaccgacacccataacggtgcccacggaaacccttgatatataa

SEQ ID NO: 357 - DNA, 135 bp, Bacteriophage D
atgaagaaattttggcatagcggtatgattgacaagaaagttattaaaaaacgtaaacaggaagagtatatgaataagatgcataggactattcttgagttgagtataaaaccaatagaagaaatggttttttaa

SEQ ID NO: 358 - DNA, 267 bp, Bacteriophage Sfi
atgaagaaattttggcgtagtggaatgattgacaagaaggttattgaaaaacgtaaacaagatgattatatgaataaattacacaggactattcttgagttgagtataaaaccacctgaacctaaaccttgctcttgtcacaaagatatagatattaatgctttgattaatgatattgagtgggatgattgggtagatgaagtgttggaatatataaataaatgggtaaataaagataaagctgatgtggaggtattagataaatga

SEQ ID NO: 359 - DNA, 633 bp, Bacteriophage D
atgaccaccccacaaaagtttcttagtatcagggaattgcttaaaccactccctagcaacggtgttaagtttcctaagttctctgcactctatcacgaaagccaagtgggagcgtggcagaagaaaatgagtaagcgaagacaccaagcaaaggtacaagtagctatggataagaaccgtggtgaactagttcctcgtgagttagaggacttctctaactggcaacgtgctagacaaatgaaagcacgctatcaagagaaggtggctaacaagcgtaaggactacctacacaaactaaccacttatcttgttaagacttatgatgttatcgtgattgaggacttgaaagctaagaacttgatgaagaaccattacttagctaaatcaatcgctaacgcttcatggcatgagtttaagagactgctagaatacaagtgttcgtggtatggcaaggaacttattgttgttccggctcaccatactagtcaagagtgttctaactgtcaccacaattcaggtaagaaaccgctccatatccgtgagtggatgtgtgataattgtggtactcaccatgatagagacattaacgcaagtatcaatatcttgcaccgtggacttgccacgttaaattaa

SEQ ID NO: 360 - DNA, 303 bp, Bacteriophage D
atgtcaacagttttcttgattttttttcaagtttttttgattttattattaaacatcttgaaaattagtaaaacatactatatattgttctttgtatgtatccattgtttttacctcgtttttttattttttatcgaatgttttccaagttgctctcaatccattctagtctattttggcgaccagacggaaactgtttttataaaaaaatatatatttttttgcaaaacaaaaaccctgactaattcaagtcagggcaagagagagtttatcgaagactcagcttttaactgtatccattaa

SEQ ID NO: 361 - DNA, 303 bp, Bacteriophage D
atgtcaacagttttcttgattttttttcaagttttcttgatttttttattaaacatcttgaaaattagtaaaacatactatatattgttctttgtatgtatccattgtttttacctcgtttttttattttttatcgaatgttttccaagttgctctcaatccattctagtctattttggtgaccagacggaaactgtttttataaaaaaatatatatttttttgcaaaacaaaaaccctgactaattcaagtcagggtgagagagagtttatcgaagactcagcttttaactgtattcattaa

SEQ ID NO: 362 - DNA, 303 bp, Bacteriophage P
atgtcaacagttttcttgattttttttcaagttttcttgatttttttattaaacatcttgaaaattagtaaaacatactatatattgttctttgtatgtatccattgtttttacctcgtttttttattttttatcgaatgttttccaagttgctctcaatccattctagtctattttggtgaccagacggaaactgtttttataaaaaaatatatatttttttgcaaaacaaaaaccctgactaattcaagtcagggtgagagagagtttatcgaagataacagcttttactgtaaccattaa

SEQ ID NO: 363 - DNA, 231 bp, Bacteriophage P
ttgattttttttaaagtttttttgattttattattaaacaacttgaaaattagtaaaacatactatatattgttctttgtatgtatccattgtttttacctcgtttttttattttttatcgaatattttccagattgttttcaatccattcaagtcgatttttgcgaccagacggaaactgtttttataaaaaattatatattttttttgcaaaacaaaaaccctgactaa

SEQ ID NO: 364 - DNA, 246 bp, Bacteriophage P
atgtcaatagttttcttgattttttttaaagtttttttgattttattattaaacaacttgaaaattagtaaaacatactatatattgttctttgtatgtatccattgtttttacctcgtttttttattttttatcgaatattttccagattgttttcaatccattcaagtcgatttttgcgaccagacggaaactgtttttataaaaaaatatatattttttttgcaaaacaaaaaccctgactaa

SEQ ID NO: 365 - DNA, 234 bp, Bacteriophage P
atgtcaacagttttcttgattttttttcaagtttttttgatttttttatatatttactttaaaattagtaaaacatactatatattgttctttgtatgtatccattgtttttttattttttatcgaatgttttccaagttgctctcaatccattctagtctattttggcgaccagacggaaactgtttttataaaaaaatatatatttttttgcaaaacaaaaaccctgactaa

SEQ ID NO: 366 - DNA, 219 bp, Bacteriophage P
ttgattttttttcaagttttcttgatttttttattaaacatcttgaaaattagtaaaacatactatatattgttctttgtatgtatccattgttttttattttttatcgaatgttttccaagttgctctcaatccattctagtctattttggcgaccagacggaaactgtttttataaaaaaaatatatatttttttgcaaaacaaaaaccctgactaa

SEQ ID NO: 367 - DNA, 198 bp, Bacteriophage D
ttgtttatttttgggaactgttgtataatgtttatactatatatatcatgtatgatagtttgtcaacagttttacctaaattattttagttttttttgcaaaaaaagaaaacctcgactaaaagtcgaggttacagttcgagaatttaaccgaaacgataccaagtattccaacaattatattaccacttttctatga

SEQ ID NO: 368 - DNA, 189 bp, Bacteriophage D
gtgagttctgaacatagtattcaaaatcaaattcgagtggaattatccaaggctggcaacatggtatttagaattaacgttggtaaagtcagaatggctgatggacgttggtttgatactggagcaccaaaaggattttgtgacctgtttggatttagaccagctactgtaatagcacttatctattag

SEQ ID NO: 369 - DNA, 141 bp, Bacteriophage P
ttgccaatcctctttattgtcggtaacgcacagggagcaagtcactgcactagaccgaagcccttacatcccgccaccttagaggtgggggaattacgggctgttaggttaaaaaaagcaaacaaaaaagccccagcataa

SEQ ID NO: 370 - DNA, 171 bp, Bacteriophage P
atgtcaacagttttcttgattttttttcaagttttcttgatttttttattaaacatcttgaaaattagtaaaacatactatatattgttctttgtatgtatccattgtttttttattttttatcgaatgttttccaagttgctctcaatccattctagtctattttggtga

SEQ ID NO: 371 - DNA, 144 bp, Bacteriophage P
ttgattttttttcaagttttcttgatttttttattaaacatcttgaaaattagtaaaacatactatatattgttctttgtatgtatccattgttttttttattttttatcgaatgttttccaagttgctctcaatccattctag

SEQ ID NO: 372 - DNA, 171 bp, Bacteriophage P
ttggtcttagcccccaacaaaacgttcccttatgcttgtgtgtgcgcaagcaatagggcgctgaacctaatcagtcttttaccttttgcactagataaattgtatctaggttatccaattacattttatcaaattatcatttataagtcaaataaaaaagccccagcataa

SEQ ID NO: 373 - DNA, 198 bp, Bacteriophage P
ttgagaataaatgaagctgtactaagtttttatagtttttatttttatttattaaggaatttagtttttttttgcaaaaaaagaaaacctcgactaaaagtcgaggttacagttcgagaatttaaccgaaacgatgccaagtattccaacaattatatgaaaatagcaaacaaaaagagctacgagattatctcatag

SEQ ID NO: 374 - DNA, 195 bp, Bacteriophage Sequence
ttgttctacctattgactaaagcgagtttttacctctctctttatcttatgtatacattacatatcatatatgatagtctgccaactgtttttataaaaaaatatatatttttttgcaaaacaaaaaccctgactaattcaagtcagggtgagagagagtttatcgaagactcagcttttaactgtattcattaa

SEQ ID NO: 375 - protein, 108 aa, Bacteriophage O; identical to SEQ ID NO: 2

SEQ ID NO: 376 - protein, 140 aa, Bacteriophage Sfi; identical to SEQ ID NO: 4

SEQ ID NO: 377 - protein, 140 aa, Bacteriophage TPL; identical to SEQ ID NO: 6

SEQ ID NO: 378 - protein, 140 aa, Streptococcus sp; identical to SEQ ID NO: 8

SEQ ID NO: 379 - protein, 140 aa, Bacteriophage D; identical to SEQ ID NO: 10

SEQ ID NO: 380 - protein, 140 aa, Bacteriophage D; identical to SEQ ID NO: 12

SEQ ID NO: 381 - protein, 140 aa, Bacteriophage D; identical to SEQ ID NO: 14

SEQ ID NO: 382 - protein, 140 aa, Bacteriophage D; identical to SEQ ID NO: 16

SEQ ID NO: 383 - protein, 140 aa, Bacteriophage D; identical to SEQ ID NO: 18

SEQ ID NO: 384 - protein, 140 aa, Streptococcus mutans; identical to SEQ ID NO: 20

SEQ ID NO: 385 - protein, 140 aa, Streptococcus mutans; identical to SEQ ID NO: 22

SEQ ID NO: 386 - protein, 140 aa, Streptococcus mutans; identical to SEQ ID NO: 24

SEQ ID NO: 387 - protein, 140 aa, Streptococcus mutans; identical to SEQ ID NO: 26

SEQ ID NO: 388 - protein, 183 aa, Bacteriophage D; identical to SEQ ID NO: 28

SEQ ID NO: 389 - protein, 183 aa, Bacteriophage D; identical to SEQ ID NO: 30

SEQ ID NO: 390 - protein, 183 aa, Bacteriophage D; identical to SEQ ID NO: 32

SEQ ID NO: 391 - protein, 183 aa, Bacteriophage D; identical to SEQ ID NO: 34

SEQ ID NO: 392 - protein, 183 aa, Bacteriophage D; identical to SEQ ID NO: 36

SEQ ID NO: 393 - protein, 183 aa, Bacteriophage M; identical to SEQ ID NO: 38

SEQ ID NO: 394 - protein, 183 aa, Bacteriophage D; identical to SEQ ID NO: 40

SEQ ID NO: 395 - protein, 183 aa, Bacteriophage D; identical to SEQ ID NO: 42

SEQ ID NO: 396 - protein, 183 aa, Bacteriophage ALQ; identical to SEQ ID NO: 44

SEQ ID NO: 397 - protein, 183 aa, Bacteriophage D; identical to SEQ ID NO: 46

SEQ ID NO: 398 - protein, 183 aa, Bacteriophage; identical to SEQ ID NO: 48

SEQ ID NO: 399 - protein, 183 aa, Bacteriophage DT; identical to SEQ ID NO: 50

SEQ ID NO: 400 - protein, 183 aa, Bacteriophage D; identical to SEQ ID NO: 52

SEQ ID NO: 401 - protein, 183 aa, Bacteriophage N; identical to SEQ ID NO: 54

SEQ ID NO: 402 - protein, 183 aa, Bacteriophage D; identical to SEQ ID NO: 56

SEQ ID NO: 403 - protein, 183 aa, Bacteriophage D; identical to SEQ ID NO: 58

SEQ ID NO: 404 - protein, 183 aa, Bacteriophage CHPC; identical to SEQ ID NO: 60

SEQ ID NO: 405 - protein, 183 aa, Bacteriophage D; identical to SEQ ID NO: 62

SEQ ID NO: 406 - protein, 183 aa, Bacteriophage; identical to SEQ ID NO: 64

SEQ ID NO: 407 - protein, 183 aa, Bacteriophage; identical to SEQ ID NO: 66

SEQ ID NO: 408 - protein, 183 aa, Bacteriophage D; identical to SEQ ID NO: 68

SEQ ID NO: 409 - protein, 183 aa, Streptococcus thermophilus; identical to SEQ ID NO: 70

SEQ ID NO: 410 - protein, 183 aa, Streptococcus thermophilus; identical to SEQ ID NO: 72

SEQ ID NO: 411 - protein, 183 aa, Bacteriophage Sfi; identical to SEQ ID NO: 74

SEQ ID NO: 412 - protein, 183 aa, Bacteriophage Sfi; identical to SEQ ID NO: 76

SEQ ID NO: 413 - protein, 183 aa, Streptococcus thermophilus; identical to SEQ ID NO: 78

SEQ ID NO: 414 - protein, 183 aa, Bacteriophage D; identical to SEQ ID NO: 80

SEQ ID NO: 415 - protein, 183 aa, Bacteriophage D; identical to SEQ ID NO: 82

SEQ ID NO: 416 - protein, 183 aa, Streptococcus sp; identical to SEQ ID NO: 84

SEQ ID NO: 417 - protein, 183 aa, Streptococcus sp; identical to SEQ ID NO: 86

SEQ ID NO: 418 - protein, 104 aa, Bacteriophage D
MKKAKQLLKEIKTNNVSYAIMDEDNEIYCNKETNNIMDIYEYDNENGHFYGVYSDVVGGKVDSRYLSDEYILKAIDKLLNLGDPVKRTELPADADFKRTFFFEE

SEQ ID NO: 419 - protein, 104 aa, Bacteriophage D
MKKAQQLLKEIKNTNVSYAIMDEDNEIYCNKETNNIMDIYGYDNENGHFYGVYSDVVGGKVDSRYLSDEYILKAIDKLLFLGDPIKRTDLPSDADFKRTFFFEE

SEQ ID NO: 420 - protein, 96 aa, Bacteriophage P
MKNRLLGSRYTDAIKNDCGTANKMSNIYNKLNKDSLREIHSALYGLLTAGYDISNMRNIEDLEKYVNLKKSRGQLLNVSSDDIKLYHKLFVIRFEK

SEQ ID NO: 421 - protein, 92 aa, Bacteriophage CHPC
MKNKLYTDAIKNDSRTASKMANIYNKLESDTMREIHSALSGLLTAGYDISNMRNIEELEKYVTLKKSRGQLLNVSSEDIKLYHKLFVIRFGK

SEQ ID NO: 422 - protein, 98 aa, Bacteriophage D
MKNRLLGSRYTDAIKNDCGTANKMSNIYNKLNKDSLREIHSALYGLLTAGYDISNMRKIEELEKYVNLKKSRGQLLNVSSNDIKLYHKLFVIRFGKER

SEQ ID NO: 423 - protein, 94 aa, Bacteriophage D
MKNRLYTDAIKNDCGTANKMSNIYNKLNKDSLREIHSALYGLLTAGYDISNMRKIEELEKYVNLKKSRGQLLNVSSNDIKLYHKLFVIRFGKER

SEQ ID NO: 424 - protein, 92 aa, Bacteriophage D
MKNKLYTDAIKNDSATANKMANIYSKLNKDSLREIHSALSGLLTAGYDISNMQNIAELQKYVILKKSRGQLLNVSSKDIELYHKLFVIRFGK

SEQ ID NO: 425 - protein, 96 aa, Bacteriophage D
MKNRLLGSRYTDAIKNDCGTANKMSNIYNKLNKDSLREIHSALYGLLTAGYDISNMRKIEELEKYVNLKKSRGQLLNVSSNDIKLYHKLFVIRFGK

SEQ ID NO: 426 - protein, 94 aa, Bacteriophage D
MKNRLLGSRYTDAIKNDCGTANKMSNIYNKLNKDSLREIHSALYGLLTAGYDISNMRKIEELEKYVNLSRGQLLNVSSNDIKLYHKLFVIRFGK

SEQ ID NO: 427 - protein, 100 aa, Bacteriophage D
MKNRLLGSRYTDAIKNDSGTANKMSNIYNSVINKEGLRGIHSALYGLLTAGYDISNMRKIEELEKYVNLKKSRGQLLNVSSSDIKLYHKLFVIRFGKKLK

SEQ ID NO: 428 - protein, 98 aa, Bacteriophage D
MKNGNKILGYRYTDEIKNDSATENKMSNLYNKLDKDSLREIHSALYGLLTAGYDISNMRNVEELEKYVNVKKSHGKLLDVTNSDIQLYHKLFVVRFGK

SEQ ID NO: 429 - protein, 96 aa, Bacteriophage D
MKNRLLGSRYTDAIKNDCGTANKMSNIYNKLNKDSLREIHSALYGLLTAGYDISNMRNIEELEKYVNLKKSRGQLLNVSSSDIKLYHKLFVIRFGK

SEQ ID NO: 430 - protein, 97 aa, Bacteriophage N
MKNRLLGSRYTDAIKNDSGTANKMSNIYNSVINKEGLRGIHSALYGLLTAGYDISNMRKIEELEKYVNLKKSRGQLLNVSSSDIKLYHKLFVIRFGK

SEQ ID NO: 431 - protein, 97 aa, Bacteriophage N
MKNRLLGSRYTDAIKNDSGTANKMSNIYNSVINKEGLREIHSALYGLLTAGYDISNMRKIEELEKYVNLKKSRGQLLNVSSNDIKLYHKLFVTRFGK

SEQ ID NO: 432 - protein, 96 aa, Bacteriophage P
MKNRLLGSRYTDAIKNDSGTANKMSNIYNKLNKDSLREIHSALYGLLTAGYDISNMRNIEELEKYVNLKKSRGQLLNVTSNDIKLYHKLFVIRFGK

SEQ ID NO: 433 - protein, 96 aa, Bacteriophage P
MKNRLLGSRYTDAIKNDCGTANKMSNIYNKLNKDSLREIHSALYGLLTAGYDISNMRNIEELEKYVNLKKSRGQLLNVSSDDIKLYHKLFVIRFGK

SEQ ID NO: 434 - protein, 98 aa, Bacteriophage V
MKNGNKILGYRYTDEIKNDSATENKMSNLYNKLDKDSLREIHSALYGLLTAGYDISNMRNVEELEKYVNVKKSHGKLLDVTNSDIQLYHKLFVVRFGR

SEQ ID NO: 435 - protein, 128 aa, Bacteriophage D
MTEWKTINFNAQNIEYEAAKAILIKMPNNSEWHGYTFWHPSKCVRTLSKGNGYFKTFSYTENWEFTIFKSNKKGERTIEQVLTARDMEKAFSVVNEQIASNASTESYLEIEEPKKVDKTVSINNELKR

SEQ ID NO: 436 - protein, 128 aa, Bacteriophage D
MTEWKTINFNKQNIEHETAKAVLIKMPNNSEWYGYKFWHPSKCVRTLSKGNGYFKTFSYTENWEFTIFKSNKKGERTAEQILTAEDMEIAFDVVNEQISANASTESYLEIEEPKKVDKTVSINNELKR

SEQ ID NO: 437 - protein, 128 aa, Bacteriophage D
MTEWKTINFNAQNIEYEAAKAILIKMPNNSEWHGYTFWHPSKCVRTLSKGNGYFKTFSYTENWEFTIFKSNKKGERTAEQILTAEDMEIAFDVVNEQISVDASTESYLEIEEPKKVDKTVSINNELKR

SEQ ID NO: 438 - protein, 126 aa, Bacteriophage D
MWKSINFNAQNIEHETAKAVLIKMPNNSEWSGYKFWHPSKCVRTLSKGKGYFKIFSYTENWEFTIFKSNKKGERTAEQILTAEDMEIAFDVVNEQISANASTESYLEIEEPKKVDKTVSINNELKR

SEQ ID NO: 439 - protein, 126 aa, Bacteriophage D
MWKSINFNAQNIEHETAKAVLIKMPNNSEWSGYKFWHPSKFVRTLSKGKGYFKIFSYTENWEFTIFKSNKKGERTAEQILTAEDMEIAFDVVNEQISANASTESYLEIEEPKKVDKTVSINNELKR

SEQ ID NO: 440 - protein, 126 aa, Bacteriophage D
MWKSINFNAQNIEHETAKAVLIKMPNNSEWSGYKFWHSSKCVRTLSKGKGYFQSFSYTENWEFTIFKSNKKGERTAEQILTAEDMEIAFDVVNEQISANASTESYLEIEEPKKVDKTVSINNELKR

SEQ ID NO: 441 - protein, 128 aa, Bacteriophage D
MTEWKTINFNKQNIEHETVKAVLIKMPNNSEWYGYKFWHPSKCVRTLSKGNGYFKTFSYTENWEFTIFKSNKKGERTAEQILTAEDMEIAFDVVNEQISANASTESYLEIEEPKKVDKTVSINNELKR

SEQ ID NO: 442 - protein, 123 aa, Bacteriophage D
MWKSIKFNAQNIKFETAKAVLIKMPNKSRYAGYMFWHPLKLVRVEGGKGYFMSFSYTDDFEFKVFKQGKNRQITAESILSHEEIEEAFEIVNEQLSYMDECYLEVTEPTKIDKEVEVKEELRK

SEQ ID NO: 443 - protein, 123 aa, Bacteriophage D
MWKSIKFNAQNIKFETAKAVLIKMPNKSRYAGYMFWHPAKLVRVVGGKGYFMSFSYTDEFEFKIFKQGKNRQITVEKILSPEEIEDAFEVVNEQLSDIDECYLEVTEPTKINDKVEIRAELRK

SEQ ID NO: 444 - protein, 123 aa, Bacteriophage D
MWKSIKFNAQNIKFETAKAVLIKMPNKSRYAGYMFWHPSKLVRVEGGKGYFMSFSYTDDFEFKVFKQGKNRQITAESILSHEEIEEAFEIVNEQLSYMDECYLEVTEPTKIDKEVEVKEELRK

SEQ ID NO: 445 - protein, 123 aa, Bacteriophage D
MWKSIKFNAQNVKFETANSVLIKMPNKSSYAGYMFWHPAKLVRVLGGKGYFLSFSYTDEFEFKVFKQGKNRQITAEAILSHEEMEDAFEIVNEHLSYTDECYLEVAEPTKIDKEVEIREELRK

SEQ ID NO: 446 - protein, 59 aa, Bacteriophage D
MKVYYNLADSGLFKEIKKQLALDDAENGDLIHTTEDNEASDGTKIVAIWNANRQNYFIK

SEQ ID NO: 447 - protein, 145 aa, Bacteriophage D
MRNDFINKVYDELNQIINHWAKQKYLSDKIFEYTNTFSIKKVYGLYWEVKILCKNDYRILLRFYKNYEWYNDSNILNVSVLAPAVERVKNEDGSVDVYPSKIIKDKIEFIEGDFDIDGDDWVDEVLEYINKWVNKDKADVEVLDK

SEQ ID NO: 448 - protein, 145 aa, Bacteriophage D
MRNDFINKVYDELNQIINHWAKQKYLSDKIFEYTNTFSIKKVYGLYWEVKILCKNDYRILLRFYKNYEWYNDSNILNVSVLAPAVERVKNEDGSVDVYPSKKIKDKIEFIEGDFDIDGDDWVDEVLEYINKWVNKDKADVEVLDK

SEQ ID NO: 449 - protein, 145 aa, Bacteriophage D
MRNDFINKVYDELNQIINHWAKQKYLSDKIFEYTNTFSIKKVYGLYWEVKILCKNDYRILLRFYKNYEWYNDSNILNVSVLAPAVERVKNEDGSVDVYPSKKIKDKIEFIEGNFDIDGDDWVDEVLEYINKWVNKDKADVEVLDK

SEQ ID NO: 450 - protein, 121 aa, Bacteriophage D
MRNDFINKVYDELNQIINHWAKQKYLSDKIFEYTNTFSIKKVYGLYWEVKILCKNDYRILLRFYKNYEWYNDSNILNVSVLAPAVERVKNEDGSVDVYPSKKLKIKLNLLKVILILMEMIG

SEQ ID NO: 451 - protein, 145 aa, Bacteriophage D
MRNDFINKVYDELNQIINHWAKQKYLSDKIFEYTNTFSIKKVYGLYWEVKILCKNDYRILLRFYKNYEWYNDSNILNVSVLAPAVERVENEDGSVDVYPSKIIKDKIEFIEGDFDIDGDDWVDEVLEYINKWVNKDKADVEVLDK

SEQ ID NO: 452 - protein, 145 aa, Bacteriophage D
MRNDFINKVYDELNPIINHWAKQKYLSDKIFEYTNTFSIKKVYGLYWEVKILCKNDYRILLRFYKNHEWYNDSNILNVSVLAPAVERVKHEDGSVDVYPSKIIKDKIEFIEGDFDIDGYDWVDEVLEYINKWVNKDKDDVEVLDK

SEQ ID NO: 453 - protein, 145 aa, Bacteriophage O
MRNDFINKVYDELNQIINHWAKQKYLSDKIFEYTNTFSIKKVYGLYWEVKILCKNDYRILLRFYKNYEWYNDSNILNVSVLAPAVERVKNEDGSVDVYPSKIIKDKIEFIEGNFDIDGDDWVDEVLEYINKWVNKDKADVEVLDK

SEQ ID NO: 454 - protein, 105 aa, Bacteriophage D
MKNFKISSTYRAARKQQKTANRKSFYNDEGYMISPSEWADGVIKGLINPKNSWSNDHVKGYLPRVSPRSHWTKNGYREYLGIGKSRDIPEKEPEVIEMMDLELVP

SEQ ID NO: 455 - protein, 105 aa, Bacteriophage P
MKNFKISSTYRAARKQQKTANRKSFYNDEGYMISPSEWVDGVIKGLINPKNSWSNDHVKGYLPRVSPRSHWTKNGYREYLGIGKSRDIPEKEPEVIEMMDLELVP

SEQ ID NO: 456 - protein, 105 aa, Bacteriophage Proph
MKNFKISSTYRAARKQQKTANRKSFYNDEGYMISPSEWADGVIKGLINPKNSWSNDHVKGYLPRVSPRSHWTKNGYREYLGIGKSRDIPKKEPEVIEMMDLELVP

SEQ ID NO: 457 - protein, 128 aa, Bacteriophage D
MKYDKSGIMKEAWNLFNNDDITFADFEYLTREERQGKKTFTLCLKEAWAHEKEIVDSIKKDHADAEHSVEAKAWDWACKKLGVSIEMDAYTKFVNVNDMKKEAWPGTSVWSLAMRAVKLHIKLFGQVA

SEQ ID NO: 458 - protein, 173 aa, Bacteriophage D
MNGLKTILKTFDKNIYFLTKSVDIRQHRRYNIYVKLREEVNDMKKSTYDKSGIMKEAWNLFNNDDITTADFEYLTRGELQEGKTFAICLKEAWAHEKDIVESLNEDYENAEHSVQAKAWDWACKKLGVSIEVDAYTKLVNVNDMQKESWPGTSAWSLAMRAVKLHIKLFGQAA

SEQ ID NO: 459 - protein, 173 aa, Bacteriophage D; identical to SEQ ID NO: 458

SEQ ID NO: 460 - protein, 111 aa, Bacteriophage
MKKEVMTNAWKIAKEAVKKFGGKAIEYIAEALKMAWAAAKGGNASLAKFQAVESKMRKAGKYSMIQVLNFAKEVKFNEVMHKVGAYYGIEVVADGDSIGTYYIAEKVWDAA

SEQ ID NO: 461 - protein, 111 aa, Bacteriophage P
MKKEIMTKAWKIAKEAVKTFGGKAIEYIAGAMKMAWAAIKDNGTSLAKFQAVEAKMRKAGKYSMIQVLDFAKEVRFNEVMHKVGAYYGIEVIADGDSIGTYYIAENVWNAA

SEQ ID NO: 462 - protein, 111 aa, Bacteriophage CHPC
MKKEIMTKAWKIAKNASTKFGGKAIEYIAGAMKMAWAAIKENGTSLAKFQAVEAKMRKAGKHSMVQVLNFAKEVKFNEVMHKVGAYYGIEVIADGDSIGTYYIAEKVWNAA

SEQ ID NO: 463 - protein, 111 aa, Bacteriophage D
MKKEIMTKAWKIAKEAVEKFGGKAIEYIAGAMKMAWAAAKAGNTSVAKFQAVEDKMRKAGKYSMIQVLNFANEVKFNEVMHKAGAYYGIEVIADGDSIGTYYIAEKVWEVA

SEQ ID NO: 464 - protein, 108 aa, Bacteriophage D
MKKEVMTNAWEIAKNASKKFGGKAIEYIAGAMKMAWAAAKGGLAKFQAVESKMRKAGKHSMVQVLNFAKEVKFNEVMHKAGAYYGIEVIADGDSIGTYYISEKVWEVA

SEQ ID NO: 465 - protein, 111 aa, Bacteriophage D
MKKEIMTKAWKIAKEAVKTFGGKAIEYIAGAMKMAWAAAKAGNTSLAKFQAVESKMRKAGKYSMIQVLNFAKEVKFNEVMHKVGAYYGIEVIADGDSIGTYYIAESVWEVA

SEQ ID NO: 466 - protein, 111 aa, Bacteriophage D; identical to SEQ ID NO: 463

SEQ ID NO: 467 - protein, 105 aa, Bacteriophage D
MKKEIMTKAWKIAKEAVKTFGGKAIEYIAEAMKMAWAAAKGGLAKFQAVESKMRKAGMIQVLNFAKEVKFNEVMHKVGAYYGIEVIADGDSIGTYYIAESVWEVA

SEQ ID NO: 468 - protein, 111 aa, Bacteriophage D
MKSQVMSLAWKIAKNASTKFGGKAIEYIARAMKMAWSAIKENGTSLAKFQAIEAKIRKAGKHSMVQVLKFAKEVKFNEVMHKVGAYYGIEVIADGDSIGTYYIAEKVWDAA

SEQ ID NO: 469 - protein, 111 aa, Bacteriophage D
MKKEIMKKAWKIAKEAVKKFGGKAIEYIAEALKMAWADAKGGNTSLAKFQAVEEKMRKAGKYSMIQVLNFAKEVKFNEVMHKVGAYYGIEVIADGDKIGTYFIAEKVWDAA

SEQ ID NO: 470 - protein, 111 aa, Bacteriophage D
MKKELMKDAWEIAKNASKKFGGKAIEYIAGAMKMAWAAAKAGNTSVAKFQAVEAKMRKAGKHSMIQVLDFAKEVKFNEVMHKVGAYYGIEVVADGDSIGTYYIAEKVWDVA

SEQ ID NO: 471 - protein, 111 aa, Bacteriophage D
MKKEVMTNAWKIAKEAVKKFGGKAIEYISEAMKMAWAAAKGENTSLAKFQAVEEKMRKAGKYSMIQVLDFAKEVKFNEVMHKVGAYYGIEVIADGDNIGTYYIAEKVWEVA

SEQ ID NO: 472 - protein, 106 aa, Bacteriophage D
MTNAWKIAKEAVKKFGGKAIEYISEAMKIAWADAKEGNTSVAKFQAVEAKMRKAGKHSMVQVLNFAKEVKFNEVMHKVGAYYGIEVIADGDSIGTYYISEKVWEVA

SEQ ID NO: 473 - protein, 111 aa, Bacteriophage D
MKKEIMTKAWKIAKEAVKTFGGKAIEYIAEAMKMAWAAAKGGNASLAKFQAVESKMRKAGKYSMIQVLNFAKEVKFNEVMHKVGAYYGIEVIADGDSIGTYYIAESVWEVA

SEQ ID NO: 474 - protein, 108 aa, Bacteriophage D
MKKEIMTKAWKIAKEAVKTFGGKAIEYIAEAMKMAWAAAKGGLAKFQAVESKMRKAGKYSMIQVLNFAKEVKFNEVMHKVGAYYGIEVIADGDSIGTYYIAESVWEVA

SEQ ID NO: 475 - protein, 111 aa, Bacteriophage D
MKKEIMKKAWEIAKEAVKKFGGKAIEYIAEALKMAWSDAKGSNTSLAKFQAVEEKMRKAGKYSMIQVLDFAKEVKFNEVMHKEGAYYGIEVVADGDSIGTYYIAEKVWEVA

SEQ ID NO: 476 - protein, 111 aa, Bacteriophage D
MKKEIMTKAWEIAKNASKKFGGKAIEYIAGAMKMAWAAAKAGNTSVAKFQAVEAKMRKAGKHSMVQVLNFAKEVKFNEVMHKVGTYYGIEVVADGDSIGTYYIAEKVWDAA

SEQ ID NO: 477 - protein, 111 aa, Bacteriophage D
MKKEIMTKAWEIAKNASKKFGGKAIEYIAGAMKMAWAAAKAGKTSVAKFQAVEAKMRKAGKHSMVQVLNFAKEVRFNEVMHKAGAYYGIEVIADGDSIGTYFIAENVWNAA

SEQ ID NO: 478 - protein, 111 aa, Bacteriophage D
MKKEIMTKAWKIAKEAVKTFGGKAIEYIAEALKMAWAAAKGENTSLAKIQAVEEKMRKSGKYSMIQVLDFAKEVKFNEVMHKAGAYYGIEVIADGDSIGTYYIAEKVWEVA

SEQ ID NO: 479 - protein, 111 aa, Bacteriophage D
MKKEIMTKAWKIAKEAVKTFGGKAIEYIAEAMKMAWAAAKGGNASLAKFQAVESKMRKAGKYSMIQVLNFAKEVKFNEVMHKVGAYYGIEVIADGDSIGTYYIAENVWNAA

SEQ ID NO: 480 - protein, 111 aa, Bacteriophage D
MKKEIMTKAWKIAKEAVEKFGGKSIEYIAEAMKMAWAAAKGGNASLAKFQAVEAKMRKAGKYSMIQVLNFAKEVKFNEVMHKAGAYYGIEVVADGDSIGTYYIAEKVWEVA

SEQ ID NO: 481 - protein, 111 aa, Bacteriophage N; identical to SEQ ID NO: 476

SEQ ID NO: 482 - protein, 111 aa, Bacteriophage O
MKSQVMSQAWKIAKEAVKKFGGKAIEYISEAMKMAWAAAKGENTSLTKFQAVEEKMRKAGKYSMIQVLDFAKEVKFNEVMHKVGAYYGIEVIADGDSIGTYFIAEKVWDVA

SEQ ID NO: 483 - protein, 111 aa, Bacteriophage P
MKKEIMKKAWKIAKEAVKKFGGKAIEYIAEALKMAWSDAKGSNTSLAKFQAVEEKMRKAGKYSMIQVLDFAKEVKFNEVMHKAGAYYGIEVIADGDSIGTYYIAEKVWEVA

SEQ ID NO: 484 - protein, 111 aa, Bacteriophage P
MKKEIMTKAWEIAKNASKKFGGKAIEYIAGAMKMAWAAAKAGNTSVAKFQAVEAKMRKAGKHSMVQVLNFAKEVKFNEVMHKVGAYYGIEVVADGDSIGTYYIAEKVWEVA

SEQ ID NO: 485 - protein, 111 aa, Bacteriophage P
MKKEIMTNAWEIAKNASKKFGGKAIEYIAEALKMAWSDAKGSNTSLAKFQAVEEKMRKAGKYSMIQVLNFAKEVKFNEVMHKEGAYYGIEVVADGDSIGTYYIAEKVWDAA

SEQ ID NO: 486 - protein, 111 aa, Bacteriophage SFi
MKKEVMTNAWKIAKEAVKKFGGKAIEYISEAMKMAWAAAKGENTSLAKFQAVEEKMRKAGKYSMIQVLDFAKEVKINEVMHKVGAYYGIEVIADGDNIGTYYIAEKVWEVA

SEQ ID NO: 487 - protein, 111 aa, Bacteriophage Sfi
MKKEVMTNAWKIAKEAVKKFGGKAIEYISEGYEMAWAAAKGENTSLAKFQAVEEKMRKAGKYSMIQVLDFAKEVKFNEVMHKVGAYYGIEVIADGDNIGTYYIAEKVWEVA

SEQ ID NO: 488 - protein, 111 aa, Bacteriophage Sfi; identical to SEQ ID NO: 475

SEQ ID NO: 489 - protein, 110 aa, Bacteriophage Sfi
MKKIMTNAWKIAKEAVKKFGGKAIEYISEAMKIAWADAKEGNTSVAKFQAVEAKMRKAGKHSMVQVLNFAKEVKFNEVMHKVGAYYGIEVIADGDSIGTYYISEKVWEVA

SEQ ID NO: 490 - protein, 111 aa, Bacteriophage Proph
MKKEIMKKAWKIAKEAVKKFGGKAIEYIAEALKMAWSDAKGSNTSLAKFQAVEDKMNKTGKHSMVQVLNFAKEVNFKEVMHKVGAYYGIEVVADGDSIGTYYIAEKVWDAA

SEQ ID NO: 491 - protein, 36 aa, Bacteriophage D
MKKEVMTNAWEIAKNASKKFGGKAIEYIAENVWNAA

SEQ ID NO: 492 - protein, 114 aa, Bacteriophage D
MKSQVMSLAWKIFKNEKNDVTFSEALKFAWKAVKRQNMADDFYFFHSSNVKFQGVKKWFAEKEFRGRNKKDLAFMSVSAISVKGLVEETDKAVKLEIVTPYGVSAKWYPKSVIA

SEQ ID NO: 493 - protein, 114 aa, Bacteriophage D
MKSQVMSLAWKIFKNEKNDVTFSEALKFAWKAVKRQNMADDFYFFRSSNVKFQGVKKWFAEKEFRGRNKKDLAFMSVTAISVKGLIEETDKAVKLEIVTPYGVSTKWYPKSVIA

SEQ ID NO: 494 - protein, 114 aa, Bacteriophage D
MKSQVMSLAWKIFKNEKNDVTFSEALKFAWKAVKRQNMADDFYFFRSSNVKFQGVKKWFAEKEFRGRNKKDLAFMSVTAISIKGLVEETDKAVKLEIVTPYGISTKWYPKSVIA

SEQ ID NO: 495 - protein, 114 aa, Bacteriophage Proph; identical to SEQ ID NO: 493

SEQ ID NO: 496 - protein, 114 aa, Bacteriophage Proph; identical to SEQ ID NO: 494

SEQ ID NO: 497 - protein, 86 aa, Bacteriophage
MKTMDAYKEQFQELQEYAFNVLREYPLDKTAVNVLSALVNSKKKDRIEFFKLNKGEDAMKVYYNLADSGTIEKYLETSAFLDYINE

SEQ ID NO: 498 - protein, 83 aa, Bacteriophage D
MDTYKEQFQKLQEYAFNVLREYPLDKTAVNVLSALVNSKKKDRIEFFKLNKGEDAMKVYYNLADSGTIEKYLETSAFLEYINE

SEQ ID NO: 499 - protein, 83 aa, Bacteriophage D
MDTYKEQFQELQEYAFNVLREYPLDKTAVNVLSALVNSKKKDRIEFFKLNKDEDAMKVYYNLADSGTIEKYLETSAFLEYINE

SEQ ID NO: 500 - protein, 83 aa, Bacteriophage D
MDTYKEQFQELQEYAFNILREYPLDKTAVNVLSALVNSKKKDRIEFFKLNKDEDAMKVYYNLADSGTIEKYLETSAFLEYINE

SEQ ID NO: 501 - protein, 83 aa, Bacteriophage D
MDTYKEQFQKLQEYAFNVLREYPLDKTAVNVLSALVNSKKKDRIEFFKLNKGEDAMKVYYNLADSGTIEKYLETSAFLEYTNE

SEQ ID NO: 502 - protein, 83 aa, Bacteriophage Sfi; identical to SEQ ID NO: 500

SEQ ID NO: 503 - protein, 83 aa, Bacteriophage Proph
MDTYKEQFQELQEYAFNVLREYPLDKTAVNVLSALVNSKKKDRIEFFKLNKGEDAMKVYYNLADSGTIEKYLETSAFLEYINE

SEQ ID NO: 504 - protein, 83 aa, Bacteriophage Proph
MDTYKEQFQELQEYAFNVLREYPLDKTAVNVLSALVNSKKKDRIEFFKLNKGEDAMKVYYSLADSGTIERYLEVCGFLEYINE

SEQ ID NO: 505 - protein, 93 aa, Bacteriophage D
MITKEQLKEYYSEHLEELVEWADDINKICLFAYLDEDDNLYCGINQLSYTQFRVPIQAEVTVDDDWNYDFFKNPAAYDGWDETLEEMLEELND

SEQ ID NO: 506 - protein, 93 aa, Bacteriophage D; identical to SEQ ID NO: 505

SEQ ID NO: 507 - protein, 93 aa, Bacteriophage D
MITKEQLKEYYSEHLEELVEWADDINKICLFAYLDEDDNLYCGINQLSYTQFRVPIQAEVTVDDDWNYDFFNNPASYDGWDETLEEMLEELND

SEQ ID NO: 508 - protein, 46 aa, Bacteriophage D
MKTMDTYKEQFYYLDPIYISVDINRRTFILGKRGQSLSFFYCNKTI

SEQ ID NO: 509 - protein, 74 aa, Bacteriophage O
MTQIKDGWHMVYDEKVYVESGKVVRGITKDNNNSEIACYPYEYNKDYDCWINISGKVTLSAYRSGRKKGTKCMK

SEQ ID NO: 510 - protein, 74 aa, Bacteriophage Sfi
MTQIKDGWHIVYDEKVYVESGKVVRGITKDNNNSEIACYPYEYNEDYDCWINISGKVTLSAYRSGRKKGTKCMK

SEQ ID NO: 511 - protein, 50 aa, Bacteriophage D
MFECLASFRLNSRTVTSTFCRGFLFLQKNLNSFIKSVDKLSYMIYNVYIR

SEQ ID NO: 512 - protein, 63 aa, Bacteriophage D
MNESELLEQFCVSLCEFSSRQWPRDGFLDPINRVVYINRDLPTERRLKVLLHELGHLEHDPKH

SEQ ID NO: 513 - protein, 49 aa, Bacteriophage D
MLGAKTTLFDIIYLYQWLPTHTRRYVLREVFYLLCFDRNATILMDTVKS

SEQ ID NO: 514 - protein, 49 aa, Bacteriophage D
MLGVKTTLFDIIYLYQWLPTHTRRYVLREVFYLLCFDRNATILMDTVKS

SEQ ID NO: 515 - protein, 45 aa, Bacteriophage
MRRCLFFGLLKKRNNGIIIFATTNPLQPHGQIRSDAGLFLFALFL

SEQ ID NO: 516 - protein, 140 aa, Bacteriophage
MKINTTRVKMVLKNEAIPADYLESEIGISRSVVEKVREDESEFKNLTLDFVAKIQKWIDDGNYTFSYDYSDLIEELEEDIAEGLTDEYIYVVRGQYNEILEKCPIIDYYYTSEEIEEGDLAEKTLTASALSEMKQDNEIF

SEQ ID NO: 517 - protein, 140 aa, Bacteriophage D
MKINTTRVKMVLKNKVIPAIYLENELGISRSVIEKVRDGERKIENLTLETIIKVQKWIDSGKYTFSYDYSDLIEELEEDIAEGLVDEYIYVVRGPYNELLDKCPIIDYYYTSEEIEEGDLAEKTLTASVLAEMKKDNEIF

SEQ ID NO: 518 - protein, 140 aa, Bacteriophage D
MKINTTRIKMVLKNEAIPAIYLENELGISRSVIEKVREDESEFKNLTLDVVAKIQKWIDDGNYTFSYDYSEFIEELEEDLAEGLIDDYLFVVRGDYDEALGKCPIIDYYYTSEEIEEGDLAEKTLTASVLAEMKKDNGIF

SEQ ID NO: 519 - protein, 140 aa, Bacteriophage D
MKINTTRVNMVLKNEAIPADYLENVIGISRSVIERVREDESGFKNLTLDVIAKIQKWIDEGNYTFSYDYSDLIEELEEDIAEGLVDEYIYVVRGPYNEILEKCPIIDYYYTSEEIEEGDLAEKTLTASALAEMKLDNKIF

SEQ ID NO: 520 - protein, 140 aa, Bacteriophage D
MKINTTRVNMVLKNKAIPANYLEKELGINRSTITRVRNGERKLENLTLETIIKVQKWIDSGKYTFSYDYSDLIEELEEDIEEGLTDEYIYVVRGPYNELLEKCPIIDYYYTSEEIEEGDLTEKTLTASALAEMKQDNEIF

SEQ ID NO: 521 - protein, 140 aa, Bacteriophage O
MIINTARVELVLMNKAIPANYLESEIGISRSAITRVRNDERKIENLKLETIIKVQKWIDSGKYTFSYDYSDLIEELEEDIAKGLAGKYIYVVRGPYNEILEKCPIIDYYYTSEEIEEGELAEKTLTASVLAEMKSDNEIF

SEQ ID NO: 522 - protein, 131 aa, Bacteriophage Proph
MVLKNEAIPADYLESEIGISRSVVEKVREDESEFKNLTLDVVAKIQKWIDDGNYTFSYDYSDLIEELEEDIAEGLVDEYIYVVRGPYNELLEKCPIIDYYYTSEEIEEGDLAEKTLITSVLAEMKSDNKIF

SEQ ID NO: 523 - protein, 140 aa, Bacteriophage Sfi
MIINVARVETVLMNNAIPANYLEREIGISRSAITRVRNGERKIENLKLETIIKVQKWIDSGKYTFSYDYSDLIEELEEDIAEGLTDEYIYVVRGAYNEILEKCPIIDYYYTSEEIEEGDLAEKTLTASALSEMKQDNEIF

SEQ ID NO: 524 - protein, 140 aa, Bacteriophage TPL
MIINTARVELVLMNKAIPANYLEREIGISRSAITRVRNGERKLENLTLETIMTIQKWIDEGNYRFSYDYSELIEDLEEDIAEGLTDEYIYVVRGPYNELLEKCPIIDYYYTSEEIEEGNLAEKTLTASVLAEMKQDNEIF

SEQ ID NO: 525 - protein, 140 aa, Bacteriophage TPJ
MKINTTRIKMVLKNEAIPAIYLENELGISRSIIEKVRDDESEFKNLTLETIIKIQSLINSGKYTFSYDYSDLIEELEEDIAEGLTDEYIYVVRGPYNEILEKCPIIDYYYTSEEIEEGNLAEKTLTASVLAEMKQDNEIF

SEQ ID NO: 526 - protein, 140 aa, Bacteriophage Proph
MKINTTRVKMVLKNEVIPAIYLENELGISRSVIEKVRDGERKIENLTLETIIKIQKWIDDGNYTFSYDYSDLIEELEEDIAEGLVDEYIYVVRGPYNELLEKCPIIDYYYTSEEIEEGDLAEKTLITSVLAEMKSDNKIF

SEQ ID NO: 527 - protein, 60 aa, Bacteriophage D
MDQVKLVLMNKAIPANYLERQTGVSRSAITRVRNGERKIENLTLETIIKIQSWIDSENTI

SEQ ID NO: 528 - protein, 64 aa, Bacteriophage D
MIINVDRVKAVLMDKSIPANYLEMQTGISRSAITRVRNGERKIENLTIGTIIKIQSWLDRRMIR

SEQ ID NO: 529 - protein, 60 aa, Bacteriophage D
MDRVKLVLMNKAIPANFLERQTGVSRSAITRVRNNERKIENLTLETIIKIQSWIDSDNTI

SEQ ID NO: 530 - protein, 75 aa, Bacteriophage D
MGRRIRIKIKIMIINMDQVKLVLMNKDIPANFIERQTGVSRSAITKVRNGERKIENLRLETIIKIQSWIDSGNTI

SEQ ID NO: 531 - protein, 71 aa, Bacteriophage D
MGSRIRIMIINVDRVKAVLMDKSIPANYLEMQTGISRSAITRVRNGERKIENLTIGTIIKIQSWLDRRMIR

SEQ ID NO: 532 - protein, 64 aa, Bacteriophage D
MIINMDRVKLVLMNKDIPANFLERQTGVSRSAITKVRNGERKIENLTLETIIKIQSWLDSENTI

SEQ ID NO: 533 - protein, 64 aa, Bacteriophage D
MIINTARVELVLMNKAIPANFLERQTGVSRSAITRVRDGERKIENLTLETIIKIQSWIDSDNKI

SEQ ID NO: 534 - protein, 71 aa, Bacteriophage D
MTKRIKTMIINMDRVKLVLMKKDIPANFLERQTGVSRSAITRVRNGERKIENLTLETIIKIQSWIDSENTI

SEQ ID NO: 535 - protein, 64 aa, Bacteriophage D
MIINTARVELVLMNKAIPANYLERQTGVSRSAITRVRNGERKIENLTLETIIKIQSWIDSDNKI

SEQ ID NO: 536 - protein, 64 aa, Bacteriophage P
MIINVDRVKAVLMDKSISANYLEIETGISRSAITRVRNGERKIENLTIGTIIKIQSWLDRRMIR

SEQ ID NO: 537 - protein, 170 aa, Bacteriophage D
MVVKIKRIVWVKNNGFEIRERELDCYFKNDGSYKKSSGDWESRCYEQFGDEFQLIRDSKALESYSGLTRDYQKDLKILRKYKHRDMTISEYEAMKYVVENWTKEWSQSPYSYSFYSSKNIDWGYKPEGSLRISDHWNFGENGEHCPTAEPVDGWAVCKFENGKYHLIKKF

SEQ ID NO: 538 - protein, 170 aa, Bacteriophage D
MVVKIKRIVWVKNNGFEIRERELDCYFKNDGSYKKSSGDWESRCYEQFGDEFQLIRDSKALESYSGLTRDYQKDLKILRKYKHRDMTISEYEAMKYVVENWTKEWSQSPYSNSFYSSKDIDWGYKPEGSLRVSDHWNFGENGEHCPTAEPVDGWAVCKFENGKYHLIKKF

SEQ ID NO: 539 - protein, 157 aa, Bacteriophage D
MVVKIKRIVWVKNNGFEIRERELDCYFKNDGSYKKSSGDWESRCYEQFGNKLQLIKDSKKLESYNGLTKDYQKDLKILRKCGRSEMNATEYEAMKYVEENWTKEWSQSPYSNSFYSSKDIDWGYKPEGSLRVSDHWNFGENGEHCPTAEPVDGWAVF

SEQ ID NO: 540 - protein, 170 aa, Bacteriophage D; identical to SEQ ID NO: 538

SEQ ID NO: 541 - protein, 170 aa, Bacteriophage D
MVVKIKRIVWVKNNGFEIRERELDCYFKNDGSYKKSSGDWESRCYEQFGDEFQLIRDNKALESYSGLTRDYQKDLKILRKYKHRDMTISEYEAMKYVVENWTKEWSQSPYSNSFYSSKDIDWGYKPEGSLRVSDHWNFGENGEHCPTAEPVDGWAVCKFENGKYHLIKKF

SEQ ID NO: 542 - protein, 170 aa, Bacteriophage D; identical to SEQ ID NO: 541

SEQ ID NO: 543 - protein, 74 aa, Bacteriophage D
MIKTEMIDDILTLIEEIEAVSDKNKEKFIEKFDELETNLQALNKQTTDDLVEILQEDYSDNWVAKEVIELVTNS

SEQ ID NO: 544 - protein, 74 aa, Bacteriophage D
MNKIEMIDDILTLIEEIDAISDKSKETFFEKIDELETNLQALNRQITDELVEILQEDYSDNWVAKEVIELVTNS

SEQ ID NO: 545 - protein, 74 aa, Bacteriophage D
MIKTEMIDDILTLIEEIEAVSDKNKEKFIEKFDELETNLQALNKQTTDDLVEILQEDYSDNWVAKEVIELVDDY

SEQ ID NO: 546 - protein, 74 aa, Bacteriophage D; identical to SEQ ID NO: 545

SEQ ID NO: 547 - protein, 170 aa, Bacteriophage D
MSYTSPVYNIKRVPIDKIQANSYNPNHVAPPEMKLLYKSILEDGYTMPIVCYYLKDEDKYEIVDGFHRYSTMLNHKDIYEREGGCLPVSVIDKPISDRMASTIRHNRARGSHDIDLMTNIVADLVDSGMSDAWILKNIGMDADELLRLKQLTGLASLFADKEFSKSWDVE

SEQ ID NO: 548 - protein, 170 aa, Bacteriophage D
MSYTSPVYNIKRVPIDKIQANSYNPNHVAPPEMKLLYKSILEDGYTMPIVCYYLKDEDKYEIVDGFHRYSTMLNHKDIYEREGGCLPVSVIDKPISDRMASTIRHNRARGSHDIDLMTNIVADLVDSGMSDAWILKNIGMDADELLRLKQLTGLSSLFADKEFSKSWDVE

SEQ ID NO: 549 - protein, 170 aa, Bacteriophage D
MSYTSPVYNIKRVPIDKIQANSYNPNHVAPPEMKLLYKSILEDGYTMPIVCYYLKDEDKYEIVDGFHRYSTMLNHKDIYDREGGCLPVSVINKPISDRMASTIRHNRARGSHDIDLMTNIVADLVDSGMSDAWILKNIGMDADELLRLKQLTGLASLFADKEFSKSWDVE

SEQ ID NO: 550 - protein, 170 aa, Bacteriophage D; identical to SEQ ID NO: 547

SEQ ID NO: 551 - protein, 170 aa, Bacteriophage D
MSYTSPVYNIKRVPIDKIQANSYNPNHVAPPEMKLLYKSILEDGYTMPIVCYYLKDEDKYEIVDGFHRYSTMLNHKDIYDREGGCLPVSVINKPISDRMASTIRHNRARGSHDIDLMTNIVADLVDSGMSDAWILKNIGMDADELLRLKQLTGLASLFADKEFSKSWIVE

SEQ ID NO: 552 - protein, 170 aa, Bacteriophage D; identical to SEQ ID NO: 547

SEQ ID NO: 553 - protein, 59 aa, Bacteriophage D
MPKVSESKRKANDKWDKKNKERKQYINRRSVARNFIKNMEGEDIPEFKKLIEERASKIK

SEQ ID NO: 554 - protein, 59 aa, Bacteriophage D
MPKVSESKRKANDKWDKKNKERKQYINRRSVARNFIKNMEDEDIPEFKKLMEERASKIK

SEQ ID NO: 555 - protein, 59 aa, Bacteriophage D
MPKVSESKRKANDKWDKKNKERKQYINRRSVARNFIKNMEDEDIPEFKKLMEERTSKIK

SEQ ID NO: 556 - protein, 65 aa, Bacteriophage D
MPKVSESKRRANNKWDKKNKERKQYINKRSVARNFIKNMEDEDVPEFKKLMEERASKTNKTCFSS

SEQ ID NO: 557 - protein, 59 aa, Bacteriophage D
MPKVSESKRKANDKWDKNNKERKQYINRRSVARNFIKNMEDEDIPEFKKLMEERTSKIK

SEQ ID NO: 558 - protein, 81 aa, Bacteriophage D
MKLTNQQNQAFKKFKNLRVGALFMEQGTGKTRVALELIRKTDADLALFFCPFSTKNNLLSEIEKWGIDIEFMVYGYETISS

SEQ ID NO: 559 - protein, 58 aa, Bacteriophage D
METEPNFQIICYNKSTSFEVFFYLTTAPEFFQVFFFRPKITRKLWEKLEKIKINEVKT

SEQ ID NO: 560 - protein, 67 aa, Bacteriophage D
METEPNFQIICYNKSTSFEVFFILQLHPNFFRCFFCPKITQKLWEKLEKIKNKRGKNIVCFTNFQAD

SEQ ID NO: 561 - protein, 52 aa, Bacteriophage D
MGFTVTCCNNLRSLSNHNHYCCFLRLVFVPTKIEIIPIIWFIFRVSHGFQTV

SEQ ID NO: 562 - protein, 150 aa, Bacteriophage D
MEYLASFRLNSRTVTSTFSRGFLFLQKKLNSLINKNKNYKNLVQLHLFSNFIYFRSRIVLLLNLKRERNHQLYSAGTPDYLKDILFEIPALFALTWNCCLNSFLLSLFLIFNSINIIQKFPKINNMFPKINFFHIFLILVLTNGNVLDIL

SEQ ID NO: 563 - protein, 93 aa, Bacteriophage D
MEVEQRLEQLRQDWLKHPNLTDTLKEYLNEYFYDDYSYCEKCDRIASDSDWFWYEGEDYTDFLHIDCNKEKFYEATKKTSGRRRPEENIKGES

SEQ ID NO: 564 - protein, 75 aa, Bacteriophage D
MKTKTLGRRLRRLRKINGETQKEFAENFGRHYRTVQNWELDCSIPDVFTAMALAEYYNMDVEELVNGEDDYDKEF

SEQ ID NO: 565 - protein, 125 aa, Bacteriophage D
MEKMTMTKNFENFKKGWDNVQQVVNEYSKKLVENSQENVTNRDSEEYQQIKGKDNVISPNHYVTDKGFEVFDVQEAFIHELKGMAASYWCNVVKYILRFQRKNGVEDLKKAKYYLEKLIEKEEGK

SEQ ID NO: 566 - protein, 181 aa, Bacteriophage D
MNKQEAIELVKNTSYSVPIDSPVKHLTEDTVINIIKQLDEPEKATVPDFVAKYIEESREFDRKLNDALSYSNTTVAMDDWFEENEVDNTEIFAKAWLHGYEVEKEKLYTVEIPDPNASGYGKTFLGRDDDGKVVLSTWTGFSSIEFADDWKQSERAQLTEDEIKKGFTWAWNEGFAEEVKE

SEQ ID NO: 567 - protein, 53 aa, Bacteriophage D
MKRFVVTGYKDGWFVFSFPLNAINSYYAIQYASEDELVEGMEFDKLVIKEVKE

SEQ ID NO: 568 - protein, 48 aa, Bacteriophage D
MNIKEVFCIDCYEWKKKEDLTGSKFSNDILYCKECGYALVRTCDRNNK

SEQ ID NO: 569 - protein, 54 aa, Bacteriophage D
MTNIVADLVDSGMSDAWILKNIGMDADELLRLKQLSGLASLFKDKEFTTAWEVG

SEQ ID NO: 570 - protein, 90 aa, Bacteriophage D
METYKEYKQQQKEERERVRALRSEVFSGNAEKLATDIVRISSGDVYKIIPRFGTRYEKSPIIKLDPEEVERHIKEAREVRELAKIMASKE

SEQ ID NO: 571 - protein, 80 aa, Bacteriophage D
MAVVVEASALCWGFFCYNIPISMASHAYAQIRSDGRFFLLPLKRTKKFKKFDFIVDNTRISVYNVIKDKESEENKNGSKN

SEQ ID NO: 572 - protein, 156 aa, Bacteriophage D
MLGLFLCYNRIKKQIDEVRKTAIDLYRELDIQSLEQRLEKNEENTQRFLQQTAKSLNQDKTELSLRTDQLGRSVEKIENKLDDMYAKNELDLKFQMMDQKIDAKFDTFGQRMENMFLAQTNRQLEEQAKNRKEFTYWFICILVAIAVIAIPVWFGK

SEQ ID NO: 573 - protein, 67 aa, Bacteriophage D
MSFFTSTKTATSTFFIASNRILASFRLNSRTVHPSFLGGFFVLQKNLNLFIKSIDKLSCMIYNILIR

SEQ ID NO: 574 - protein, 42 aa, Bacteriophage D
MLLIVTFSYIINYLLFDLGSSLIKKGERKCYYKGFKTKKDVI

SEQ ID NO: 575 - protein, 28 aa, Bacteriophage D
MECLYFRKKEGACSLFFMYSIKSILYKF

SEQ ID NO: 576 - protein, 229 aa, Bacteriophage D
MDIYVYTDESGVFDKEHETIYVYGGVIFLTSEDKENSGRRYIYAEKALRKSHSNYRKGELKASRLKNRHKASLFRSLNREIKFSIVVSIGRVHDRIFCEKKSKQRYLDYVYKVGLKKVLQRLVADCKIETTEVDTISIFTDEHSTATNGKYELREALLNEFKYGTFNPDWNIFYPPLFEKLSSLTVEYCNSAKKPHIRMADIIANRAYYLAKNDLFGELGEKTISIHFP

SEQ ID NO: 577 - protein, 44 aa, Bacteriophage D
MESWERKLYQSTSLSFRKRRGCKPLFIIMVKYVGFCLILFMTLG

SEQ ID NO: 578 - protein, 49 aa, Bacteriophage M
MHKKGIHIKKVGYFSRLFFLCHVNSSIAFSIMLSMSCRFSNFFKCWKLF

SEQ ID NO: 579 - protein, 46 aa, Bacteriophage M
MLGGLRRPLFDISTASHPSFLGGFFVLQKIFLSKVRIHTKNTLLTF

SEQ ID NO: 580 - protein, 145 aa, Bacteriophage P
MNEIALSDNLAQIELEINHHKQIAGQSIWEIGRRLNHVKEHDLAHGQFMEWVEKLGINQPEANRMMRVAKELPNSSTLSNLGSTALYLIATLPDDEKQEQIEKIEQGESPTVRELQEIKRRLKLKDQALEAVKGELERAILGIKV

SEQ ID NO: 581 - protein, 145 aa, Bacteriophage P
MNEIALSDNLAQIELEINHHKQIAGQSIWEIGRRLNHVKEHDLAHGQFMEWVEKLGINQPEANRMMRVAKELPNSSTLSNLGSTALYLIATLPDDEKQEQIEKIEQGESPTVRELQEIKRRLKLKDQELEAVKGELERAILGIKV

SEQ ID NO: 582 - protein, 111 aa, Bacteriophage P
MEELEQAFENLDDWYLSSMKDSAYKDFGKYEIRLSNHSADNKYHDLENGRLIVNVKASKLNFVDIIENKIYKIIEKIETLDLDKYRFINATKMENDIKCYYKGFKTKKDVI

SEQ ID NO: 583 - protein, 58 aa, Bacteriophage P
MTDAHKKAVKKWNKNNREHRNYLNKRSSARGFIRNNATAEDLRELEELIAERRKKNFR

SEQ ID NO: 584 - protein, 97 aa, Bacteriophage P
MLNLKRERNHQLYSAGTPDYLKDILFEIPALFALTWNCCLNSFLLSLFLIFNSINIIQKFPKNKQYVPKNKLFSYFFDFSVDKWERVRYTIIVLRNK

SEQ ID NO: 585 - protein, 34 aa, Bacteriophage P
MQKKYIIFYKNSFRLVAKIDLNGLKTILKTFDKK

SEQ ID NO: 586 - protein, 34 aa, Bacteriophage P
MRTHKHKGKFCWGGLRRPLFDIIYLYQRPPTRLF

SEQ ID NO: 587 - protein, 43 aa, Bacteriophage P
MLGLFFNINATILMDTVKREASRYDGFYGPDRLVFRKSQTIRY

SEQ ID NO: 588 - protein, 73 aa, Bacteriophage TPL
MYAKNELDLKFQMMDQKIDAKFDTFGQRMENMFLAQTNRQLEEQAKNRKEFTYWFICILVAIAVIAIPVWFGK

SEQ ID NO: 589 - protein, 73 aa, Bacteriophage TPJ; identical to SEQ ID NO: 588

SEQ ID NO: 590 - protein, 60 aa, Bacteriophage D
MDTYKEQFYYLDPIYISVDINRRTFILGKRGQSLSFFIVIKQFKNITKKTSKKSKKNIDK

SEQ ID NO: 591 - protein, 58 aa, Bacteriophage P
MLGLFLCYNMNEMSIPPHPFMDRYVLSGGFFVLLFFNLTARNSPTSKVAGCKGFGLVQ

SEQ ID NO: 592 - protein, 64 aa, Bacteriophage D
MFSDLVRSKVYKGTFCCGLRPPFFDIIYLYQCPPTHKRRYVLREVFYLFYFDKNATILTDTVKS

SEQ ID NO: 593 - protein, 64 aa, Bacteriophage D
MFSDLVRSQVYKGTFCCGLRPPFFDIIYLYQCPPTHKRRYVLREVFYLFYFDINATIIMDTVKS

SEQ ID NO: 594 - protein, 87 aa, Bacteriophage P
MNSMKKPHTAENGDLIHTTEDNEASDISIITISFVRKTNKQILKNSKVCLKRYKLKYLNHLPIQRLIKQYSTEISKQKEIIALEKNE

SEQ ID NO: 595 - protein, 80 aa, Bacteriophage P
MNSMKKPHTAENGDLIHTTEDNEASDISIITISFVRKTNKQILKNSKVCLKRYKLKYLNHLPIQRLIKQYSTEISKQKEY

SEQ ID NO: 596 - protein, 26 aa, Bacteriophage D
MFSDLVRSKVYKGTFCCGLRPPFFLI

SEQ ID NO: 597 - protein, 50 aa, Bacteriophage D
MAVVVEASAFLLGLFLCYNMKHHFMDRYLLCFDKNATILMVFDKLSLALT

SEQ ID NO: 598 - protein, 91 aa, Bacteriophage D
MITKEQLKGYYSEHLEELVEWADDINKIAYEIDGKSHQTKIGWVNDRLKDHFMKEKGVLVIHYTNEQVETAYNEWVKITEEAFNGFFNNTI

SEQ ID NO: 599 - protein, 45 aa, Bacteriophage P
MAAVVEASAFLLGLFLCYNMNEMSIPPHPFMDRYVLMGSFLFALF

SEQ ID NO: 600 - protein, 48 aa, Bacteriophage D
MAVVVEASALCWGFFCVIIYLYQWPPTHTRRYVLMGGFFVAVKTDKKI

SEQ ID NO: 601 - protein, 39 aa, Bacteriophage D
MVEASALCWGFFCVIIHISMASHAYAQIRSEGSFLFAFF

SEQ ID NO: 602 - protein, 41 aa, Bacteriophage D
MAVVVEASAFCWGFFCVIIYMERQTPCIHMDRYALTQGFFI

SEQ ID NO: 603 - protein, 43 aa, Bacteriophage P
MAAVVEASAFLLGLFLCYNIPISMASHAYAQIRSEGGFLFALF

SEQ ID NO: 604 - protein, 172 aa, Bacteriophage D
MENYSSPVYNIKKIPIEKIQANSYNPNHVATPEMKLLYESIKADGYTMPIVCYYLKDEDKYEIVDGFHRYTTMLNHKDIYERENGCLPVSVIDKPLEERMASTVRHNRARGSHDIGLMANIVTELVDSGMSDAKVMKSLGMDADELLRLKQVSGLASLFANKEFSKSWDIKK

SEQ ID NO: 605 - protein, 171 aa, Bacteriophage D
MQTYSSPVYNIKRVPIEKIQANSYNPNHVASPEMKLLYQSIKEDGYTMPIVCYYLEDEDKYEIVDGFHRYTTMKEHKDIYEREEGCLPVSVIDKPISDRMASTIRHNRARGSHDIGLMTNIISDLVDSGMSDAWIMKNIGMDADELLRLKQVSGLASLFKDKEFTTAWEEG

SEQ ID NO: 606 - protein, 171 aa, Bacteriophage D
MQTYSSPVYNIKRVPIDKIQANSYNPNHVASPEMKLLYQSIKEDGYTMPIVCYYLEDEDKYEIVDGFHRYTTMKEHKDIYEREEGCLPVSVIDKPISDRMASTIRHNRARGSHDIGLMTNIISDLVDSGMSDAWIMKNIGMDADELLRLKQVSGLASLFKDKEFTTAWEEG

SEQ ID NO: 607 - protein, 170 aa, Bacteriophage D
MQTYYSPVYNIKRVPIEKIQANSYNPNHVASPEMKLLYQSIKEDGYTMPIVCYYLEDEDKYEIVDGFHRYTTMKEHKDIYEREEGCLPVSVIDKPISDRMASTIRHNRARGSHDIGLMTNIISDLVDSGMSDAWIMKNIGMDADELLRLKQVSGLASLFKDKEFTTAWEE

SEQ ID NO: 608 - protein, 74 aa, Bacteriophage D
MAQIKDGWHKVYNENVYVENEKVVRGTKKDYNGSEVTCYPYEYDKNQDCWINISGKATLSSYRAGLKKGTKCMK

SEQ ID NO: 609 - protein, 45 aa, Bacteriophage D
MFSDLVRSKVYKGTFCCGLRPPFFDIIYLYQCPPTHKRRYVLSLR

SEQ ID NO: 610 - protein, 40 aa, Bacteriophage D
MLGLFLCYNMNEMSIPPHPFMDRYVLSGGFFVLLFFKNVV

SEQ ID NO: 611 - protein, 46 aa, Bacteriophage D
MLGLFLCYNMNEMSIPPHPFMDRYVLSGGFLFCYFLKMWYNINIHS

SEQ ID NO: 612 - protein, 85 aa, Bacteriophage D
MKKFWHSGMIDKKVIEKRKQDDYMNKLHRTILELSIKPPEPEPWYRHPEMRALLDRIDSMDMIDWYSKYLKHRKPYDNYSGELEK

SEQ ID NO: 613 - protein, 59 aa, Bacteriophage
MKKFWRSGMIDKKVIEKRQQEEYINKLHRTILELSIKPPEPEPWYRHPEMRALLDRIDD

SEQ ID NO: 614 - protein, 65 aa, Bacteriophage D
MKKFWRSGMIDKKVIEKRQQDDYMNKLHRTILELSIKPPEPEPWYRHPEMRAFLDRIYDSRSNLK

SEQ ID NO: 615 - protein, 59 aa, Bacteriophage D
MKKFWRSGMIDKKIIAKREQDEYLNKLHRTILELSRKPPEQEPWYRHPEMRALLDRIDD

SEQ ID NO: 616 - protein, 59 aa, Bacteriophage D
MKKFWHSGMIDKKVIEKRKQDDYMNKLHRTILELSIKPPEPEPWYRHPEMRALLDRIDD

SEQ ID NO: 617 - protein, 65 aa, Bacteriophage D
MKKFWRSGMIDKKVIEKRQQDDYMNKLHRTILELSIKPPEPEPWYRHPEMRALLDRIYDSRSNLK

SEQ ID NO: 618 - protein, 59 aa, Bacteriophage TPJ
MKKFWRSGMIDKKVIEKRKQDDYMNKLHRTILELSIKPPEPEPWYRHPEMRALLDRIDD

SEQ ID NO: 619 - protein, 59 aa, Bacteriophage Proph; identical to SEQ ID NO: 618

SEQ ID NO: 620 - protein, 58 aa, Bacteriophage D
MKKFWRSGMIDKKVIKKRKQEEYMNKMHRTILELKNEKHPDMMDFMDLIDWYLENRKP

SEQ ID NO: 621 - protein, 62 aa, Bacteriophage D
MKKFWHSGMIDKKVIEKRKQDEYLNKLHRTILELKNEKHPDMMDFMDLIDWYLENRKPRDID

SEQ ID NO: 622 - protein, 62 aa, Bacteriophage D
MKKFWHSGMIDKKVIEKRKQEECINELHRTILELKNEKHPDMMDFMDLIDWYLENRKPRDIY

SEQ ID NO: 623 - protein, 60 aa, Bacteriophage D
MIDKKVIEKRKQDEYLNKLHRTILELKNEKHPDMIDFMDLIDFMDLIDWYLENRKPRDID

SEQ ID NO: 624 - protein, 62 aa, Bacteriophage D
MNKFWHSGMIDKKVIENRKQEEYINKLHSTILELKNEKHPDMMDFMDLIDWYLENRKPQDID

SEQ ID NO: 625 - protein, 62 aa, Bacteriophage P
MKKFWRSGMIDNKVIEKRKQDDYMNKLHRTILELTREIELRRGPDMMDFMDLIDWYLNSRKP

SEQ ID NO: 626 - protein, 71 aa, Bacteriophage D
MKKFWHSGMIDKKVIEKRQHDEYINKIHKTIIELRKEPPEPKPCSCHKDIDINALINDIEWDDYYTWFKDK

SEQ ID NO: 627 - protein, 71 aa, Bacteriophage D
MKKFWRSGMIDKKVIEKRKQDDYMNKLHRTILELSIKPPEPKPCSCHKDIDINALINDIEWDDYYTWFKDK

SEQ ID NO: 628 - protein, 71 aa, Bacteriophage D
MKKFWRSGMIDKKVIEKRKQEEYMNKMHRTILELSIKPPEPKPCSCHKDIDINALINDIEWDDYYTWFKDK

SEQ ID NO: 629 - protein, 63 aa, Bacteriophage D
MIDKKVIEKRKQDDYMNKLHRTILELSIKPPEPKPCSCHKDIDINALINDIEWDDYYTWFKDK

SEQ ID NO: 630 - protein, 71 aa, Bacteriophage D
MKKFWHSGMIDKKVIKKRKQEEYMNKLQRIILELSIKPPEPKPCSCHKDIDINALINDIEWDDYYTWFKDK

SEQ ID NO: 631 - protein, 70 aa, Bacteriophage O
MKKFWHSGMIDKKIIEKREHDEYLNKLHMTIIELRKEPPETKPCSCHKNVDINELINYIEWNDYYTWFKD

SEQ ID NO: 632 - protein, 60 aa, Bacteriophage D
MKKFWHSGMIDKKVIEKRKQDEYLNKLHRTILEIDFPIQRVCHRSLSPTPITVPTETLDI

SEQ ID NO: 633 - protein, 44 aa, Bacteriophage D
MKKFWHSGMIDKKVIKKRKQEEYMNKMHRTILELSIKPIEEMVF

SEQ ID NO: 634 - protein, 88 aa, Bacteriophage Sfi
MKKFWRSGMIDKKVIEKRKQDDYMNKLHRTILELSIKPPEPKPCSCHKDIDINALINDIEWDDWVDEVLEYINKWVNKDKADVEVLDK

SEQ ID NO: 635 - protein, 210 aa, Bacteriophage D
MTTPQKFLSIRELLKPLPSNGVKFPKFSALYHESQVGAWQKKMSKRRHQAKVQVAMDKNRGELVPRELEDFSNWQRARQMKARYQEKVANKRKDYLHKLTTYLVKTYDVIVIEDLKAKNLMKNHYLAKSIANASWHEFKRLLEYKCSWYGKELIVVPAHHTSQECSNCHHNSGKKPLHIREWMCDNCGTHHDRDINASINILHRGLATLN

SEQ ID NO: 636 - protein, 100 aa, Bacteriophage D
MSTVFLIFFQVFLILLLNILKISKTYYILFFVCIHCFYLVFLFFIECFPSCSQSILVYFGDQTETVFIKKYIFFCKTKTLTNSSQGKREFIEDSAFNCIH

SEQ ID NO: 637 - protein, 100 aa, Bacteriophage D
MSTVFLIFFQVFLIFLLNILKISKTYYILFFVCIHCFYLVFLFFIECFPSCSQSILVYFGDQTETVFIKKYIFFCKTKTLTNSSQGEREFIEDSAFNCIH

SEQ ID NO: 638 - protein, 100 aa, Bacteriophage P
MSTVFLIFFQVFLIFLLNILKISKTYYILFFVCIHCFYLVFLFFIECFPSCSQSILVYFGDQTETVFIKKYIFFCKTKTLTNSSQGEREFIEDNSFYCNH

SEQ ID NO: 639 - protein, 76 aa, Bacteriophage P
MIFFKVFLILLLNNLKISKTYYILFFVCIHCFYLVFLFFIEYFPDCFQSIQVDFCDQTETVFIKNYIFFLQNKNPD

SEQ ID NO: 640 - protein, 81 aa, Bacteriophage P
MSIVFLIFFKVFLILLLNNLKISKTYYILFFVCIHCFYLVFLFFIEYFPDCFQSIQVDFCDQTETVFIKKYIFFLQNKNPD

SEQ ID NO: 641 - protein, 77 aa, Bacteriophage P
MSTVFLIFFQVFLIFLYIYFKISKTYYILFFVCIHCFFIFYRMFSKLLSIHSSLFWRPDGNCFYKKIYIFLQNKNPD

SEQ ID NO: 642 - protein, 72 aa, Bacteriophage P
MIFFQVFLIFLLNILKISKTYYILFFVCIHCFLFFIECFPSCSQSILVYFGDQTETVFIKKIYIFLQNKNPD

SEQ ID NO: 643 - protein, 65 aa, Bacteriophage D
MFIFGNCCIMFILYISCMIVCQQFYLNYFSFFCKKRKPRLKVEVTVREFNRNDTKYSNNYITTFL

SEQ ID NO: 644 - protein, 62 aa, Bacteriophage D
MSSEHSIQNQIRVELSKAGNMVFRINVGKVRMADGRWFDTGAPKGFCDLFGFRPATVIALIY

SEQ ID NO: 645 - protein, 46 aa, Bacteriophage P
MPILFIVGNAQGASHCTRPKPLHPATLEVGELRAVRLKKANKKAPA

SEQ ID NO: 646 - protein, 56 aa, Bacteriophage P
MSTVFLIFFQVFLIFLLNILKISKTYYILFFVCIHCFFIFYRMFSKLLSIHSSLFW

SEQ ID NO: 647 - protein, 47 aa, Bacteriophage P
MIFFQVFLIFLLNILKISKTYYILFFVCIHCFFYFLSNVFQVALNPF

SEQ ID NO: 648 - protein, 56 aa, Bacteriophage P
MVLAPNKTFPYACVCASNRALNLISLLPFALDKLYLGYPITFYQIIIYKSNKKAPA

SEQ ID NO: 649 - protein, 65 aa, Bacteriophage P
MRINEAVLSFYSFYFYLLRNLVFFCKKRKPRLKVEVTVREFNRNDAKYSNNYMKIANKKSYEIIS

SEQ ID NO: 650 - protein, 64 aa, Bacteriophage Sequence
MFYLLTKASFYLSLYLMYTLHIIYDSLPTVFIKKYIFFCKTKTLTNSSQGEREFIEDSAFNCIH